European Patent Application EP 4 477 759 A1, published December 18, 2024. Title: METHOD FOR PREDICTING OFF-TARGET WHICH CAN OCCUR IN PROCESS OF EDITING GENOME BY USING PRIME EDITING SYSTEM. Applicant: TOOLGEN INCORPORATED. Application KR PCT/KR2023/001867, filed February 8, 2023. The sequence listing filed with the application follows.

SEQUENCE LISTING (524 sequences)

SEQ ID NO: 1 - protein, 7 aa, synthetic construct
PKKKRKV

SEQ ID NO: 2 - protein, 16 aa, synthetic construct
KRPAATKKAGQAKKKK

SEQ ID NO: 3 - protein, 9 aa, synthetic construct
PAAKRVKLD

SEQ ID NO: 4 - protein, 11 aa, synthetic construct
RQRRNELKRSP

SEQ ID NO: 5 - protein, 38 aa, synthetic construct
NQSSNFGPMKGGNFGGRSSGPYGGGGQYFAKPRNQGGY

SEQ ID NO: 6 - protein, 42 aa, synthetic construct
RMRIZFKNKGKDTAELRRRRVEVSVELRKAKKDEQILKRRNV

SEQ ID NO: 7 - protein, 8 aa, synthetic construct
VSRKRPRP

SEQ ID NO: 8 - protein, 8 aa, synthetic construct
PPKKARED

SEQ ID NO: 9 - protein, 8 aa, synthetic construct
PQPKKKPL

SEQ ID NO: 10 - protein, 12 aa, synthetic construct
SALIKKKKKMAP

SEQ ID NO: 11 - protein, 5 aa, synthetic construct
DRLRR

SEQ ID NO: 12 - protein, 7 aa, synthetic construct
PKQKKRK

SEQ ID NO: 13 - protein, 10 aa, synthetic construct
RKLKKKIKKL

SEQ ID NO: 14 - protein, 10 aa, synthetic construct
REKKKFLKRR

SEQ ID NO: 15 - protein, 20 aa, synthetic construct
KRKGDEVDGVDEVAKKKSKK

SEQ ID NO: 16 - protein, 17 aa, synthetic construct
RKCLQAGMNLEARKTKK

SEQ ID NO: 17 - protein, 30 aa, synthetic construct
MDSLLMNRRKFLYQFKNVRWAKGRRETYLC

SEQ ID NO: 18 - protein, 19 aa, synthetic construct
KRTADGSEFESPKKKRKVE

SEQ ID NO: 19-25 - skipped (7 entries)

SEQ ID NO: 26 - protein, 672 aa, synthetic construct
TLNIEDEHRLHETSKEPDVSLGSTWLSDFPQAWAETGGMGLAVRQAPLIIPLKATSTPVSIKQYPMSQEARLGIKPHIQRLLDQGILVPCQSPWNTPLLPVKKPGTNDYRPVQDLREVNKRVEDIHPTVPNPYNLLSGLPPSHQWYTVLDLKDAFFCLRLHPTSQPLFAFEWRDPEMGISGQLTWTRLPQGFKNSPTLFDEALHRDLADFRIQHPDLILLQYVDDLLLAATSELDCQQGTRALLQTLGNLGYRASAKKAQICQKQVKYLGYLLKEGQRWLTEARKETVMGQPTPKTPRQLREFLGTAGFCRLWIPGFAEMAAPLYPLTKTGTLFNWGPDQQKAYQEIKQALLTAPALGLPDLTKPFELFVDEKQGYAKGVLTQKLGPWRRPVAYLSKKLDPVAAGWPPCLRMVAAIAVLTKDAGKLTMGQPLVILAPHAVEALVKQPPDRWLSNARMTHYQALLLDTDRVQFGPVVALNPATLLPLPEEGLQHNCLDILAEAHGTRPDLTDQPLPDADHTWYTDGSSLLQEGQRKAGAAVTTETEVIWAKALPAGTSAQRAELIALTQALKMAEGKKLNVYTDSRYAFATAHIHGEIYRRRGLLTSEGKEIKNKDEILALLKALFLPKRLSIIHCPGHQKGHSAEARGNRMADQAARKAAITETPDTSTLLI

SEQ ID NO: 27 - protein, 672 aa, synthetic construct
TLNIEDEYRLHETSKEPDVSLGSTWLSDFPQAWAETGGMGLAVRQAPLIIPLKATSTPVSIKQYPMSQEARLGIKPHIQRLLDQGILVPCQSPWNTPLLPVKKPGTNDYRPVQDLREVNKRVEDIHPTVPNPYNLLSGLPPSHQWYTVLDLKDAFFCLRLHPTSQPLFAFEWRDPEMGISGQLTWTRLPQGFKNSPTLFNEALHRDLADFRIQHPDLILLQYVDDLLLAATSELDCQQGTRALLQTLGNLGYRASAKKAQICQKQVKYLGYLLKEGQRWLTEARKETVMGQPTPKTPRQLREFLGKAGFCRLFIPGFAEMAAPLYPLTKPGTLFNWGPDQQKAYQEIKQALLTAPALGLPDLTKPFELFVDEKQGYAKGVLTQKLGPWRRPVAYLSKKLDPVAAGWPPCLRMVAAIAVLTKDAGKLTMGQPLVILAPHAVEALVKQPPDRWLSNARMTHYQALLLDTDRVQFGPVVALNPATLLPLPEEGLQHNCLDILAEAHGTRPDLTDQPLPDADHTWYTDGSSLLQEGQRKAGAAVTTETEVIWAKALPAGTSAQRAELIALTQALKMAEGKKLNVYTDSRYAFATAHIHGEIYRRRGWLTSEGKEIKNKDEILALLKALFLPKRLSIIHCPGHQKGHSAEARGNRMADQAARKAAITETPDTSTLLI

SEQ ID NO: 28 - protein, 1368 aa, synthetic construct [sequence omitted]

SEQ ID NO: 29 - protein, 1368 aa, synthetic construct
MDKKYSIGLDIGTNSVGWAVITDEYKVPSKKFKVLGNTDRHSIKKNLIGALLFDSGETAEATRLKRTARRRYTRRKNRICYLQEIFSNEMAKVDDSFFHRLEESFLVEEDKKHERHPIFGNIVDEVAYHEKYPTIYHLRKKLVDSTDKADLRLIYLALAHMIKFRGHFLIEGDLNPDNSDVDKLFIQLVQTYNQLFEENPINASGVDAKAILSARLSKSRRLENLIAQLPGEKKNGLFGNLIALSLGLTPNFKSNFDLAEDAKLQLSKDTYDDDLDNLLAQIGDQYADLFLAAKNLSDAILLSDILRVNTEITKAPLSASMIKRYDEHHQDLTLLKALVRQQLPEKYKEIFFDQSKNGYAGYIDGGASQEEFYKFIKPILEKMDGTEELLVKLNREDLLRKQRTFDNGSIPHQIHLGELHAILRRQEDFYPFLKDNREKIEKILTFRIPYYVGPLARGNSRFAWMTRKSEETITPWNFEEVVDKGASAQSFIERMTNFDKNLPNEKVLPKHSLLYEYFTVYNELTKVKYVTEGMRKPAFLSGEQKKAIVDLLFKTNRKVTVKQLKEDYFKKIECFDSVEISGVEDRFNASLGTYHDLLKIIKDKDFLDNEENEDILEDIVLTLTLFEDREMIEERLKTYAHLFDDKVMKQLKRRRYTGWGRLSRKLINGIRDKQSGKTILDFLKSDGFANRNFMQLIHDDSLTFKEDIQKAQVSGQGDSLHEHIANLAGSPAIKKGILQTVKVVDELVKVMGRHKPENIVIEMARENQTTQKGQKNSRERMKRIEEGIKELGSQILKEHPVENTQLQNEKLYLYYLQNGRDMYVDQELDINRLSDYDVDAIVPQSFLKDDSIDNKVLTRSDKNRGKSDNVPSEEVVKKMKNYWRQLLNAKLITQRKFDNLTKAERGGLSELDKAGFIKRQLVETRQITKHVAQILDSRMNTKYDENDKLIREVKVITLKSKLVSDFRKDFQFYKVREINNYHHAHDAYLNAVVGTALIKKYPKLESEFVYGDYKVYDVRKMIAKSEQEIGKATAKYFFYSNIMNFFKTEITLANGEIRKRPLIETNGETGEIVWDKGRDFATVRKVLSMPQVNIVKKTEVQTGGFSKESILPKRNSDKLIARKKDWDPKKYGGFDSPTVAYSVLVVAKVEKGKSKKLKSVKELLGITIMERSSFEKNPIDFLEAKGYKEVKKDLIIKLPKYSLFELENGRKRMLASAGELQKGNELALPSKYVNFLYLASHYEKLKGSPEDNEQKQLFVEQHKHYLDEIIEQISEFSKRVILADANLDKVLSAYNKHRDKPIREQAENIIHLFTLTNLGAPAAFKYFDTTIDRKRYTSTKEVLDATLIHQSITGLYETRIDLSQLGGD

SEQ ID NO: 30 - protein, 1368 aa, synthetic construct
MDKKYSIGLDIGTNSVGWAVITDEYKVPSKKFKVLGNTDRHSIKKNLIGALLFDSGETAEATRLKRTARRRYTRRKNRICYLQEIFSNEMAKVDDSFFHRLEESFLVEEDKKHERHPIFGNIVDEVAYHEKYPTIYHLRKKLVDSTDKADLRLIYLALAHMIKFRGHFLIEGDLNPDNSDVDKLFIQLVQTYNQLFEENPINASGVDAKAILSARLSKSRKLENLIAQLPGEKKNGLFGNLIALSLGLTPNFKSNFDLAEDAKLQLSKDTYDDDLDNLLAQIGDQYADLFLAAKNLSDAILLSDILRVNTEITKAPLSASMIKRYDEHHQDLTLLKALVRQQLPEKYKEIFFDQSKNGYAGYIDGGASQEEFYKFIKPILEKMDGTEELLVKLKREDLLRKQRTFDNGSIPHQIHLGELHAILRRQEDFYPFLKDNREKIEKILTFRIPYYVGPLARGNSRFAWMTRKSEETITPWNFEEVVDKGASAQSFIERMTNFDKNLPNEKVLPKHSLLYEYFTVYNELTKVKYVTEGMRKPAFLSGEQKKAIVDLLFKTNRKVTVKQLKEDYFKKIECFDSVEISGVEDRFNASLGTYHDLLKIIKDKDFLDNEENEDILEDIVLTLTLFEDREMIEERLKTYAHLFDDKVMKQLKRRRYTGWGRLSRKLINGIRDKQSGKTILDFLKSDGFANRNFMQLIHDDSLTFKEDIQKAQVSGQGDSLHEHIANLAGSPAIKKGILQTVKVVDELVKVMGRHKPENIVIEMARENQTTQKGQKNSRERMKRIEEGIKELGSQILKEHPVENTQLQNEKLYLYYLQNGRDMYVDQELDINRLSDYDVDHIVPQSFLKDDSIDNKVLTRSDKNRGKSDNVPSEEVVKKMKNYWRQLLNAKLITQRKFDNLTKAERGGLSELDKAGFIKRQLVETRQITKHVAQILDSRMNTKYDENDKLIREVKVITLKSKLVSDFRKDFQFYKVREINNYHHAHDAYLNAVVGTALIKKYPKLESEFVYGDYKVYDVRKMIAKSEQEIGKATAKYFFYSNIMNFFKTEITLANGEIRKRPLIETNGETGEIVWDKGRDFATVRKVLSMPQVNIVKKTEVQTGGFSKESILPKRNSDKLIARKKDWDPKKYGGFDSPTVAYSVLVVAKVEKGKSKKLKSVKELLGITIMERSSFEKNPIDFLEAKGYKEVKKDLIIKLPKYSLFELENGRKRMLASAGELQKGNELALPSKYVNFLYLASHYEKLKGSPEDNEQKQLFVEQHKHYLDEIIEQISEFSKRVILADANLDKVLSAYNKHRDKPIREQAENIIHLFTLTNLGAPAAFKYFDTTIDRKRYTSTKEVLDATLIHQSITGLYETRIDLSQLGGD

SEQ ID NO: 31 - protein, 1368 aa, synthetic construct
MDKKYSIGLDIGTNSVGWAVITDEYKVPSKKFKVLGNTDRHSIKKNLIGALLFDSGETAEATRLKRTARRRYTRRKNRICYLQEIFSNEMAKVDDSFFHRLEESFLVEEDKKHERHPIFGNIVDEVAYHEKYPTIYHLRKKLVDSTDKADLRLIYLALAHMIKFRGHFLIEGDLNPDNSDVDKLFIQLVQTYNQLFEENPINASGVDAKAILSARLSKSRKLENLIAQLPGEKKNGLFGNLIALSLGLTPNFKSNFDLAEDAKLQLSKDTYDDDLDNLLAQIGDQYADLFLAAKNLSDAILLSDILRVNTEITKAPLSASMIKRYDEHHQDLTLLKALVRQQLPEKYKEIFFDQSKNGYAGYIDGGASQEEFYKFIKPILEKMDGTEELLVKLKREDLLRKQRTFDNGSIPHQIHLGELHAILRRQEDFYPFLKDNREKIEKILTFRIPYYVGPLARGNSRFAWMTRKSEETITPWNFEEVVDKGASAQSFIERMTNFDKNLPNEKVLPKHSLLYEYFTVYNELTKVKYVTEGMRKPAFLSGEQKKAIVDLLFKTNRKVTVKQLKEDYFKKIECFDSVEISGVEDRFNASLGTYHDLLKIIKDKDFLDNEENEDILEDIVLTLTLFEDREMIEERLKTYAHLFDDKVMKQLKRRRYTGWGRLSRKLINGIRDKQSGKTILDFLKSDGFANRNFMQLIHDDSLTFKEDIQKAQVSGQGDSLHEHIANLAGSPAIKKGILQTVKVVDELVKVMGRHKPENIVIEMARENQTTQKGQKNSRERMKRIEEGIKELGSQILKEHPVENTQLQNEKLYLYYLQNGRDMYVDQELDINRLSDYDVDAIVPQSFLKDDSIDNKVLTRSDKNRGKSDNVPSEEVVKKMKNYWRQLLNAKLITQRKFDNLTKAERGGLSELDKAGFIKRQLVETRQITKHVAQILDSRMNTKYDENDKLIREVKVITLKSKLVSDFRKDFQFYKVREINNYHHAHDAYLNAVVGTALIKKYPKLESEFVYGDYKVYDVRKMIAKSEQEIGKATAKYFFYSNIMNFFKTEITLANGEIRKRPLIETNGETGEIVWDKGRDFATVRKVLSMPQVNIVKKTEVQTGGFSKESILPKRNSDKLIARKKDWDPKKYGGFDSPTVAYSVLVVAKVEKGKSKKLKSVKELLGITIMERSSFEKNPIDFLEAKGYKEVKKDLIIKLPKYSLFELENGRKRMLASAGELQKGNELALPSKYVNFLYLASHYEKLKGSPEDNEQKQLFVEQHKHYLDEIIEQISEFSKRVILADANLDKVLSAYNKHRDKPIREQAENIIHLFTLTNLGAPAAFKYFDTTIDRKRYTSTKEVLDATLIHQSITGLYETRIDLSQLGGD

SEQ ID NO: 32 - protein, 2117 aa, synthetic construct
MKRTADGSEFESPKKKRKVDKKYSIGLDIGTNSVGWAVITDEYKVPSKKFKVLGNTDRHSIKKNLIGALLFDSGETAEATRLKRTARRRYTRRKNRICYLQEIFSNEMAKVDDSFFHRLEESFLVEEDKKHERHPIFGNIVDEVAYHEKYPTIYHLRKKLVDSTDKADLRLIYLALAHMIKFRGHFLIEGDLNPDNSDVDKLFIQLVQTYNQLFEENPINASGVDAKAILSARLSKSRRLENLIAQLPGEKKNGLFGNLIALSLGLTPNFKSNFDLAEDAKLQLSKDTYDDDLDNLLAQIGDQYADLFLAAKNLSDAILLSDILRVNTEITKAPLSASMIKRYDEHHQDLTLLKALVRQQLPEKYKEIFFDQSKNGYAGYIDGGASQEEFYKFIKPILEKMDGTEELLVKLNREDLLRKQRTFDNGSIPHQIHLGELHAILRRQEDFYPFLKDNREKIEKILTFRIPYYVGPLARGNSRFAWMTRKSEETITPWNFEEVVDKGASAQSFIERMTNFDKNLPNEKVLPKHSLLYEYFTVYNELTKVKYVTEGMRKPAFLSGEQKKAIVDLLFKTNRKVTVKQLKEDYFKKIECFDSVEISGVEDRFNASLGTYHDLLKIIKDKDFLDNEENEDILEDIVLTLTLFEDREMIEERLKTYAHLFDDKVMKQLKRRRYTGWGRLSRKLINGIRDKQSGKTILDFLKSDGFANRNFMQLIHDDSLTFKEDIQKAQVSGQGDSLHEHIANLAGSPAIKKGILQTVKVVDELVKVMGRHKPENIVIEMARENQTTQKGQKNSRERMKRIEEGIKELGSQILKEHPVENTQLQNEKLYLYYLQNGRDMYVDQELDINRLSDYDVDAIVPQSFLKDDSIDNKVLTRSDKNRGKSDNVPSEEVVKKMKNYWRQLLNAKLITQRKFDNLTKAERGGLSELDKAGFIKRQLVETRQITKHVAQILDSRMNTKYDENDKLIREVKVITLKSKLVSDFRKDFQFYKVREINNYHHAHDAYLNAVVGTALIKKYPKLESEFVYGDYKVYDVRKMIAKSEQEIGKATAKYFFYSNIMNFFKTEITLANGEIRKRPLIETNGETGEIVWDKGRDFATVRKVLSMPQVNIVKKTEVQTGGFSKESILPKRNSDKLIARKKDWDPKKYGGFDSPTVAYSVLVVAKVEKGKSKKLKSVKELLGITIMERSSFEKNPIDFLEAKGYKEVKKDLIIKLPKYSLFELENGRKRMLASAGELQKGNELALPSKYVNFLYLASHYEKLKGSPEDNEQKQLFVEQHKHYLDEIIEQISEFSKRVILADANLDKVLSAYNKHRDKPIREQAENIIHLFTLTNLGAPAAFKYFDTTIDRKRYTSTKEVLDATLIHQSITGLYETRIDLSQLGGDSGGSSGGSSGSETPGTSESATPESSGGSSGGSSTLNIEDEYRLHETSKEPDVSLGSTWLSDFPQAWAETGGMGLAVRQAPLIIPLKATSTPVSIKQYPMSQEARLGIKPHIQRLLDQGILVPCQSPWNTPLLPVKKPGTNDYRPVQDLREVNKRVEDIHPTVPNPYNLLSGLPPSHQWYTVLDLKDAFFCLRLHPTSQPLFAFEWRDPEMGISGQLTWTRLPQGFKNSPTLFNEALHRDLADFRIQHPDLILLQYVDDLLLAATSELDCQQGTRALLQTLGNLGYRASAKKAQICQKQVKYLGYLLKEGQRWLTEARKETVMGQPTPKTPRQLREFLGKAGFCRLFIPGFAEMAAPLYPLTKPGTLFNWGPDQQKAYQEIKQALLTAPALGLPDLTKPFELFVDEKQGYAKGVLTQKLGPWRRPVAYLSKKLDPVAAGWPPCLRMVAAIAVLTKDAGKLTMGQPLVILAPHAVEALVKQPPDRWLSNARMTHYQALLLDTDRVQFGPVVALNPATLLPLPEEGLQHNCLDILAEAHGTRPDLTDQPLPDADHTWYTDGSSLLQEGQRKAGAAVTTETEVIWAKALPAGTSAQRAELIALTQALKMAEGKKLNVYTDSRYAFATAHIHGEIYRRRGWLTSEGKEIKNKDEILALLKALFLPKRLSIIHCPGHQKGHSAEARGNRMADQAARKAAITETPDTSTLLIENSSPSGGSKRTADGSEFEPKKKRKV

SEQ ID NO: 33 - protein, 2117 aa, synthetic construct
MKRTADGSEFESPKKKRKVDKKYSIGLDIGTNSVGWAVITDEYKVPSKKFKVLGNTDRHSIKKNLIGALLFDSGETAEATRLKRTARRRYTRRKNRICYLQEIFSNEMAKVDDSFFHRLEESFLVEEDKKHERHPIFGNIVDEVAYHEKYPTIYHLRKKLVDSTDKADLRLIYLALAHMIKFRGHFLIEGDLNPDNSDVDKLFIQLVQTYNQLFEENPINASGVDAKAILSARLSKSRRLENLIAQLPGEKKNGLFGNLIALSLGLTPNFKSNFDLAEDAKLQLSKDTYDDDLDNLLAQIGDQYADLFLAAKNLSDAILLSDILRVNTEITKAPLSASMIKRYDEHHQDLTLLKALVRQQLPEKYKEIFFDQSKNGYAGYIDGGASQEEFYKFIKPILEKMDGTEELLVKLNREDLLRKQRTFDNGSIPHQIHLGELHAILRRQEDFYPFLKDNREKIEKILTFRIPYYVGPLARGNSRFAWMTRKSEETITPWNFEEVVDKGASAQSFIERMTNFDKNLPNEKVLPKHSLLYEYFTVYNELTKVKYVTEGMRKPAFLSGEQKKAIVDLLFKTNRKVTVKQLKEDYFKKIECFDSVEISGVEDRFNASLGTYHDLLKIIKDKDFLDNEENEDILEDIVLTLTLFEDREMIEERLKTYAHLFDDKVMKQLKRRRYTGWGRLSRKLINGIRDKQSGKTILDFLKSDGFANRNFMQLIHDDSLTFKEDIQKAQVSGQGDSLHEHIANLAGSPAIKKGILQTVKVVDELVKVMGRHKPENIVIEMARENQTTQKGQKNSRERMKRIEEGIKELGSQILKEHPVENTQLQNEKLYLYYLQNGRDMYVDQELDINRLSDYDVDHIVPQSFLKDDSIDNKVLTRSDKNRGKSDNVPSEEVVKKMKNYWRQLLNAKLITQRKFDNLTKAERGGLSELDKAGFIKRQLVETRQITKHVAQILDSRMNTKYDENDKLIREVKVITLKSKLVSDFRKDFQFYKVREINNYHHAHDAYLNAVVGTALIKKYPKLESEFVYGDYKVYDVRKMIAKSEQEIGKATAKYFFYSNIMNFFKTEITLANGEIRKRPLIETNGETGEIVWDKGRDFATVRKVLSMPQVNIVKKTEVQTGGFSKESILPKRNSDKLIARKKDWDPKKYGGFDSPTVAYSVLVVAKVEKGKSKKLKSVKELLGITIMERSSFEKNPIDFLEAKGYKEVKKDLIIKLPKYSLFELENGRKRMLASAGELQKGNELALPSKYVNFLYLASHYEKLKGSPEDNEQKQLFVEQHKHYLDEIIEQISEFSKRVILADANLDKVLSAYNKHRDKPIREQAENIIHLFTLTNLGAPAAFKYFDTTIDRKRYTSTKEVLDATLIHQSITGLYETRIDLSQLGGDSGGSSGGSSGSETPGTSESATPESSGGSSGGSSTLNIEDEYRLHETSKEPDVSLGSTWLSDFPQAWAETGGMGLAVRQAPLIIPLKATSTPVSIKQYPMSQEARLGIKPHIQRLLDQGILVPCQSPWNTPLLPVKKPGTNDYRPVQDLREVNKRVEDIHPTVPNPYNLLSGLPPSHQWYTVLDLKDAFFCLRLHPTSQPLFAFEWRDPEMGISGQLTWTRLPQGFKNSPTLFNEALHRDLADFRIQHPDLILLQYVDDLLLAATSELDCQQGTRALLQTLGNLGYRASAKKAQICQKQVKYLGYLLKEGQRWLTEARKETVMGQPTPKTPRQLREFLGKAGFCRLFIPGFAEMAAPLYPLTKPGTLFNWGPDQQKAYQEIKQALLTAPALGLPDLTKPFELFVDEKQGYAKGVLTQKLGPWRRPVAYLSKKLDPVAAGWPPCLRMVAAIAVLTKDAGKLTMGQPLVILAPHAVEALVKQPPDRWLSNARMTHYQALLLDTDRVQFGPVVALNPATLLPLPEEGLQHNCLDILAEAHGTRPDLTDQPLPDADHTWYTDGSSLLQEGQRKAGAAVTTETEVIWAKALPAGTSAQRAELIALTQALKMAEGKKLNVYTDSRYAFATAHIHGEIYRRRGWLTSEGKEIKNKDEILALLKALFLPKRLSIIHCPGHQKGHSAEARGNRMADQAARKAAITETPDTSTLLIENSSPSGGSKRTADGSEFEPKKKRKV

SEQ ID NO: 34 - protein, 2131 aa, synthetic construct
MKRTADGSEFESPKKKRKVDKKYSIGLDIGTNSVGWAVITDEYKVPSKKFKVLGNTDRHSIKKNLIGALLFDSGETAEATRLKRTARRRYTRRKNRICYLQEIFSNEMAKVDDSFFHRLEESFLVEEDKKHERHPIFGNIVDEVAYHEKYPTIYHLRKKLVDSTDKADLRLIYLALAHMIKFRGHFLIEGDLNPDNSDVDKLFIQLVQTYNQLFEENPINASGVDAKAILSARLSKSRKLENLIAQLPGEKKNGLFGNLIALSLGLTPNFKSNFDLAEDAKLQLSKDTYDDDLDNLLAQIGDQYADLFLAAKNLSDAILLSDILRVNTEITKAPLSASMIKRYDEHHQDLTLLKALVRQQLPEKYKEIFFDQSKNGYAGYIDGGASQEEFYKFIKPILEKMDGTEELLVKLKREDLLRKQRTFDNGSIPHQIHLGELHAILRRQEDFYPFLKDNREKIEKILTFRIPYYVGPLARGNSRFAWMTRKSEETITPWNFEEVVDKGASAQSFIERMTNFDKNLPNEKVLPKHSLLYEYFTVYNELTKVKYVTEGMRKPAFLSGEQKKAIVDLLFKTNRKVTVKQLKEDYFKKIECFDSVEISGVEDRFNASLGTYHDLLKIIKDKDFLDNEENEDILEDIVLTLTLFEDREMIEERLKTYAHLFDDKVMKQLKRRRYTGWGRLSRKLINGIRDKQSGKTILDFLKSDGFANRNFMQLIHDDSLTFKEDIQKAQVSGQGDSLHEHIANLAGSPAIKKGILQTVKVVDELVKVMGRHKPENIVIEMARENQTTQKGQKNSRERMKRIEEGIKELGSQILKEHPVENTQLQNEKLYLYYLQNGRDMYVDQELDINRLSDYDVDHIVPQSFLKDDSIDNKVLTRSDKNRGKSDNVPSEEVVKKMKNYWRQLLNAKLITQRKFDNLTKAERGGLSELDKAGFIKRQLVETRQITKHVAQILDSRMNTKYDENDKLIREVKVITLKSKLVSDFRKDFQFYKVREINNYHHAHDAYLNAVVGTALIKKYPKLESEFVYGDYKVYDVRKMIAKSEQEIGKATAKYFFYSNIMNFFKTEITLANGEIRKRPLIETNGETGEIVWDKGRDFATVRKVLSMPQVNIVKKTEVQTGGFSKESILPKRNSDKLIARKKDWDPKKYGGFDSPTVAYSVLVVAKVEKGKSKKLKSVKELLGITIMERSSFEKNPIDFLEAKGYKEVKKDLIIKLPKYSLFELENGRKRMLASAGELQKGNELALPSKYVNFLYLASHYEKLKGSPEDNEQKQLFVEQHKHYLDEIIEQISEFSKRVILADANLDKVLSAYNKHRDKPIREQAENIIHLFTLTNLGAPAAFKYFDTTIDRKRYTSTKEVLDATLIHQSITGLYETRIDLSQLGGDSGGSSGGSKRTADGSEFESPKKKRKVSGGSSGGSTLNIEDEYRLHETSKEPDVSLGSTWLSDFPQAWAETGGMGLAVRQAPLIIPLKATSTPVSIKQYPMSQEARLGIKPHIQRLLDQGILVPCQSPWNTPLLPVKKPGTNDYRPVQDLREVNKRVEDIHPTVPNPYNLLSGLPPSHQWYTVLDLKDAFFCLRLHPTSQPLFAFEWRDPEMGISGQLTWTRLPQGFKNSPTLFNEALHRDLADFRIQHPDLILLQYVDDLLLAATSELDCQQGTRALLQTLGNLGYRASAKKAQICQKQVKYLGYLLKEGQRWLTEARKETVMGQPTPKTPRQLREFLGKAGFCRLFIPGFAEMAAPLYPLTKPGTLFNWGPDQQKAYQEIKQALLTAPALGLPDLTKPFELFVDEKQGYAKGVLTQKLGPWRRPVAYLSKKLDPVAAGWPPCLRMVAAIAVLTKDAGKLTMGQPLVILAPHAVEALVKQPPDRWLSNARMTHYQALLLDTDRVQFGPVVALNPATLLPLPEEGLQHNCLDILAEAHGTRPDLTDQPLPDADHTWYTDGSSLLQEGQRKAGAAVTTETEVIWAKALPAGTSAQRAELIALTQALKMAEGKKLNVYTDSRYAFATAHIHGEIYRRRGWLTSEGKEIKNKDEILALLKALFLPKRLSIIHCPGHQKGHSAEARGNRMADQAARKAAITETPDTSTLLIENSSPSGGSKRTADGSEFESPKKKRKVGSGPAAKRVKLD

SEQ ID NO: 35 - protein, 5 aa, synthetic construct
EAAAK

SEQ ID NO: 36 - skipped

SEQ ID NO: 37 - protein, 4 aa, synthetic construct
SGGS

SEQ ID NO: 38 - protein, 5 aa, synthetic construct
GGGGS

SEQ ID NO: 39 - protein, 16 aa, synthetic construct
SGSETPGTSESATPES

SEQ ID NO: 40 - protein, 32 aa, synthetic construct
SGGSSGGSSGSETPGTSESATPESSGGSSGGS

SEQ ID NO: 41 - RNA, 37 nt, synthetic construct
  source 1..37: mol_type = other RNA
cgcggttctatctagttacgcgttaaaccaactagaa

SEQ ID NO: 42 - RNA, 34 nt, synthetic construct
  source 1..34: mol_type = other RNA
ataccgttattaacatatgacaactcaattaaac

SEQ ID NO: 43 - RNA, 29 nt, synthetic construct
  source 1..29: mol_type = other RNA
gttattaacatatgacaactcaattaaac

SEQ ID NO: 44 - RNA, 19 nt, synthetic construct
  source 1..19: mol_type = other RNA
tatgacaactcaattaaac

SEQ ID NO: 45 - RNA, 13 nt, synthetic construct
  source 1..13: mol_type = other RNA
attaacatatgac

SEQ ID NO: 46-47 - skipped (2 entries)

SEQ ID NO: 48 - DNA, 34 bp, synthetic construct
  source 1..34: mol_type = other DNA
gtttaattgagttgtcatatgttaataacggtat

SEQ ID NO: 49 - DNA, 29 bp, synthetic construct
  source 1..29: mol_type = other DNA
gtttaattgagttgtcatatgttaataac

SEQ ID NO: 50 - DNA, 19 bp, synthetic construct
  source 1..19: mol_type = other DNA
gtttaattgagttgtcata

SEQ ID NO: 51 - DNA, 20 bp, synthetic construct
  source 1..20: mol_type = other DNA
ggcactgagggtggaggtgg

SEQ ID NO: 52 - DNA, 20 bp, synthetic construct
  source 1..20: mol_type = other DNA
ggcactgcggctggaggtgg

SEQ ID NO: 53 - DNA, 18 bp, synthetic construct
  source 1..18: mol_type = other DNA
ggcactgcctggaggtgg

SEQ ID NO: 54 - DNA, 20 bp, synthetic construct
  source 1..20: mol_type = other DNA
ggcactgcggctggaggtgg

SEQ ID NO: 55 - DNA, 20 bp, synthetic construct
  source 1..20: mol_type = other DNA
ggcactgcggctggaggtgg

SEQ ID NO: 56 - DNA, 18 bp, synthetic construct
  source 1..18: mol_type = other DNA
ggcactggctggaggtgg

SEQ ID NO: 57 - DNA, 22 bp, synthetic construct
  source 1..22: mol_type = other DNA
gtttaattgagttgtcatatgt

SEQ ID NO: 58 - DNA, 22 bp, synthetic construct
  source 1..22: mol_type = other DNA
acatatgacaactcaattaaac

SEQ ID NO: 59 - DNA, 27 bp, synthetic construct
  source 1..27: mol_type = other DNA
ttgagttgtcatatgttaataacggta

SEQ ID NO: 60 - DNA, 27 bp, synthetic construct
  source 1..27: mol_type = other DNA
taccgttattaacatatgacaactcaa

SEQ ID NO: 61 - DNA, 22 bp, synthetic construct
  source 1..22: mol_type = other DNA
ataccgttattaacatatgaca

SEQ ID NO: 62 - DNA, 29 bp, synthetic construct
  source 1..29: mol_type = other DNA
gtttaattgagttgtcatatgttaataac

SEQ ID NO: 63 - DNA, 56 bp, synthetic construct
  source 1..56: mol_type = other DNA
gtgactggagttcagacgtgtgctcttccgatctacatatgacaactcaattaaac

SEQ ID NO: 64 - DNA, 61 bp, synthetic construct
  source 1..61: mol_type = other DNA
gtgactggagttcagacgtgtgctcttccgatctttgagttgtcatatgttaataacggta

SEQ ID NO: 65 - DNA, 58 bp, synthetic construct
  source 1..58: mol_type = other DNA
aatgatacggcgaccaccgagatctacacnnnnnnnnacactctttccctacacgacg

SEQ ID NO: 66 - DNA, 57 bp, synthetic construct
  source 1..57: mol_type = other DNA
caagcagaagacggcatacgagattannnnnnnngactggagttcagacgtgtgctc

SEQ ID NO: 67 - DNA, 20 bp, synthetic construct
  source 1..20: mol_type = other DNA
ctaaatagcgcgaatccgtc

SEQ ID NO: 68 - DNA, 18 bp, synthetic construct
  source 1..18: mol_type = other DNA
tcattttgactcacgcgg

SEQ ID NO: 69 - RNA, 155 nt, synthetic construct
  source 1..155: mol_type = other RNA
ggcactgcggctggaggtgggttttagagctagaaatagcaagttaaaataaggctagtccgttatcaacttgaaaaagtggcaccgagtcggtgcttaaccccaaataccgttattaacatatgacaactcaattaaaccctccagcctttttt

SEQ ID NO: 70 - RNA, 20 nt, synthetic construct
  source 1..20: mol_type = other RNA
ggcactgcggctggaggtgg

SEQ ID NO: 71 - RNA, 10 nt, synthetic construct
  source 1..10: mol_type = other RNA
ttaaccccaa

SEQ ID NO: 72 - RNA, 34 nt, synthetic construct; identical to SEQ ID NO: 42
  source 1..34: mol_type = other RNA

SEQ ID NO: 73 - skipped

SEQ ID NO: 74 - RNA, 158 nt, synthetic construct
  source 1..158: mol_type = other RNA
ggcactgcggctggaggtgggttttagagctagaaatagcaagttaaaataaggctagtccgttatcaacttgaaaaagtggcaccgagtcggtgcttaaccccttacaataccgttattaacatatgacaactcaattaaaccctccagcctttttt

SEQ ID NO: 75 - RNA, 20 nt, synthetic construct
  source 1..20: mol_type = other RNA
ggcactgcggctggaggtgg

SEQ ID NO: 76 - RNA, 13 nt, synthetic construct
  source 1..13: mol_type = other RNA
ttaaccccttaca

SEQ ID NO: 77 - RNA, 34 nt, synthetic construct; identical to SEQ ID NO: 42
  source 1..34: mol_type = other RNA

SEQ ID NO: 78 - skipped

SEQ ID NO: 79 - RNA, 163 nt, synthetic construct
  source 1..163: mol_type = other RNA
catggtgcacctgactcctggttttagagctagaaatagcaagttaaaataaggctagtccgttatcaacttgaaaaagtggcaccgagtcggtgcagacttctccacagataccgttattaacatatgacaactcaattaaacgagtcaggtgcactttttt

SEQ ID NO: 80 - RNA, 20 nt, synthetic construct
  source 1..20: mol_type = other RNA
catggtgcacctgactcctg

SEQ ID NO: 81 - RNA, 14 nt, synthetic construct
  source 1..14: mol_type = other RNA
agacttctccacag

SEQ ID NO: 82 - RNA, 34 nt, synthetic construct; identical to SEQ ID NO: 42
  source 1..34: mol_type = other RNA

SEQ ID NO: 83 - RNA, 13 nt, synthetic construct
  source 1..13: mol_type = other RNA
gagtcaggtgcac

SEQ ID NO: 84 - RNA, 162 nt, synthetic construct
  source 1..162: mol_type = other RNA
ggcccagactgagcacgtgagttttagagctagaaatagcaagttaaaataaggctagtccgttatcaacttgaaaaagtggcaccgagtcggtgctctgccatcaaagataccgttattaacatatgacaactcaattaaaccgtgctcagtctgtttttt

SEQ ID NO: 85 - RNA, 20 nt, synthetic construct
  source 1..20: mol_type = other RNA
ggcccagactgagcacgtga

SEQ ID NO: 86 - RNA, 13 nt, synthetic construct
  source 1..13: mol_type = other RNA
tctgccatcaaag

SEQ ID NO: 87 - RNA, 34 nt, synthetic construct; identical to SEQ ID NO: 42
  source 1..34: mol_type = other RNA

SEQ ID NO: 88 - RNA, 13 nt, synthetic construct
  source 1..13: mol_type = other RNA
cgtgctcagtctg

SEQ ID NO: 89 - RNA, 167 nt, synthetic construct
  source 1..167: mol_type = other RNA
ggaatcccttctgcagcaccgttttagagctagaaatagcaagttaaaataaggctagtccgttatcaacttgaaaaagtggcaccgagtcggtgcggaaaagcgatgcaggtataccgttattaacatatgacaactcaattaaacgctgcagaagggattttttt

SEQ ID NO: 90 - RNA, 20 nt, synthetic construct
  source 1..20: mol_type = other RNA
ggaatcccttctgcagcacc

SEQ ID NO: 91 - RNA, 17 nt, synthetic construct
  source 1..17: mol_type = other RNA
ggaaaagcgatgcaggt

SEQ ID NO: 92 - RNA, 34 nt, synthetic construct; identical to SEQ ID NO: 42
  source 1..34: mol_type = other RNA

SEQ ID NO: 93 - RNA, 14 nt, synthetic construct
  source 1..14: mol_type = other RNA
gctgcagaagggat

SEQ ID NO: 94 - RNA, 164 nt, synthetic construct
  source 1..164: mol_type = other RNA
gagtccgagcagaagaagaagttttagagctagaaatagcaagttaaaataaggctagtccgttatcaacttgaaaaagtggcaccgagtcggtgcatgggagcacttcataccgttattaacatatgacaactcaattaaacttcttctgctcggactttttt

SEQ ID NO: 95 - RNA, 20 nt, synthetic construct
  source 1..20: mol_type = other RNA
gagtccgagcagaagaagaa

SEQ ID NO: 96 - RNA, 13 nt, synthetic construct
  source 1..13: mol_type = other RNA
atgggagcacttc

SEQ ID NO: 97 - RNA, 34 nt, synthetic construct; identical to SEQ ID NO: 42
  source 1..34: mol_type = other RNA

SEQ ID NO: 98 - RNA, 15 nt, synthetic construct
  source 1..15: mol_type = other RNA
ttcttctgctcggac

SEQ ID NO: 99 - RNA, 160 nt, synthetic construct
  source 1..160: mol_type = other RNA
gattcctggtgccagaaacagttttagagctagaaatagcaagttaaaataaggctagtccgttatcaacttgaaaaagtggcaccgagtcggtgcgtcacgcctgtataccgttattaacatatgacaactcaattaaacttctggcaccaggtttttt

SEQ ID NO: 100 - RNA, 20 nt, synthetic construct
  source 1..20: mol_type = other RNA
gattcctggtgccagaaaca

SEQ ID NO: 101 - RNA, 11 nt, synthetic construct
  source 1..11: mol_type = other RNA
gtcacgcctgt

SEQ ID NO: 102 - RNA, 34 nt, synthetic construct; identical to SEQ ID NO: 42
  source 1..34: mol_type = other RNA

SEQ ID NO: 103 - RNA, 13 nt, synthetic construct
  source 1..13: mol_type = other RNA
ttctggcaccagg

SEQ ID NO: 104 - RNA, 166 nt, synthetic construct
  source 1..166: mol_type = other RNA
gcattttcaggaggaagcgagttttagagctagaaatagcaagttaaaataaggctagtccgttatcaacttgaaaaagtggcaccgagtcggtgctgtctgaaggcatcgataccgttattaacatatgacaactcaattaaaccttcctcctgaaaattttttt

SEQ ID NO: 105 - RNA, 20 nt, synthetic construct
  source 1..20: mol_type = other RNA
gcattttcaggaggaagcga

SEQ ID NO: 106 - RNA, 15 nt, synthetic construct
  source 1..15: mol_type = other RNA
tgtctgaaggcatcg

SEQ ID NO: 107 - RNA, 34 nt, synthetic construct; identical to SEQ ID NO: 42
  source 1..34: mol_type = other RNA

SEQ ID NO: 108 - RNA, 15 nt, synthetic construct
  source 1..15: mol_type = other RNA
cttcctcctgaaaat

SEQ ID NO: 109 - RNA, 171 nt, synthetic construct
  source 1..171: mol_type = other RNA
gatgtctgcaggccagatgagttttagagctagaaatagcaagttaaaataaggctagtccgttatcaacttgaaaaagtggcaccgagtcggtgcaatgtgccatctggagcactcaataccgttattaacatatgacaactcaattaaactctggcctgcagatttttt

SEQ ID NO: 110 - RNA, 20 nt, synthetic construct
  source 1..20: mol_type = other RNA
gatgtctgcaggccagatga

SEQ ID NO: 111 - RNA, 22 nt, synthetic construct
  source 1..22: mol_type = other RNA
aatgtgccatctggagcactca

SEQ ID NO: 112 - RNA, 34 nt, synthetic construct; identical to SEQ ID NO: 42
  source 1..34: mol_type = other RNA

SEQ ID NO: 113 - RNA, 13 nt, synthetic construct
  source 1..13: mol_type = other RNA
tctggcctgcaga

SEQ ID NO: 114 - RNA, 165 nt, synthetic construct
  source 1..165: mol_type = other RNA
gtcatcttagtcattacctggttttagagctagaaatagcaagttaaaataaggctagtccgttatcaacttgaaaaagtggcaccgagtcggtgcaacgaacaccgcagataccgttattaacatatgacaactcaattaaacgtaatgactaagatgtttttt

SEQ ID NO: 115 - RNA, 20 nt, synthetic construct
  source 1..20: mol_type = other RNA
gtcatcttagtcattacctg

SEQ ID NO: 116 - RNA, 14 nt, synthetic construct
  source 1..14: mol_type = other RNA
aacgaacaccgcag

SEQ ID NO: 117 - RNA, 34 nt, synthetic construct; identical to SEQ ID NO: 42
  source 1..34: mol_type = other RNA

SEQ ID NO: 118 - RNA, 15 nt, synthetic construct
  source 1..15: mol_type = other RNA
gtaatgactaagatg

SEQ ID NO: 119 - RNA, 200 nt, synthetic construct
  source 1..200: mol_type = other RNA
ggcactgcggctggaggtgggttttagagctagaaatagcaagttaaaataaggctagtccgttatcaacttgaaaaagtggcaccgagtcggtgcttaaccccaaataccgttattaacatatgacaactcaattaaaccctccagccatcttaaccgcggttctatctagttacgcgttaaaccaactagaatttttt

SEQ ID NO: 120 - skipped

SEQ ID NO: 121 - RNA, 37 nt, synthetic construct; identical to SEQ ID NO: 41
  source 1..37: mol_type = other RNA

SEQ ID NO: 122 - RNA, 208 nt, synthetic construct
  source 1..208: mol_type = other RNA
catggtgcacctgactcctggttttagagctagaaatagcaagttaaaataaggctagtccgttatcaacttgaaaaagtggcaccgagtcggtgcagacttctccacagataccgttattaacatatgacaactcaattaaacgagtcaggtgcacaaataaagcgcggttctatctagttacgcgttaaaccaactagaatttttt

SEQ ID NO: 123 - skipped

SEQ ID NO: 124 - RNA, 37 nt, synthetic construct; identical to SEQ ID NO: 41
  source 1..37: mol_type = other RNA

SEQ ID NO: 125 - RNA, 207 nt, synthetic construct
  source 1..207: mol_type = other RNA
ggcccagactgagcacgtgagttttagagctagaaatagcaagttaaaataaggctagtccgttatcaacttgaaaaagtggcaccgagtcggtgctctgccatcaaagataccgttattaacatatgacaactcaattaaaccgtgctcagtctgttaaacttcgcggttctatctagttacgcgttaaaccaactagaatttttt

SEQ ID NO: 126 - skipped

SEQ ID NO: 127 - RNA, 37 nt, synthetic construct; identical to SEQ ID NO: 41
  source 1..37: mol_type = other RNA

SEQ ID NO: 128 - RNA, 212 nt, synthetic construct
  source 1..212: mol_type = other RNA
ggaatcccttctgcagcaccgttttagagctagaaatagcaagttaaaataaggctagtccgttatcaacttgaaaaagtggcaccgagtcggtgcggaaaagcgatgcaggtataccgttattaacatatgacaactcaattaaacgctgcagaagggatatagaacgcgcggttctatctagttacgcgttaaaccaactagaatttttt

SEQ ID NO: 129 - skipped

SEQ ID NO: 130 - RNA, 37 nt, synthetic construct; identical to SEQ ID NO: 41
  source 1..37: mol_type = other RNA

SEQ ID NO: 131 - RNA, 209 nt, synthetic construct
  source 1..209: mol_type = other RNA
gagtccgagcagaagaagaagttttagagctagaaatagcaagttaaaataaggctagtccgttatcaacttgaaaaagtggcaccgagtcggtgcatgggagcacttcataccgttattaacatatgacaactcaattaaacttcttctgctcggacaatattaccgcggttctatctagttacgcgttaaaccaactagaatttttt

SEQ ID NO: 132 - skipped

SEQ ID NO: 133 - RNA, 37 nt, synthetic construct; identical to SEQ ID NO: 41
  source 1..37: mol_type = other RNA

SEQ ID NO: 134 - RNA, 205 nt, synthetic construct
  source 1..205: mol_type = other RNA
gattcctggtgccagaaacagttttagagctagaaatagcaagttaaaataaggctagtccgttatcaacttgaaaaagtggcaccgagtcggtgcgtcacgcctgtataccgttattaacatatgacaactcaattaaacttctggcaccaggctaactaccgcggttctatctagttacgcgttaaaccaactagaatttttt

SEQ ID NO: 135 - skipped

SEQ ID NO: 136 - RNA, 37 nt, synthetic construct; identical to SEQ ID NO: 41
  source 1..37: mol_type = other RNA

SEQ ID NO: 137 - RNA, 211 nt, synthetic construct
  source 1..211: mol_type = other RNA
gcattttcaggaggaagcgagttttagagctagaaatagcaagttaaaataaggctagtccgttatcaacttgaaaaagtggcaccgagtcggtgctgtctgaaggcatcgataccgttattaacatatgacaactcaattaaaccttcctcctgaaaatatcctacccgcggttctatctagttacgcgttaaaccaactagaatttttt

SEQ ID NO: 138 - skipped

SEQ ID NO: 139 - RNA, 37 nt, synthetic construct; identical to SEQ ID NO: 41
  source 1..37: mol_type = other RNA

SEQ ID NO: 140 - RNA, 216 nt, synthetic construct
  source 1..216: mol_type = other RNA
gatgtctgcaggccagatgagttttagagctagaaatagcaagttaaaataaggctagtccgttatcaacttgaaaaagtggcaccgagtcggtgcaatgtgccatctggagcactcaataccgttattaacatatgacaactcaattaaactctggcctgcagaaagaaaggcgcggttctatctagttacgcgttaaaccaactagaatttttt

SEQ ID NO: 141 - skipped

SEQ ID NO: 142 - RNA, 37 nt, synthetic construct; identical to SEQ ID NO: 41
  source 1..37: mol_type = other RNA

SEQ ID NO: 143 - RNA, 210 nt, synthetic construct
  source 1..210: mol_type = other RNA
gtcatcttagtcattacctggttttagagctagaaatagcaagttaaaataaggctagtccgttatcaacttgaaaaagtggcaccgagtcggtgcaacgaacaccgcagataccgttattaacatatgacaactcaattaaacgtaatgactaagatgtaatataccgcggttctatctagttacgcgttaaaccaactagaatttttt

SEQ ID NO: 144 - skipped

SEQ ID NO: 145 - RNA, 37 nt, synthetic construct; identical to SEQ ID NO: 41
  source 1..37: mol_type = other RNA

SEQ ID NO: 146 - DNA, 3611 bp, synthetic construct
  source 1..3611: mol_type = other DNA
gacgaagactcaattgtcgattagtgaacggatctcgacggtatcgatcacgagactagcctcgagcggccgcccccttcaccgagggcctatttcccatgattccttcatatttgcatatacgatacaaggctgttagagagataattggaattaatttgactgtaaacacaaagatattagtacaaaatacgtgacgtagaaagtaataatttcttgggtagtttgcagttttaaaattatgttttaaaatggactatcatatgcttaccgtaacttgaaagtatttcgatttcttggctttatatatcttgtggaaaggacgaaacaccggagaccacatttccccgaaaagtgccacctgacgtctaagaaaccattattatcatgacattaacctataaaaataggcgtatcacgaggccctttcgtctcgcgcgtttcggtgatgacggtgaaaacctctgacacatgcagctcccggagacggtcacagcttgtctgtaagcggatgccgggagcagacaagcccgtcagggcgcgtcagcgggtgttggcgggtgtcggggctggcttaactatgcggcatcagagcagattgtactgagagtgcaccatatgcggtgtgaaataccgcacagatgcgtaaggagaaaataccgcatcaggcgccattcgccattcaggctgcgcaactgttgggaagggcgatcggtgcgggcctcttcgctattacgccagctggcgaaagggggatgtgctgcaaggcgattaagttgggtaacgccagggttttcccagtcacgacgttgtaaaacgacggccagtgccaagcttgcatgcctgcaggtcgactctagaggatccccgggtaccgagctcgaattcgtaatcatggtcatagctgtttcctgtgtgaaattgttatccgctcacaattccacacaacatacgagccggaagcataaagtgtaaagcctggggtgcctaatagatccggtctccgttttagagctagaaatagcaagttaaaataaggctagtccgttatcaacttgaaaaagtggcaccgagtcggtgcggagacgtgtctgtaagcggatgccgggagcagacaagcccgtcagggcgcgtcagcgggtgttggcgggtgtcggggctggcttaactatgcggcatcagagcagattgtactgagagtgcaccatatgcggtgtgaaataccgcacagatgcgtaaggagaaaataccgcatcaggcgccattcgccattcaggctgcgcaactgttgggaagggcgatcggtgcgggcctcttcgctattacgccagctggcgaaagggggatgtgctgcaaggcgattaagttgggtaacgccagggttttcccagtcacgacgttgtaaaacgacggccagtgccaagcttgcatgcctgcaggtcgactctagaggatccccgggtaccgagctcgaattcgtaatcatggtcatagctgtttcctgtgtgaaattgttatccgctcacaattccacacaacatacgagccggcgtctccctagattcgcgatgtacgggccagatatacgcgttgacattgattattgactagttgtcttcctgcattaatgaatcggccaacgcgcggggagaggcggtttgcgtattgggcgctcttccgcttcctcgctcactgactcgctgcgctcggtcgttcggctgcggcgagcggtatcagctcactcaaaggcggtaatacggttatccacagaatcaggggataacgcaggaaagaacatgtgagcaaaaggccagcaaaaggccaggaaccgtaaaaaggccgcgttgctggcgtttttccataggctccgcccccctgacgagcatcacaaaaatcgacgctcaagtcagaggtggcgaaacccgacaggactataaagataccaggcgtttccccctggaagctccctcgtgcgctctcctgttccgaccctgccgcttaccggatacctgtccgcctttctcccttcgggaagcgtggcgctttctcaatgctcacgctgtaggtatctcagttcggtgtaggtcgttcgctccaagctgggctgtgtgcacgaaccccccgttcagcccgaccgctgcgccttatccggtaactatcgtcttgagtccaacccggtaagacacgacttatcgccactggcagcagccactggtaacaggattagcagagcgaggtatgtaggcggtgctacagagttcttgaagtggtggcctaactacggctacactagaaggacagtatttggtatctgcgctctgctgaagccagttaccttcggaaaaagagttggtagctcttgatccggcaaacaaaccaccgctggtagcggtggtttttttgtttgcaagcagcagattacgcgcagaaaaaaaggatctcaagaagatcctttgatcttttctacggggtctgacgctcagtggaacgaaaactcacgttaagggattttggtcatgagattatcaaaaaggatcttcacctagatccttttaaattaaaaatgaagttttaaatcaatctaaagtatatatgagtaaacttggtctgacagttaccaatgcttaatcagtgaggcacctatctcagcgatctgtctatttcgttcatccatagttgcctgactccccgtcgtgtagataactacgatacgggagggcttaccatctggccccagtgctgcaatgataccgcgagatccacgctcaccggctccagatttatcagcaataaaccagccagccggaagggccgagcgcagaagtggtcctgcaactttatccgcctccatccagtctattaattgttgccgggaagctagagtaagtagttcgccagttaatagtttgcgcaacgttgttgccattgctacaggcatcgtggtgtcacgctcgtcgtttggtatggcttcattcagctccggttcccaacgatcaaggcgagttacatgatcccccatgttgtgcaaaaaagcggttagctccttcggtcctccgatcgttgtcagaagtaagttggccgcagtgttatcactcatggttatggcagcactgcataattctcttactgtcatgccatccgtaagatgcttttctgtgactggtgagtactcaaccaagtcattctgagaatagtgtatgcggcgaccgagttgctcttgcccggcgtcaatacgggataataccgcgccacatagcagaactttaaaagtgctcatcattggaaaacgttcttcggggcgaaaactctcaaggatcttaccgctgttgagatccagttcgatgtaacccactcgtgcacccaactgatcttcagcatcttttactttcaccagcgtttctgggtgagcaaaaacaggaaggcaaaatgccgcaaaaaagggaataagggcgacacggaaatgttgaatactcatactcttcctttttcaatattattgaagcatttatcagggttattgtctcatgagcggatacatatttgaatgtatttagaaaaataaacaaataggggttccgcgcacatttccccgaaaagtgccacctgacgtc

SEQ ID NO: 147 - DNA, 12606 bp, synthetic construct
  source 1..12606: mol_type = other DNA
cgatgtacgggccagatatacgcgcgtatatctggcccgtacatcgcgaatctagaaaaaannnnnnnnnnnnnnnnnnnnnnnnnnnnngcaccgactcggtgccactttttcaagttgataacggactagccttattttaacttgctatttctagctctaaaacnnnnnnnnnnnnnnnnnnncggtgtttcgtcctttccacaagatatataaagccaagaaatcgaaatactttcaagttacggtaagcatatgatagtccattttaaaacataattttaaaactgcaaactacccaagaaattattactttctacgtcacgtattttgtactaatatctttgtgtttacagtcaaattaattccaattatctctctaacagccttgtatcgtatatgcaaatatgaaggaatcatgggaaataggccctccgcgttgacattgattattgactagttattaatagtaatcaattacggggtcattagttcatagcccatatatggagttccgcgttacataacttacggtaaatggcccgcctggctgaccgcccaacgacccccgcccattgacgtcaataatgacgtatgttcccatagtaacgccaatagggactttccattgacgtcaatgggtggagtatttacggtaaactgcccacttggcagtacatcaagtgtatcatatgccaagtacgccccctattgacgtcaatgacggtaaatggcccgcctggcattatgcccagtacatgaccttatgggactttcctacttggcagtacatctacgtattagtcatcgctattaccatggtgatgcggttttggcagtacatcaatgggcgtggatagcggtttgactcacggggatttccaagtctccaccccattgacgtcaatgggagtttgttttggcaccaaaatcaacgggactttccaaaatgtcgtaacaactccgccccattgacgcaaatgggcggtaggcgtgtacggtgggaggtctatataagcagagctggtttagtgaaccgtcagatccgctagagatccgcggccgctaatacgactcactatagggagagccgccaccatgaaacggacagccgacggaagcgagttcgagtcaccaaagaagaagcggaaagtcgacaagaagtacagcatcggcctggacatcggcaccaactctgtgggctgggccgtgatcaccgacgagtacaaggtgcccagcaagaaattcaaggtgctgggcaacaccgaccggcacagcatcaagaagaacctgatcggagccctgctgttcgacagcggcgaaacagccgaggccacccggctgaagagaaccgccagaagaagatacaccagacggaagaaccggatctgctatctgcaagagatcttcagcaacgagatggccaaggtggacgacagcttcttccacagactggaagagtccttcctggtggaagaggataagaagcacgagcggcaccccatcttcggcaacatcgtggacgaggtggcctaccacgagaagtaccccaccatctaccacctgagaaagaaactggtggacagcaccgacaaggccgacctgcggctgatctatctggccctggcccacatgatcaagttccggggccacttcctgatcgagggcgacctgaaccccgacaacagcgacgtggacaagctgttcatccagctggtgcagacctacaaccagctgttcgaggaaaaccccatcaacgccagcggcgtggacgccaaggccatcctgtctgccagactgagcaagagcagacggctggaaaatctgatcgcccagctgcccggcgagaagaagaatggcctgttcggaaacctgattgccctgagcctgggcctgacccccaacttcaagagcaacttcgacctggccgaggatgccaaactgcagctgagcaaggacacctacgacgacgacctggacaacctgctggcccagatcggcgaccagtacgccgacctgtttctggccgccaagaacctgtccgacgccatcctgctgagcgacatcctgagagtgaacaccgagatcaccaaggcccccctgagcgcctctatgatcaagagatacgacgagcaccaccaggacctgaccctgctgaaagctctcgtgcggcagcagctgcctgagaagtacaaagagattttcttcgaccagagcaagaacggctacgccggctacattgacggcggagccagccaggaagagttctacaagttcatcaagcccatcctggaaaagatggacggcaccgaggaactgctcgtgaagctgaacagagaggacctgctgcggaagcagcggaccttcgacaacggcagcatcccccaccagatccacctgggagagctgcacgccattctgcggcggcaggaagatttttacccattcctgaaggacaaccgggaaaagatcgagaagatcctgaccttccgcatcccctactacgtgggccctctggccaggggaaacagcagattcgcctggatgaccagaaagagcgaggaaaccatcaccccctggaacttcgaggaagtggtggacaagggcgcttccgcccagagcttcatcgagcggatgaccaacttcgataagaacctgcccaacgagaaggtgctgcccaagcacagcctgctgtacgagtacttcaccgtgtataacgagctgaccaaagtgaaatacgtgaccgagggaatgagaaagcccgccttcctgagcggcgagcagaaaaaggccatcgtggacctgctgttcaagaccaaccggaaagtgaccgtgaagcagctgaaagaggactacttcaagaaaatcgagtgcttcgactccgtggaaatctccggcgtggaagatcggttcaacgcctccctgggcacataccacgatctgctgaaaattatcaaggacaaggacttcctggacaatgaggaaaacgaggacattctggaagatatcgtgctgaccctgacactgtttgaggacagagagatgatcgaggaacggctgaaaacctatgcccacctgttcgacgacaaagtgatgaagcagctgaagcggcggagatacaccggctggggcaggctgagccggaagctgatcaacggcatccgggacaagcagtccggcaagacaatcctggatttcctgaagtccgacggcttcgccaacagaaacttcatgcagctgatccacgacgacagcctgacctttaaagaggacatccagaaagcccaggtgtccggccagggcgatagcctgcacgagcacattgccaatctggccggcagccccgccattaagaagggcatcctgcagacagtgaaggtggtggacgagctcgtgaaagtgatgggccggcacaagcccgagaacatcgtgatcgaaatggccagagagaaccagaccacccagaagggacagaagaacagccgcgagagaatgaagcggatcgaagagggcatcaaagagctgggcagccagatcctgaaagaacaccccgtggaaaacacccagctgcagaacgagaagctgtacctgtactacctgcagaatgggcgggatatgtacgtggaccaggaactggacatcaaccggctgtccgactacgatgtggacgctatcgtgcctcagagctttctgaaggacgactccatcgacaacaaggtgctgaccagaagcgacaagaaccggggcaagagcgacaacgtgccctccgaagaggtcgtgaagaagatgaagaactactggcggcagctgctgaacgccaagctgattacccagagaaagttcgacaatctgaccaaggccgagagaggcggcctgagcgaactggataaggccggcttcatcaagagacagctggtggaaacccggcagatcacaaagcacgtggcacagatcctggactcccggatgaacactaagtacgacgagaatgacaagctgatccgggaagtgaaagtgatcaccctgaagtccaagctggtgtccgatttccggaaggatttccagttttacaaagtgcgcgagatcaacaactaccaccacgcccacgacgcctacctgaacgccgtcgtgggaaccgccctgatcaaaaagtaccctaagctggaaagcgagttcgtgtacggcgactacaaggtgtacgacgtgcggaagatgatcgccaagagcgagcaggaaatcggcaaggctaccgccaagtacttcttctacagcaacatcatgaactttttcaagaccgagattaccctggccaacggcgagatccggaagcggcctctgatcgagacaaacggcgaaaccggggagatcgtgtgggataagggccgggattttgccaccgtgcggaaagtgctgagcatgccccaagtgaatatcgtgaaaaagaccgaggtgcagacaggcggcttcagcaaagagtctatcctgcccaagaggaacagcgataagctgatcgccagaaagaaggactgggaccctaagaagtacggcggcttcgacagccccaccgtggcctattctgtgctggtggtggccaaagtggaaaagggcaagtccaagaaactgaagagtgtgaaagagctgctggggatcaccatcatggaaagaagcagcttcgagaagaatcccatcgactttctggaagccaagggctacaaagaagtgaaaaaggacctgatcatcaagctgcctaagtactccctgttcgagctggaaaacggccggaagagaatgctggcctctgccggcgaactgcagaagggaaacgaactggccctgccctccaaatatgtgaacttcctgtacctggccagccactatgagaagctgaagggctcccccgaggataatgagcagaaacagctgtttgtggaacagcacaagcactacctggacgagatcatcgagcagatcagcgagttctccaagagagtgatcctggccgacgctaatctggacaaagtgctgtccgcctacaacaagcaccgggataagcccatcagagagcaggccgagaatatcatccacctgtttaccctgaccaatctgggagcccctgccgccttcaagtactttgacaccaccatcgaccggaagaggtacaccagcaccaaagaggtgctggacgccaccctgatccaccagagcatcaccggcctgtacgagacacggatcgacctgtctcagctgggaggtgactctggaggatctagcggaggatcctctggcagcgagacaccaggaacaagcgagtcagcaacaccagagagcagtggcggcagcagcggcggcagcagcaccctaaatatagaagatgagtatcggctacatgagacctcaaaagagccagatgtttctctagggtccacatggctgtctgattttcctcaggcctgggcggaaaccgggggcatgggactggcagttcgccaagctcctctgatcatacctctgaaagcaacctctacccccgtgtccataaaacaataccccatgtcacaagaagccagactggggatcaagccccacatacagagactgttggaccagggaatactggtaccctgccagtccccctggaacacgcccctgctacccgttaagaaaccagggactaatgattataggcctgtccaggatctgagagaagtcaacaagcgggtggaagacatccaccccaccgtgcccaacccttacaacctcttgagcgggctcccaccgtcccaccagtggtacactgtgcttgatttaaaggatgcctttttctgcctgagactccaccccaccagtcagcctctcttcgcctttgagtggagagatccagagatgggaatctcaggacaattgacctggaccagactcccacagggtttcaaaaacagtcccaccctgtttaatgaggcactgcacagagacctagcagacttccggatccagcacccagacttgatcctgctacagtacgtggatgacttactgctggccgccacttctgagctagactgccaacaaggtactcgggccctgttacaaaccctagggaacctcgggtatcgggcctcggccaagaaagcccaaatttgccagaaacaggtcaagtatctggggtatcttctaaaagagggtcagagatggctgactgaggccagaaaagagactgtgatggggcagcctactccgaagacccctcgacaactaagggagttcctagggaaggcaggcttctgtcgcctcttcatccctgggtttgcagaaatggcagcccccctgtaccctctcaccaaaccggggactctgtttaattggggcccagaccaacaaaaggcctatcaagaaatcaagcaagctcttctaactgccccagccctggggttgccagatttgactaagccctttgaactctttgtcgacgagaagcagggctacgccaaaggtgtcctaacgcaaaaactgggaccttggcgtcggccggtggcctacctgtccaaaaagctagacccagtagcagctgggtggcccccttgcctacggatggtagcagccattgccgtactgacaaaggatgcaggcaagctaaccatgggacagccactagtcattctggccccccatgcagtagaggcactagtcaaacaaccccccgaccgctggctttccaacgcccggatgactcactatcaggccttgcttttggacacggaccgggtccagttcggaccggtggtagccctgaacccggctacgctgctcccactgcctgaggaagggctgcaacacaactgccttgatatcctggccgaagcccacggaacccgacccgacctaacggaccagccgctcccagacgccgaccacacctggtacacggatggaagcagtctcttacaagagggacagcgtaaggcgggagctgcggtgaccaccgagaccgaggtaatctgggctaaagccctgccagccgggacatccgctcagcgggctgaactgatagcactcacccaggccctaaagatggcagaaggtaagaagctaaatgtttatactgatagccgttatgcttttgctactgcccatatccatggagaaatatacagaaggcgtgggtggctcacatcagaaggcaaagagatcaaaaataaagacgagatcttggccctactaaaagccctctttctgcccaaaagacttagcataatccattgtccaggacatcaaaagggacacagcgccgaggctagaggcaaccggatggctgaccaagcggcccgaaaggcagccatcacagagactccagacacctctaccctcctcatagaaaattcatcaccctctggcggctcaaaaagaaccgccgacggcagcgaattcgagcccaagaagaagaggaaagtctaaccggtcatcatcaccatcaccattgagttttacccctacgacgtgcccgactacgcctaataactcgagcatgcatctagagggccctattctatagtgtcacctaaatgctagagctcgctgatcagcctcgactgtgccttctagttgccagccatctgttgtttgcccctcccccgtgccttccttgaccctggaaggtgccactcccactgtcctttcctaataaaatgaggaaattgcatcgcattgtctgagtaggtgtcattctattctggggggtggggtggggcaggacagcaagggggaggattgggaagacaatagcaggcatgctggggaggatctgcgatcgctccggtgcccgtcagtgggcagagcgcacatcgcccacagtccccgagaagttggggggaggggtcggcaattgaacgggtgcctagagaaggtggcgcggggtaaactgggaaagtgatgtcgtgtactggctccgcctttttcccgagggtgggggagaaccgtatataagtgcagtagtcgccgtgaacgttctttttcgcaacgggtttgccgccagaacacagctgaagcttcgaggggctcgcatctctccttcacgcgcccgccgccctacctgaggccgccatccacgccggttgagtcgcgttctgccgcctcccgcctgtggtgcctcctgaactgcgtccgccgtctaggtaagtttaaagctcaggtcgagaccgggcctttgtccggcgctcccttggagcctacctagactcagccggctctccacgctttgcctgaccctgcttgctcaactctacgtctttgtttcgttttctgttctgcgccgttacagatccaagctgtgaccggcgcctacatgaccgagtacaagcccacggtgcgcctcgccacccgcgacgacgtccccagggccgtacgcaccctcgccgccgcgttcgccgactaccccgccacgcgccacaccgtcgatccagaccgccacatcgagcgggtcaccgagctgcaagaactcttcctcacgcgcgtcgggctcgacatcggcaaggtgtgggtcgcggacgacggcgccgcggtggcggtctggaccacgccggagagcgtcgaagcgggggcggtgttcgccgagatcggcccgcgcatggccgagttgagcggttcccggctggccgcgcagcaacagatggaaggtctcctggcgccgcaccggcccaaggagcccgcgtggttcctggccaccgtcggcgtctcgcccgaccaccagggcaagggtctgggcagcgccgtcgtgctccccggagtggaggcggccgagcgcgccggggtgcccgccttcctggagacctccgcgccccgcaacctccccttctacgagcggctcggcttcaccgtcaccgccgacgtcgaggtgcccgaaggaccgcgcacctggtgcatgacccgcaagcccggtgcctgagctagaagctcgctttcttgctgtccaatttctattaaaggttcctttgttccctaagtccaactactaaactgggggatattatgaagggccttgagcatctggattctgcctaataaaaaacatttattttcattgcaatgatgtatttaaattatttctgaatattttactaaaaagggaatgtgggaggtcagtgcatttaaaacataaagaaatgaagagctagttcaaaccttgggaaaatacactatatcttaaactccatgaaagaaggtgaggctgcaaacagctaatgcacattggcaacagcccctgatgcctatgccttattcatccctcagaaaaggattcaagtagaggcttgatttggaggttaaagttttgctatgctgtattttagaattccataccacatttgtagaggttttacttgctttaaaaaacctcccacacctccccctgaacctgaaacataaaatgaatgcaattgttgttgttttaccaatgcttaatcagtgaggcacctatctcagcgatctgtctatttcgttcatccatagttgcctgactccccgtcgtgtagataactacgatacgggagggcttaccatctggccccagtgctgcaatgataccgcgagacccacgctcaccggctccagatttatcagcaataaaccagccagccggaagggccgagcgcagaagtggtcctgcaactttatccgcctccatccagtctattaattgttgccgggaagctagagtaagtagttcgccagttaatagtttgcgcaacgttgttgccattgctacaggcatcgtggtgtcacgctcgtcgtttggtatggcttcattcagctccggttcccaacgatcaaggcgagttacatgatcccccatgttgtgcaaaaaagcggttagctccttcggtcctccgatcgttgtcagaagtaagttggccgcagtgttatcactcatggttatggcagcactgcataattctcttactgtcatgccatccgtaagatgcttttctgtgactggtgagtactcaaccaagtcattctgagaatagtgtatgcggcgaccgagttgctcttgcccggcgtcaatacgggataataccgcgccacatagcagaactttaaaagtgctcatcattggaaaacgttcttcggggcgaaaactctcaaggatcttaccgctgttgagatccagttcgatgtaacccactcgtgcacccaactgatcttcagcatcttttactttcaccagcgtttctgggtgagcaaaaacaggaaggcaaaatgccgcaaaaaagggaataagggcgacacggaaatgttgaatactcatactcttcctttttcaatattattgaagcatttatcagggttattgtctcatgagcggatacatatttgaatgtatttagaaaaataaacaaataggggttccgcgaacttgtttattgcagcttataatggttacaaataaagcaatagcatcacaaatttcacaaataaagcatttttttcactgcattctagttgtggtttgtccaaactcatcaatgtatcttatcatgtctggccagctagccaacaagctcgtcatcgctttgcagaagagcagagaggatatgctcatcgtctaaagaactacccattttattatatattagtcacgatatctataacaagaaaatatatatataataagttatcacgtaagtagaacatgaaataacaatataattatcgtatgagttaaatcttaaaagtcacgtaaaagataatcatgcgtcattttgactcacgcggtcgttatagttcaaaatcagtgacacttaccgcattgacaagcacgcctcacgggagctccaagcggcgactgagatgtcctaaatgcacagcgacggattcgcgctatttagaaagagagagcaatatttcaagaatgcatgcgtcaattttacgcagactatctttctagggttaaaaaagatttgcgctttactcgacctaaactttaaacacgtcatagaatcttcgtttgacaaaaaccacattgtggccaagctgtgtgacgcgacgcgcgctaaagaatggcaaaccaagtcgcgcgaggtacccagcttttgttccctttagtgagggttaattccgagcttggcgtaatcatggtcatagctgtttcctgtgtgaaattgttatccgctcacaattccacacaacatacgagccggaagcataaagtgtaaagcctggggtgcctaatgagtgagctaactcacattaattgcgttgcgctcactgcccgctttccagtcgggaaacctgtcgtgccagctgcattaatgaatcggccaacgcgcggggagaggcggtttgcgtattgggcgctcttccgcttcctcgctcactgactcgctgcgctcggtcgttcggctgcggcgagcggtatcagctcactcaaaggcggtaatacggttatccacagaatcaggggataacgcaggaaagaacatgtgagcaaaaggccagcaaaaggccaggaaccgtaaaaaggccgcgttgctggcgtttttccataggctccgcccccctgacgagcatcacaaaaatcgacgctcaagtcagaggtggcgaaacccgacaggactataaagataccaggcgtttccccctggaagctccctcgtgcgctctcctgttccgaccctgccgcttaccggatacctgtccgcctttctcccttcgggaagcgtggcgctttctcatagctcacgctgtaggtatctcagttcggtgtaggtcgttcgctccaagctgggctgtgtgcacgaaccccccgttcagcccgaccgctgcgccttatccggtaactatcgtcttgagtccaacccggtaagacacgacttatcgccactggcagcagccactggtaacaggattagcagagcgaggtatgtaggcggtgctacagagttcttgaagtggtggcctaactacggctacactagaaggacagtatttggtatctgcgctctgctgaagccagttaccttcggaaaaagagttggtagctcttgatccggcaaacaaaccaccgctggtagcggtggtttttttgtttgcaagcagcagattacgcgcagaaaaaaaggatctcaagaagatcctttgatcttttctacggggtctgacgctcagtggaacgaaaactcacgttaagggattttggtcatgattaaccctagaaagataatcatattgtgacgtacgttaaagataatcatgcgtaaaattgacgcatgtgttttatcggtctgtatatcgaggtttatttattaatttgaatagatattaagttttattatatttacacttacatactaataataaattcaacaaacaatttatttatgtttatttatttattaaaaaaaaacaaaaactcaaaatttcttctataaagtaacaaaacttttaaacattctctcttttacaaaaataaacttattttgtactttaaaaacagtcatgttgtattataaaataagtaattagcttaacctatacataatagaaacaaattatacttattagtcagtcagaaacaactttggcacatatcaatattatgctctcgttaattaa

SEQ ID NO: 148 - DNA, 12191 bp, synthetic construct
  source 1..12191: mol_type = other DNA
cgatgtacgggccagatatacgcgttgacattgattattgactagttattaatagtaatcaattacggggtcattagttcatagcccatatatggagttccgcgttacataacttacggtaaatggcccgcctggctgaccgcccaacgacccccgcccattgacgtcaataatgacgtatgttcccatagtaacgccaatagggactttccattgacgtcaatgggtggagtatttacggtaaactgcccacttggcagtacatcaagtgtatcatatgccaagtacgccccctattgacgtcaatgacggtaaatggcccgcctggcattatgcccagtacatgaccttatgggactttcctacttggcagtacatctacgtattagtcatcgctattaccatggtgatgcggttttggcagtacatcaatgggcgtggatagcggtttgactcacggggatttccaagtctccaccccattgacgtcaatgggagtttgttttggcaccaaaatcaacgggactttccaaaatgtcgtaacaactccgccccattgacgcaaatgggcggtaggcgtgtacggtgggaggtctatataagcagagctggtttagtgaaccgtcagatccgctagagatccgcggccgctaatacgactcactatagggagagccgccaccatgaaacggacagccgacggaagcgagttcgagtcaccaaagaagaagcggaaagtcgacaagaagtacagcatcggcctggacatcggcaccaactctgtgggctgggccgtgatcaccgacgagtacaaggtgcccagcaagaaattcaaggtgctgggcaacaccgaccggcacagcatcaagaagaacctgatcggagccctgctgttcgacagcggcgaaacagccgaggccacccggctgaagagaaccgccagaagaagatacaccagacggaagaaccggatctgctatctgcaagagatcttcagcaacgagatggccaaggtggacgacagcttcttccacagactggaagagtccttcctggtggaagaggataagaagcacgagcggcaccccatcttcggcaacatcgtggacgaggtggcctaccacgagaagtaccccaccatctaccacctgagaaagaaactggtggacagcaccgacaaggccgacctgcggctgatctatctggccctggcccacatgatcaagttccggggccacttcctgatcgagggcgacctgaaccccgacaacagcgacgtggacaagctgttcatccagctggtgcagacctacaaccagctgttcgaggaaaaccccatcaacgccagcggcgtggacgccaaggccatcctgtctgccagactgagcaagagcagacggctggaaaatctgatcgcccagctgcccggcgagaagaagaatggcctgttcggaaacctgattgccctgagcctgggcctgacccccaacttcaagagcaacttcgacctggccgaggatgccaaactgcagctgagcaaggacacctacgacgacgacctggacaacctgctggcccagatcggcgaccagtacgccgacctgtttctggccgccaagaacctgtccgacgccatcctgctgagcgacatcctgagagtgaacaccgagatcaccaaggcccccctgagcgcctctatgatcaagagatacgacgagcaccaccaggacctgaccctgctgaaagctctcgtgcggcagcagctgcctgagaagtacaaagagattttcttcgaccagagcaagaacggctacgccggctacattgacggcggagccagccaggaagagttctacaagttcatcaagcccatcctggaaaagatggacggcaccgaggaactgctcgtgaagctgaacagagaggacctgctgcggaagcagcggaccttcgacaacggcagcatcccccaccagatccacctgggagagctgcacgccattctgcggcggcaggaagatttttacccattcctgaaggacaaccgggaaaagatcgagaagatcctgaccttccgcatcccctactacgtgggccctctggccaggggaaacagcagattcgcctggatgaccagaaagagcgaggaaaccatcaccccctggaacttcgaggaagtggtggacaagggcgcttccgcccagagcttcatcgagcggatgaccaacttcgataagaacctgcccaacgagaaggtgctgcccaagcacagcctgctgtacgagtacttcaccgtgtataacgagctgaccaaagtgaaatacgtgaccgagggaatgagaaagcccgccttcctgagcggcgagcagaaaaaggccatcgtggacctgctgttcaagaccaaccggaaagtgaccgtgaagcagctgaaagaggactacttcaagaaaatcgagtgcttcgactccgtggaaatctccggcgtggaagatcggttcaacgcctccctgggcacataccacgatctgctgaaaattatcaaggacaaggacttcctggacaatgaggaaaacgaggacattctggaagatatcgtgctgaccctgacactgtttgaggacagagagatgatcgaggaacggctgaaaacctatgcccacctgttcgacgacaaagtgatgaagcagctgaagcggcggagatacaccggctggggcaggctgagccggaagctgatcaacggcatccgggacaagcagtccggcaagacaatcctggatttcctgaagtccgacggcttcgccaacagaaacttcatgcagctgatccacgacgacagcctgacctttaaagaggacatccagaaagcccaggtgtccggccagggcgatagcctgcacgagcacattgccaatctggccggcagccccgccattaagaagggcatcctgcagacagtgaaggtggtggacgagctcgtgaaagtgatgggccggcacaagcccgagaacatcgtgatcgaaatggccagagagaaccagaccacccagaagggacagaagaacagccgcgagagaatgaagcggatcgaagagggcatcaaagagctgggcagccagatcctgaaagaacaccccgtggaaaacacccagctgcagaacgagaagctgtacctgtactacctgcagaatgggcgggatatgtacgtggaccaggaactggacatcaaccggctgtccgactacgatgtggacgctatcgtgcctcagagctttctgaaggacgactccatcgacaacaaggtgctgaccagaagcgacaagaaccggggcaagagcgacaacgtgccctccgaagaggtcgtgaagaagatgaagaactactggcggcagctgctgaacgccaagctgattacccagagaaagttcgacaatctgaccaaggccgagagaggcggcctgagcgaactggataaggccggcttcatcaagagacagctggtggaaacccggcagatcacaaagcacgtggcacagatcctggactcccggatgaacactaagtacgacgagaatgacaagctgatccgggaagtgaaagtgatcaccctgaagtccaagctggtgtccgatttccggaaggatttccagttttacaaagtgcgcgagatcaacaactaccaccacgcccacgacgcctacctgaacgccgtcgtgggaaccgccctgatcaaaaagtaccctaagctggaaagcgagttcgtgtacggcgactacaaggtgtacgacgtgcggaagatgatcgccaagagcgagcaggaaatcggcaaggctaccgccaagtacttcttctacagcaacatcatgaactttttcaagaccgagattaccctggccaacggcgagatccggaagcggcctctgatcgagacaaacggcgaaaccggggagatcgtgtgggataagggccgggattttgccaccgtgcggaaagtgctgagcatgccccaagtgaatatcgtgaaaaagaccgaggtgcagacaggcggcttcagcaaagagtctatcctgcccaagaggaacagcgataagctgatcgccagaaagaaggactgggaccctaagaagtacggcggcttcgacagccccaccgtggcctattctgtgctggtggtggccaaagtggaaaagggcaagtccaagaaactgaagagtgtgaaagagctgctggggatcaccatcatggaaagaagcagcttcgagaagaatcccatcgactttctggaagccaagggctacaaagaagtgaaaaaggacctgatcatcaagctgcctaagtactccctgttcgagctggaaaacggccggaagagaatgctggcctctgccggcgaactgcagaagggaaacgaactggccctgccctccaaatatgtgaacttcctgtacctggccagccactatgagaagctgaagggctcccccgaggataatgagcagaaacagctgtttgtggaacagcacaagcactacctggacgagatcatcgagcagatcagcgagttctccaagagagtgatcctggccgacgctaatctggacaaagtgctgtccgcctacaacaagcaccgggataagcccatcagagagcaggccgagaatatcatccacctgtttaccctgaccaatctgggagcccctgccgccttcaagtactttgacaccaccatcgaccggaagaggtacaccagcaccaaagaggtgctggacgccaccctgatccaccagagcatcaccggcctgtacgagacacggatcgacctgtctcagctgggaggtgactctggaggatctagcggaggatcctctggcagcgagacaccaggaacaagcgagtcagcaacaccagagagcagtggcggcagcagcggcggcagcagcaccctaaatatagaagatgagtatcggctacatgagacctcaaaagagccagatgtttctctagggtccacatggctgtctgattttcctcaggcctgggcggaaaccgggggcatgggactggcagttcgccaagctcctctgatcatacctctgaaagcaacctctacccccgtgtccataaaacaataccccatgtcacaagaagccagactggggatcaagccccacatacagagactgttggaccagggaatactggtaccctgccagtccccctggaacacgcccctgctacccgttaagaaaccagggactaatgattataggcctgtccaggatctgagagaagtcaacaagcgggtggaagacatccaccccaccgtgcccaacccttacaacctcttgagcgggctcccaccgtcccaccagtggtacactgtgcttgatttaaaggatgcctttttctgcctgagactccaccccaccagtcagcctctcttcgcctttgagtggagagatccagagatgggaatctcaggacaattgacctggaccagactcccacagggtttcaaaaacagtcccaccctgtttaatgaggcactgcacagagacctagcagacttccggatccagcacccagacttgatcctgctacagtacgtggatgacttactgctggccgccacttctgagctagactgccaacaaggtactcgggccctgttacaaaccctagggaacctcgggtatcgggcctcggccaagaaagcccaaatttgccagaaacaggtcaagtatctggggtatcttctaaaagagggtcagagatggctgactgaggccagaaaagagactgtgatggggcagcctactccgaagacccctcgacaactaagggagttcctagggaaggcaggcttctgtcgcctcttcatccctgggtttgcagaaatggcagcccccctgtaccctctcaccaaaccggggactctgtttaattggggcccagaccaacaaaaggcctatcaagaaatcaagcaagctcttctaactgccccagccctggggttgccagatttgactaagccctttgaactctttgtcgacgagaagcagggctacgccaaaggtgtcctaacgcaaaaactgggaccttggcgtcggccggtggcctacctgtccaaaaagctagacccagtagcagctgggtggcccccttgcctacggatggtagcagccattgccgtactgacaaaggatgcaggcaagctaaccatgggacagccactagtcattctggccccccatgcagtagaggcactagtcaaacaaccccccgaccgctggctttccaacgcccggatgactcactatcaggccttgcttttggacacggaccgggtccagttcggaccggtggtagccctgaacccggctacgctgctcccactgcctgaggaagggctgcaacacaactgccttgatatcctggccgaagcccacggaacccgacccgacctaacggaccagccgctcccagacgccgaccacacctggtacacggatggaagcagtctcttacaagagggacagcgtaaggcgggagctgcggtgaccaccgagaccgaggtaatctgggctaaagccctgccagccgggacatccgctcagcgggctgaactgatagcactcacccaggccctaaagatggcagaaggtaagaagctaaatgtttatactgatagccgttatgcttttgctactgcccatatccatggagaaatatacagaaggcgtgggtggctcacatcagaaggcaaagagatcaaaaataaagacgagatcttggccctactaaaagccctctttctgcccaaaagacttagcataatccattgtccaggacatcaaaagggacacagcgccgaggctagaggcaaccggatggctgaccaagcggcccgaaaggcagccatcacagagactccagacacctctaccctcctcatagaaaattcatcaccctctggcggctcaaaaagaaccgccgacggcagcgaattcgagcccaagaagaagaggaaagtctaaccggtcatcatcaccatcaccattgagttttacccctacgacgtgcccgactacgcctaataactcgagcatgcatctagagggccctattctatagtgtcacctaaatgctagagctcgctgatcagcctcgactgtgccttctagttgccagccatctgttgtttgcccctcccccgtgccttccttgaccctggaaggtgccactcccactgtcctttcctaataaaatgaggaaattgcatcgcattgtctgagtaggtgtcattctattctggggggtggggtggggcaggacagcaagggggaggattgggaagacaatagcaggcatgctggggaggatctgcgatcgctccggtgcccgtcagtgggcagagcgcacatcgcccacagtccccgagaagttggggggaggggtcggcaattgaacgggtgcctagagaaggtggcgcggggtaaactgggaaagtgatgtcgtgtactggctccgcctttttcccgagggtgggggagaaccgtatataagtgcagtagtcgccgtgaacgttctttttcgcaacgggtttgccgccagaacacagctgaagcttcgaggggctcgcatctctccttcacgcgcccgccgccctacctgaggccgccatccacgccggttgagtcgcgttctgccgcctcccgcctgtggtgcctcctgaactgcgtccgccgtctaggtaagtttaaagctcaggtcgagaccgggcctttgtccggcgctcccttggagcctacctagactcagccggctctccacgctttgcctgaccctgcttgctcaactctacgtctttgtttcgttttctgttctgcgccgttacagatccaagctgtgaccggcgcctacatgaccgagtacaagcccacggtgcgcctcgccacccgcgacgacgtccccagggccgtacgcaccctcgccgccgcgttcgccgactaccccgccacgcgccacaccgtcgatccagaccgccacatcgagcgggtcaccgagctgcaagaactcttcctcacgcgcgtcgggctcgacatcggcaaggtgtgggtcgcggacgacggcgccgcggtggcggtctggaccacgccggagagcgtcgaagcgggggcggtgttcgccgagatcggcccgcgcatggccgagttgagcggttcccggctggccgcgcagcaacagatggaaggtctcctggcgccgcaccggcccaaggagcccgcgtggttcctggccaccgtcggcgtctcgcccgaccaccagggcaagggtctgggcagcgccgtcgtgctccccggagtggaggcggccgagcgcgccggggtgcccgccttcctggagacctccgcgccccgcaacctccccttctacgagcggctcggcttcaccgtcaccgccgacgtcgaggtgcccgaaggaccgcgcacctggtgcatgacccgcaagcccggtgcctgagctagaagctcgctttcttgctgtccaatttctattaaaggttcctttgttccctaagtccaactactaaactgggggatattatgaagggccttgagcatctggattctgcctaataaaaaacatttattttcattgcaatgatgtatttaaattatttctgaatattttactaaaaagggaatgtgggaggtcagtgcatttaaaacataaagaaatgaagagctagttcaaaccttgggaaaatacactatatcttaaactccatgaaagaaggtgaggctgcaaacagctaatgcacattggcaacagcccctgatgcctatgccttattcatccctcagaaaaggattcaagtagaggcttgatttggaggttaaagttttgctatgctgtattttagaattccataccacatttgtagaggttttacttgctttaaaaaacctcccacacctccccctgaacctgaaacataaaatgaatgcaattgttgttgttttaccaatgcttaatcagtgaggcacctatctcagcgatctgtctatttcgttcatccatagttgcctgactccccgtcgtgtagataactacgatacgggagggcttaccatctggccccagtgctgcaatgataccgcgagacccacgctcaccggctccagatttatcagcaataaaccagccagccggaagggccgagcgcagaagtggtcctgcaactttatccgcctccatccagtctattaattgttgccgggaagctagagtaagtagttcgccagttaatagtttgcgcaacgttgttgccattgctacaggcatcgtggtgtcacgctcgtcgtttggtatggcttcattcagctccggttcccaacgatcaaggcgagttacatgatcccccatgttgtgcaaaaaagcggttagctccttcggtcctccgatcgttgtcagaagtaagttggccgcagtgttatcactcatggttatggcagcactgcataattctcttactgtcatgccatccgtaagatgcttttctgtgactggtgagtactcaaccaagtcattctgagaatagtgtatgcggcgaccgagttgctcttgcccggcgtcaatacgggataataccgcgccacatagcagaactttaaaagtgctcatcattggaaaacgttcttcggggcgaaaactctcaaggatcttaccgctgttgagatccagttcgatgtaacccactcgtgcacccaactgatcttcagcatcttttactttcaccagcgtttctgggtgagcaaaaacaggaaggcaaaatgccgcaaaaaagggaataagggcgacacggaaatgttgaatactcatactcttcctttttcaatattattgaagcatttatcagggttattgtctcatgagcggatacatatttgaatgtatttagaaaaataaacaaataggggttccgcgaacttgtttattgcagcttataatggttacaaataaagcaatagcatcacaaatttcacaaataaagcatttttttcactgcattctagttgtggtttgtccaaactcatcaatgtatcttatcatgtctggccagctagccaacaagctcgtcatcgctttgcagaagagcagagaggatatgctcatcgtctaaagaactacccattttattatatattagtcacgatatctataacaagaaaatatatatataataagttatcacgtaagtagaacatgaaataacaatataattatcgtatgagttaaatcttaaaagtcacgtaaaagataatcatgcgtcattttgactcacgcggtcgttatagttcaaaatcagtgacacttaccgcattgacaagcacgcctcacgggagctccaagcggcgactgagatgtcctaaatgcacagcgacggattcgcgctatttagaaagagagagcaatatttcaagaatgcatgcgtcaattttacgcagactatctttctagggttaaaaaagatttgcgctttactcgacctaaactttaaacacgtcatagaatcttcgtttgacaaaaaccacattgtggccaagctgtgtgacgcgacgcgcgctaaagaatggcaaaccaagtcgcgcgaggtacccagcttttgttccctttagtgagggttaattccgagcttggcgtaatcatggtcatagctgtttcctgtgtgaaattgttatccgctcacaattccacacaacatacgagccggaagcataaagtgtaaagcctggggtgcctaatgagtgagctaactcacattaattgcgttgcgctcactgcccgctttccagtcgggaaacctgtcgtgccagctgcattaatgaatcggccaacgcgcggggagaggcggtttgcgtattgggcgctcttccgcttcctcgctcactgactcgctgcgctcggtcgttcggctgcggcgagcggtatcagctcactcaaaggcggtaatacggttatccacagaatcaggggataacgcaggaaagaacatgtgagcaaaaggccagcaaaaggccaggaaccgtaaaaaggccgcgttgctggcgtttttccataggctccgcccccctgacgagcatcacaaaaatcgacgctcaagtcagaggtggcgaaacccgacaggactataaagataccaggcgtttccccctggaagctccctcgtgcgctctcctgttccgaccctgccgcttaccggatacctgtccgcctttctcccttcgggaagcgtggcgctttctcatagctcacgctgtaggtatctcagttcggtgtaggtcgttcgctccaagctgggctgtgtgcacgaaccccccgttcagcccgaccgctgcgccttatccggtaactatcgtcttgagtccaacccggtaagacacgacttatcgccactggcagcagccactggtaacaggattagcagagcgaggtatgtaggcggtgctacagagttcttgaagtggtggcctaactacggctacactagaaggacagtatttggtatctgcgctctgctgaagccagttaccttcggaaaaagagttggtagctcttgatccggcaaacaaaccaccgctggtagcggtggtttttttgtttgcaagcagcagattacgcgcagaaaaaaaggatctcaagaagatcctttgatcttttctacggggtctgacgctcagtggaacgaaaactcacgttaagggattttggtcatgattaaccctagaaagataatcatattgtgacgtacgttaaagataatcatgcgtaaaattgacgcatgtgttttatcggtctgtatatcgaggtttatttattaatttgaatagatattaagttttattatatttacacttacatactaataataaattcaacaaacaatttatttatgtttatttatttattaaaaaaaaacaaaaactcaaaatttcttctataaagtaacaaaacttttaaacattctctcttttacaaaaataaacttattttgtactttaaaaacagtcatgttgtattataaaataagtaattagcttaacctatacataatagaaacaaattatacttattagtcagtcagaaacaactttggcacatatcaatattatgctctcgttaattaa

SEQ ID NO: 149 - DNA, 3632 bp, synthetic construct
  source 1..3632: mol_type = other DNA
gacgaagactcaattgtcgattagtgaacggatctcgacggtatcgatcacgagactagcctcgagcggccgcccccttcaccgagggcctatttcccatgattccttcatatttgcatatacgatacaaggctgttagagagataattggaattaatttgactgtaaacacaaagatattagtacaaaatacgtgacgtagaaagtaataatttcttgggtagtttgcagttttaaaattatgttttaaaatggactatcatatgcttaccgtaacttgaaagtatttcgatttcttggctttatatatcttgtggaaaggacgaaacaccggagaccacatttccccgaaaagtgccacctgacgtctaagaaaccattattatcatgacattaacctataaaaataggcgtatcacgaggccctttcgtctcgcgcgtttcggtgatgacggtgaaaacctctgacacatgcagctcccggagacggtcacagcttgtctgtaagcggatgccgggagcagacaagcccgtcagggcgcgtcagcgggtgttggcgggtgtcggggctggcttaactatgcggcatcagagcagattgtactgagagtgcaccatatgcggtgtgaaataccgcacagatgcgtaaggagaaaataccgcatcaggcgccattcgccattcaggctgcgcaactgttgggaagggcgatcggtgcgggcctcttcgctattacgccagctggcgaaagggggatgtgctgcaaggcgattaagttgggtaacgccagggttttcccagtcacgacgttgtaaaacgacggccagtgccaagcttgcatgcctgcaggtcgactctagaggatccccgggtaccgagctcgaattcgtaatcatggtcatagctgtttcctgtgtgaaattgttatccgctcacaattccacacaacatacgagccggaagcataaagtgtaaagcctggggtgcctaatagatccggtctccgttttagagctagaaatagcaagttaaaataaggctagtccgttatcaacttgaaaaagtggcaccgagtcggtgcggagacgtgtctgtaagcggatgccgggagcagacaagcccgtcagggcgcgtcagcgggtgttggcgggtgtcggggctggcttaactatgcggcatcagagcagattgtactgagagtgcaccatatgcggtgtgaaataccgcacagatgcgtaaggagaaaataccgcatcaggcgccattcgccattcaggctgcgcaactgttgggaagggcgatcggtgcgggcctcttcgctattacgccagctggcgaaagggggatgtgctgcaaggcgattaagttgggtaacgccagggttttcccagtcacgacgttgtaaaacgacggccagtgccaagcttgcatgcctgcaggtcgactctagaggatccccgggtaccgagctcgaattcgtaatcatggtcatagctgtttcctgtgtgaaattgttatccgctcacaattccacacaacatacgagccggcgtctcccgcggttctatctagttacgcgttaaaccaactagaattttttagatatacgcgttgacattgattattgactagttgtcttcctgcattaatgaatcggccaacgcgcggggagaggcggtttgcgtattgggcgctcttccgcttcctcgctcactgactcgctgcgctcggtcgttcggctgcggcgagcggtatcagctcactcaaaggcggtaatacggttatccacagaatcaggggataacgcaggaaagaacatgtgagcaaaaggccagcaaaaggccaggaaccgtaaaaaggccgcgttgctggcgtttttccataggctccgcccccctgacgagcatcacaaaaatcgacgctcaagtcagaggtggcgaaacccgacaggactataaagataccaggcgtttccccctggaagctccctcgtgcgctctcctgttccgaccctgccgcttaccggatacctgtccgcctttctcccttcgggaagcgtggcgctttctcaatgctcacgctgtaggtatctcagttcggtgtaggtcgttcgctccaagctgggctgtgtgcacgaaccccccgttcagcccgaccgctgcgccttatccggtaactatcgtcttgagtccaacccggtaagacacgacttatcgccactggcagcagccactggtaacaggattagcagagcgaggtatgtaggcggtgctacagagttcttgaagtggtggcctaactacggctacactagaaggacagtatttggtatctgcgctctgctgaagccagttaccttcggaaaaagagttggtagctcttgatccggcaaacaaaccaccgctggtagcggtggtttttttgtttgcaagcagcagattacgcgcagaaaaaaaggatctcaagaagatcctttgatcttttctacggggtctgacgctcagtggaacgaaaactcacgttaagggattttggtcatgagattatcaaaaaggatcttcacctagatccttttaaattaaaaatgaagttttaaatcaatctaaagtatatatgagtaaacttggtctgacagttaccaatgcttaatcagtgaggcacctatctcagcgatctgtctatttcgttcatccatagttgcctgactccccgtcgtgtagataactacgatacgggagggcttaccatctggccccagtgctgcaatgataccgcgagatccacgctcaccggctccagatttatcagcaataaaccagccagccggaagggccgagcgcagaagtggtcctgcaactttatccgcctccatccagtctattaattgttgccgggaagctagagtaagtagttcgccagttaatagtttgcgcaacgttgttgccattgctacaggcatcgtggtgtcacgctcgtcgtttggtatggcttcattcagctccggttcccaacgatcaaggcgagttacatgatcccccatgttgtgcaaaaaagcggttagctccttcggtcctccgatcgttgtcagaagtaagttggccgcagtgttatcactcatggttatggcagcactgcataattctcttactgtcatgccatccgtaagatgcttttctgtgactggtgagtactcaaccaagtcattctgagaatagtgtatgcggcgaccgagttgctcttgcccggcgtcaatacgggataataccgcgccacatagcagaactttaaaagtgctcatcattggaaaacgttcttcggggcgaaaactctcaaggatcttaccgctgttgagatccagttcgatgtaacccactcgtgcacccaactgatcttcagcatcttttactttcaccagcgtttctgggtgagcaaaaacaggaaggcaaaatgccgcaaaaaagggaataagggcgacacggaaatgttgaatactcatactcttcctttttcaatattattgaagcatttatcagggttattgtctcatgagcggatacatatttgaatgtatttagaaaaataaacaaataggggttccgcgcacatttccccgaaaagtgccacctgacgtc

SEQ ID NO: 150 - DNA, 14847 bp, synthetic construct
  source 1..14847: mol_type = other DNA
cgatgtacgggccagatatacgcgcgtatatctggcccgtacatcgcgaatctagaaaaaannnnnnnnnnnnnnnnnnnnnnnnnnnnngcaccgactcggtgccactttttcaagttgataacggactagccttattttaacttgctatttctagctctaaaacnnnnnnnnnnnnnnnnnnncggtgtttcgtcctttccacaagatatataaagccaagaaatcgaaatactttcaagttacggtaagcatatgatagtccattttaaaacataattttaaaactgcaaactacccaagaaattattactttctacgtcacgtattttgtactaatatctttgtgtttacagtcaaattaattccaattatctctctaacagccttgtatcgtatatgcaaatatgaaggaatcatgggaaataggccctccgcgttgacattgattattgactagttattaatagtaatcaattacggggtcattagttcatagcccatatatggagttccgcgttacataacttacggtaaatggcccgcctggctgaccgcccaacgacccccgcccattgacgtcaataatgacgtatgttcccatagtaacgccaatagggactttccattgacgtcaatgggtggagtatttacggtaaactgcccacttggcagtacatcaagtgtatcatatgccaagtacgccccctattgacgtcaatgacggtaaatggcccgcctggcattatgcccagtacatgaccttatgggactttcctacttggcagtacatctacgtattagtcatcgctattaccatggtgatgcggttttggcagtacatcaatgggcgtggatagcggtttgactcacggggatttccaagtctccaccccattgacgtcaatgggagtttgttttggcaccaaaatcaacgggactttccaaaatgtcgtaacaactccgccccattgacgcaaatgggcggtaggcgtgtacggtgggaggtctatataagcagagctggtttagtgaaccgtcagatccgctagagatccgcggccgctaatacgactcactatagggagagccgccaccatgaaacggacagccgacggaagcgagttcgagtcaccaaagaagaagcggaaagtcgacaagaagtacagcatcggcctggacatcggcaccaactctgtgggctgggccgtgatcaccgacgagtacaaggtgcccagcaagaaattcaaggtgctgggcaacaccgaccggcacagcatcaagaagaacctgatcggagccctgctgttcgacagcggcgaaacagccgaggccacccggctgaagagaaccgccagaagaagatacaccagacggaagaaccggatctgctatctgcaagagatcttcagcaacgagatggccaaggtggacgacagcttcttccacagactggaagagtccttcctggtggaagaggataagaagcacgagcggcaccccatcttcggcaacatcgtggacgaggtggcctaccacgagaagtaccccaccatctaccacctgagaaagaaactggtggacagcaccgacaaggccgacctgcggctgatctatctggccctggcccacatgatcaagttccggggccacttcctgatcgagggcgacctgaaccccgacaacagcgacgtggacaagctgttcatccagctggtgcagacctacaaccagctgttcgaggaaaaccccatcaacgccagcggcgtggacgccaaggccatcctgtctgccagactgagcaagagcagacggctggaaaatctgatcgcccagctgcccggcgagaagaagaatggcctgttcggaaacctgattgccctgagcctgggcctgacccccaacttcaagagcaacttcgacctggccgaggatgccaaactgcagctgagcaaggacacctacgacgacgacctggacaacctgctggcccagatcggcgaccagtacgccgacctgtttctggccgccaagaacctgtccgacgccatcctgctgagcgacatcctgagagtgaacaccgagatcaccaaggcccccctgagcgcctctatgatcaagagatacgacgagcaccaccaggacctgaccctgctgaaagctctcgtgcggcagcagctgcctgagaagtacaaagagattttcttcgaccagagcaagaacggctacgccggctacattgacggcggagccagccaggaagagttctacaagttcatcaagcccatcctggaaaagatggacggcaccgaggaactgctcgtgaagctgaacagagaggacctgctgcggaagcagcggaccttcgacaacggcagcatcccccaccagatccacctgggagagctgcacgccattctgcggcggcaggaagatttttacccattcctgaaggacaaccgggaaaagatcgagaagatcctgaccttccgcatcccctactacgtgggccctctggccaggggaaacagcagattcgcctggatgaccagaaagagcgaggaaaccatcaccccctggaacttcgaggaagtggtggacaagggcgcttccgcccagagcttcatcgagcggatgaccaacttcgataagaacctgcccaacgagaaggtgctgcccaagcacagcctgctgtacgagtacttcaccgtgtataacgagctgaccaaagtgaaatacgtgaccgagggaatgagaaagcccgccttcctgagcggcgagcagaaaaaggccatcgtggacctgctgttcaagaccaaccggaaagtgaccgtgaagcagctgaaagaggactacttcaagaaaatcgagtgcttcgactccgtggaaatctccggcgtggaagatcggttcaacgcctccctgggcacataccacgatctgctgaaaattatcaaggacaaggacttcctggacaatgaggaaaacgaggacattctggaagatatcgtgctgaccctgacactgtttgaggacagagagatgatcgaggaacggctgaaaacctatgcccacctgttcgacgacaaagtgatgaagcagctgaagcggcggagatacaccggctggggcaggctgagccggaagctgatcaacggcatccgggacaagcagtccggcaagacaatcctggatttcctgaagtccgacggcttcgccaacagaaacttcatgcagctgatccacgacgacagcctgacctttaaagaggacatccagaaagcccaggtgtccggccagggcgatagcctgcacgagcacattgccaatctggccggcagccccgccattaagaagggcatcctgcagacagtgaaggtggtggacgagctcgtgaaagtgatgggccggcacaagcccgagaacatcgtgatcgaaatggccagagagaaccagaccacccagaagggacagaagaacagccgcgagagaatgaagcggatcgaagagggcatcaaagagctgggcagccagatcctgaaagaacaccccgtggaaaacacccagctgcagaacgagaagctgtacctgtactacctgcagaatgggcgggatatgtacgtggaccaggaactggacatcaaccggctgtccgactacgatgtggacgctatcgtgcctcagagctttctgaaggacgactccatcgacaacaaggtgctgaccagaagcgacaagaaccggggcaagagcgacaacgtgccctccgaagaggtcgtgaagaagatgaagaactactggcggcagctgctgaacgccaagctgattacccagagaaagttcgacaatctgaccaaggccgagagaggcggcctgagcgaactggataaggccggcttcatcaagagacagctggtggaaacccggcagatcacaaagcacgtggcacagatcctggactcccggatgaacactaagtacgacgagaatgacaagctgatccgggaagtgaaagtgatcaccctgaagtccaagctggtgtccgatttccggaaggatttccagttttacaaagtgcgcgagatcaacaactaccaccacgcccacgacgcctacctgaacgccgtcgtgggaaccgccctgatcaaaaagtaccctaagctggaaagcgagttcgtgtacggcgactacaaggtgtacgacgtgcggaagatgatcgccaagagcgagcaggaaatcggcaaggctaccgccaagtacttcttctacagcaacatcatgaactttttcaagaccgagattaccctggccaacggcgagatccggaagcggcctctgatcgagacaaacggcgaaaccggggagatcgtgtgggataagggccgggattttgccaccgtgcggaaagtgctgagcatgccccaagtgaatatcgtgaaaaagaccgaggtgcagacaggcggcttcagcaaagagtctatcctgcccaagaggaacagcgataagctgatcgccagaaagaaggactgggaccctaagaagtacggcggcttcgacagccccaccgtggcctattctgtgctggtggtggccaaagtggaaaagggcaagtccaagaaactgaagagtgtgaaagagctgctggggatcaccatcatggaaagaagcagcttcgagaagaatcccatcgactttctggaagccaagggctacaaagaagtgaaaaaggacctgatcatcaagctgcctaagtactccctgttcgagctggaaaacggccggaagagaatgctggcctctgccggcgaactgcagaagggaaacgaactggccctgccctccaaatatgtgaacttcctgtacctggccagccactatgagaagctgaagggctcccccgaggataatgagcagaaacagctgtttgtggaacagcacaagcactacctggacgagatcatcgagcagatcagcgagttctccaagagagtgatcctggccgacgctaatctggacaaagtgctgtccgcctacaacaagcaccgggataagcccatcagagagcaggccgagaatatcatccacctgtttaccctgaccaatctgggagcccctgccgccttcaagtactttgacaccaccatcgaccggaagaggtacaccagcaccaaagaggtgctggacgccaccctgatccaccagagcatcaccggcctgtacgagacacggatcgacctgtctcagctgggaggtgactctggaggatctagcggaggatcctctggcagcgagacaccaggaacaagcgagtcagcaacaccagagagcagtggcggcagcagcggcggcagcagcaccctaaatatagaagatgagtatcggctacatgagacctcaaaagagccagatgtttctctagggtccacatggctgtctgattttcctcaggcctgggcggaaaccgggggcatgggactggcagttcgccaagctcctctgatcatacctctgaaagcaacctctacccccgtgtccataaaacaataccccatgtcacaagaagccagactggggatcaagccccacatacagagactgttggaccagggaatactggtaccctgccagtccccctggaacacgcccctgctacccgttaagaaaccagggactaatgattataggcctgtccaggatctgagagaagtcaacaagcgggtggaagacatccaccccaccgtgcccaacccttacaacctcttgagcgggctcccaccgtcccaccagtggtacactgtgcttgatttaaaggatgcctttttctgcctgagactccaccccaccagtcagcctctcttcgcctttgagtggagagatccagagatgggaatctcaggacaattgacctggaccagactcccacagggtttcaaaaacagtcccaccctgtttaatgaggcactgcacagagacctagcagacttccggatccagcacccagacttgatcctgctacagtacgtggatgacttactgctggccgccacttctgagctagactgccaacaaggtactcgggccctgttacaaaccctagggaacctcgggtatcgggcctcggccaagaaagcccaaatttgccagaaacaggtcaagtatctggggtatcttctaaaagagggtcagagatggctgactgaggccagaaaagagactgtgatggggcagcctactccgaagacccctcgacaactaagggagttcctagggaaggcaggcttctgtcgcctcttcatccctgggtttgcagaaatggcagcccccctgtaccctctcaccaaaccggggactctgtttaattggggcccagaccaacaaaaggcctatcaagaaatcaagcaagctcttctaactgccccagccctggggttgccagatttgactaagccctttgaactctttgtcgacgagaagcagggctacgccaaaggtgtcctaacgcaaaaactgggaccttggcgtcggccggtggcctacctgtccaaaaagctagacccagtagcagctgggtggcccccttgcctacggatggtagcagccattgccgtactgacaaaggatgcaggcaagctaaccatgggacagccactagtcattctggccccccatgcagtagaggcactagtcaaacaaccccccgaccgctggctttccaacgcccggatgactcactatcaggccttgcttttggacacggaccgggtccagttcggaccggtggtagccctgaacccggctacgctgctcccactgcctgaggaagggctgcaacacaactgccttgatatcctggccgaagcccacggaacccgacccgacctaacggaccagccgctcccagacgccgaccacacctggtacacggatggaagcagtctcttacaagagggacagcgtaaggcgggagctgcggtgaccaccgagaccgaggtaatctgggctaaagccctgccagccgggacatccgctcagcgggctgaactgatagcactcacccaggccctaaagatggcagaaggtaagaagctaaatgtttatactgatagccgttatgcttttgctactgcccatatccatggagaaatatacagaaggcgtgggtggctcacatcagaaggcaaagagatcaaaaataaagacgagatcttggccctactaaaagccctctttctgcccaaaagacttagcataatccattgtccaggacatcaaaagggacacagcgccgaggctagaggcaaccggatggctgaccaagcggcccgaaaggcagccatcacagagactccagacacctctaccctcctcatagaaaattcatcaccctctggcggctcaaaaagaaccgccgacggcagcgaattcgagcccaagaagaagaggaaagtcggaagcggagctactaacttcagcctgctgaagcaggctggagacgtggaggagaaccctggacctagcttcgttgctggagtcatccggagactggacgagacagtggtgaacagaattgccgccggcgaggtgatccagagacctgccaatgcaataaaggagatgatcgagaactgtctggacgccaagtccacaagcattcaggtgatcgtgaaggagggcggactgaagctgatccagatccaagacaacggcacaggcatcagaaaggaagatctggacatcgtgtgtgaacggttcaccacatctaagctgcagtcttttgaggatctggcctctatcagtacctacggcttcagaggcgaggccctggccagcatcagccacgtggcccatgtgaccatcaccaccaaaaccgccgacggcaaatgcgcttatcgcgctagctacagcgacggcaagctgaaagccccgccaaagccttgcgccggcaaccagggtacacagataacagtggaggatctgttctacaacatcgccacccggagaaaggccctgaaaaatcccagcgaggagtacggcaagatcctggaagtcgtcggcagatactccgtgcacaacgccggaatcagctttagcgtaaagaagcagggagaaaccgtggccgatgtgcgcaccctgccaaatgccagcaccgtggataacatcagaagcattttcggaaatgccgtgtccagagaactgatcgagatcggctgcgaagataagaccctggcttttaagatgaacggctacatcagcaacgccaattactctgtgaagaagtgcatctttcttctgttcatcaaccacagactggtggaaagcaccagcctgcggaaagccatcgagacagtgtacgccgcctacctgcctaagaacacccaccccttcctgtacctgagcctcgagatcagccctcagaacgtggacgtcaatgtgcatcctacaaagcacgaggtgcacttcctgcacgaggaaagcatcctggaaagagtgcagcagcacattgagagcaagctgctgggctctaacagcagcagaatgtacttcacacagaccctgctgcctggcctggccggcccctcaggcgaaatggttaagtccacaacctctctgacctcatccagcaccagcggttcttccgataaggtgtacgcccaccagatggtgcggaccgactctcgggagcagaagctggacgcctttctgcaacctctgagcaaacctctgagctctcagcctcaggccatcgtgaccgaggacaagacagatatctcctccggccgtgccagacagcaggacgaagaaatgctcgagctgccagctcctgccgaggtggccgccaagaaccagagcctggagggagataccacaaagggcaccagcgaaatgagcgagaagcggggccctacctccagcaaccccagaaaacggcaccgggaggacagcgacgtggaaatggtggaggacgacagcagaaaggaaatgacagccgcttgtacccctagaagaagaatcatcaacctgacctccgtgctgagcctgcaggaggagatcaacgagcagggccacgaggtgctgagagagatgctgcacaatcacagcttcgtgggctgcgtgaaccctcaatgggccctggctcagcatcaaacaaagctgtacctgctgaacaccaccaagctgagcgaagagctgttctaccagatcctcatctacgacttcgccaacttcggcgtgctacgcctgagcgagcccgcccctctgtttgacctggccatgctggctctggatagcccagaaagcggctggacagaagaggacggacctaaagaggggctggctgaatacatcgtggagttcctgaagaaaaaggccgagatgctggccgactacttttctctggaaatcgacgaggaaggcaacctgatcggcctgcctctgctgatcgataactacgtgcctcccctggaaggcctgcccatcttcatcctgagactggctacagaggtgaactgggacgaggaaaaggaatgcttcgagtctctgagcaaggagtgcgccatgttctatagcatcagaaaacagtacatctctgaagagagcactctgtctggccagcagagtgaagtgcccggaagcatccccaacagctggaagtggaccgtggaacacatcgtgtacaaggccctgcggagccacattctccctcctaagcacttcaccgaggacggcaacatcctgcagctggccaacctgcccgacctttataaggttttctaactcgagcatgcatctagagggccctattctatagtgtcacctaaatgctagagctcgctgatcagcctcgactgtgccttctagttgccagccatctgttgtttgcccctcccccgtgccttccttgaccctggaaggtgccactcccactgtcctttcctaataaaatgaggaaattgcatcgcattgtctgagtaggtgtcattctattctggggggtggggtggggcaggacagcaagggggaggattgggaagacaatagcaggcatgctggggaggatctgcgatcgctccggtgcccgtcagtgggcagagcgcacatcgcccacagtccccgagaagttggggggaggggtcggcaattgaacgggtgcctagagaaggtggcgcggggtaaactgggaaagtgatgtcgtgtactggctccgcctttttcccgagggtgggggagaaccgtatataagtgcagtagtcgccgtgaacgttctttttcgcaacgggtttgccgccagaacacagctgaagcttcgaggggctcgcatctctccttcacgcgcccgccgccctacctgaggccgccatccacgccggttgagtcgcgttctgccgcctcccgcctgtggtgcctcctgaactgcgtccgccgtctaggtaagtttaaagctcaggtcgagaccgggcctttgtccggcgctcccttggagcctacctagactcagccggctctccacgctttgcctgaccctgcttgctcaactctacgtctttgtttcgttttctgttctgcgccgttacagatccaagctgtgaccggcgcctacatgaccgagtacaagcccacggtgcgcctcgccacccgcgacgacgtccccagggccgtacgcaccctcgccgccgcgttcgccgactaccccgccacgcgccacaccgtcgatccagaccgccacatcgagcgggtcaccgagctgcaagaactcttcctcacgcgcgtcgggctcgacatcggcaaggtgtgggtcgcggacgacggcgccgcggtggcggtctggaccacgccggagagcgtcgaagcgggggcggtgttcgccgagatcggcccgcgcatggccgagttgagcggttcccggctggccgcgcagcaacagatggaaggtctcctggcgccgcaccggcccaaggagcccgcgtggttcctggccaccgtcggcgtctcgcccgaccaccagggcaagggtctgggcagcgccgtcgtgctccccggagtggaggcggccgagcgcgccggggtgcccgccttcctggagacctccgcgccccgcaacctccccttctacgagcggctcggcttcaccgtcaccgccgacgtcgaggtgcccgaaggaccgcgcacctggtgcatgacccgcaagcccggtgcctgagctagaagctcgctttcttgctgtccaatttctattaaaggttcctttgttccctaagtccaactactaaactgggggatattatgaagggccttgagcatctggattctgcctaataaaaaacatttattttcattgcaatgatgtatttaaattatttctgaatattttactaaaaagggaatgtgggaggtcagtgcatttaaaacataaagaaatgaagagctagttcaaaccttgggaaaatacactatatcttaaactccatgaaagaaggtgaggctgcaaacagctaatgcacattggcaacagcccctgatgcctatgccttattcatccctcagaaaaggattcaagtagaggcttgatttggaggttaaagttttgctatgctgtattttagaattccataccacatttgtagaggttttacttgctttaaaaaacctcccacacctccccctgaacctgaaacataaaatgaatgcaattgttgttgttttaccaatgcttaatcagtgaggcacctatctcagcgatctgtctatttcgttcatccatagttgcctgactccccgtcgtgtagataactacgatacgggagggcttaccatctggccccagtgctgcaatgataccgcgagacccacgctcaccggctccagatttatcagcaataaaccagccagccggaagggccgagcgcagaagtggtcctgcaactttatccgcctccatccagtctattaattgttgccgggaagctagagtaagtagttcgccagttaatagtttgcgcaacgttgttgccattgctacaggcatcgtggtgtcacgctcgtcgtttggtatggcttcattcagctccggttcccaacgatcaaggcgagttacatgatcccccatgttgtgcaaaaaagcggttagctccttcggtcctccgatcgttgtcagaagtaagttggccgcagtgttatcactcatggttatggcagcactgcataattctcttactgtcatgccatccgtaagatgcttttctgtgactggtgagtactcaaccaagtcattctgagaatagtgtatgcggcgaccgagttgctcttgcccggcgtcaatacgggataataccgcgccacatagcagaactttaaaagtgctcatcattggaaaacgttcttcggggcgaaaactctcaaggatcttaccgctgttgagatccagttcgatgtaacccactcgtgcacccaactgatcttcagcatcttttactttcaccagcgtttctgggtgagcaaaaacaggaaggcaaaatgccgcaaaaaagggaataagggcgacacggaaatgttgaatactcatactcttcctttttcaatattattgaagcatttatcagggttattgtctcatgagcggatacatatttgaatgtatttagaaaaataaacaaataggggttccgcgaacttgtttattgcagcttataatggttacaaataaagcaatagcatcacaaatttcacaaataaagcatttttttcactgcattctagttgtggtttgtccaaactcatcaatgtatcttatcatgtctggcagctagccaacaagctcgtcatcgctttgcagaagagcagagaggatatgctcatcgtctaaagaactacccattcgatatctataacaagaaaatatatatataataagttatcacgtaagtagaacatgaaataacaatataattatcgtatgagttaaatcttaaaagtcacgtaaaagataatcatgcgtcattttgactcacgcggtcgttatagttcaaaatcagtgacacttaccgcattgacaagcacgcctcacgggagctccaagcggcgactgagatgtcctaaatgcacagcgacggattcgcgctatttagaaagagagagcaatatttcaagaatgcatgcgtcaattttacgcagactatctttctagggttaaaaaagatttgcgctttactcgacctaaactttaaacacgtcatagaatcttcgtttgacaaaaaccacattgtggccaagctgtgtgacgcgacgcgcgctaaagaatggcaaaccaagtcgcgcgaggtacccagcttttgttccctttagtgagggttaattccgagcttggcgtaatcatggtcatagctgtttcctgtgtgaaattgttatccgctcacaattccacacaacatacgagccggaagcataaagtgtaaagcctggggtgcctaatgagtgagctaactcacattaattgcgttgcgctcactgcccgctttccagtcgggaaacctgtcgtgccagctgcattaatgaatcggccaacgcgcggggagaggcggtttgcgtattgggcgctcttccgcttcctcgctcactgactcgctgcgctcggtcgttcggctgcggcgagcggtatcagctcactcaaaggcggtaatacggttatccacagaatcaggggataacgcaggaaagaacatgtgagcaaaaggccagcaaaaggccaggaaccgtaaaaaggccgcgttgctggcgtttttccataggctccgcccccctgacgagcatcacaaaaatcgacgctcaagtcagaggtggcgaaacccgacaggactataaagataccaggcgtttccccctggaagctccctcgtgcgctctcctgttccgaccctgccgcttaccggatacctgtccgcctttctcccttcgggaagcgtggcgctttctcatagctcacgctgtaggtatctcagttcggtgtaggtcgttcgctccaagctgggctgtgtgcacgaaccccccgttcagcccgaccgctgcgccttatccggtaactatcgtcttgagtccaacccggtaagacacgacttatcgccactggcagcagccactggtaacaggattagcagagcgaggtatgtaggcggtgctacagagttcttgaagtggtggcctaactacggctacactagaaggacagtatttggtatctgcgctctgctgaagccagttaccttcggaaaaagagttggtagctcttgatccggcaaacaaaccaccgctggtagcggtggtttttttgtttgcaagcagcagattacgcgcagaaaaaaaggatctcaagaagatcctttgatcttttctacggggtctgacgctcagtggaacgaaaactcacgttaagggattttggtcatgattaaccctagaaagataatcatattgtgacgtacgttaaagataatcatgcgtaaaattgacgcatgtgttttatcggtctgtatatcgaggtttatttattaatttgaatagatattaagttttattatatttacacttacatactaataataaattcaacaaacaatttatttatgtttatttatttattaaaaaaaaacaaaaactcaaaatttcttctataaagtaacaaaacttttaaacattctctcttttacaaaaataaacttattttgtactttaaaaacagtcatgttgtattataaaataagtaattagcttaacctatacataatagaaacaaattatacttattagtcagtcagaaacaactttggcacatatcaatattatgctctcgttaattaa

SEQ ID NO: 151 - DNA, 12689 bp, synthetic construct
  source 1..12689: mol_type = other DNA
cgatgtacgggccagatatacgcgcgtatatctggcccgtacatcgcgaatctagaaaaaannnnnnnnnnnnnnnnnnnnnnnnnnnnngcaccgactcggtgccactttttcaagttgataacggactagccttattttaacttgctatttctagctctaaaacnnnnnnnnnnnnnnnnnnncggtgtttcgtcctttccacaagatatataaagccaagaaatcgaaatactttcaagttacggtaagcatatgatagtccattttaaaacataattttaaaactgcaaactacccaagaaattattactttctacgtcacgtattttgtactaatatctttgtgtttacagtcaaattaattccaattatctctctaacagccttgtatcgtatatgcaaatatgaaggaatcatgggaaataggccctccgcgttgacattgattattgactagttattaatagtaatcaattacggggtcattagttcatagcccatatatggagttccgcgttacataacttacggtaaatggcccgcctggctgaccgcccaacgacccccgcccattgacgtcaataatgacgtatgttcccatagtaacgccaatagggactttccattgacgtcaatgggtggagtatttacggtaaactgcccacttggcagtacatcaagtgtatcatatgccaagtacgccccctattgacgtcaatgacggtaaatggcccgcctggcattatgcccagtacatgaccttatgggactttcctacttggcagtacatctacgtattagtcatcgctattaccatggtgatgcggttttggcagtacatcaatgggcgtggatagcggtttgactcacggggatttccaagtctccaccccattgacgtcaatgggagtttgttttggcaccaaaatcaacgggactttccaaaatgtcgtaacaactccgccccattgacgcaaatgggcggtaggcgtgtacggtgggaggtctatataagcagagctctctggctaactagagaacccactgcttactggcttatcgaaatttccctatcagtgatagagattgacatccctatcagtgatagagatactgagcacatcagcaggacgcactgaccagggagacccaagcttgccaccatggtgtacccctacgacgtgcccgactacgccgaattgcctccaaaaaagaagagaaaggtagggatcctggacaagaagtacagcatcggcctggacatcggtaccaacagcgtgggctgggccgtgatcaccgacgagtacaaggtgcccagcaagaagttcaaggtgctgggcaacaccgaccgccacagcatcaagaagaacctgatcggcgccctgctgttcgacagcggcgagaccgccgaggccacccgcctgaagcgcaccgcccgccgccgctacacccgccgcaagaaccgcatctgctacctgcaggagatcttcagcaacgagatggccaaggtggacgacagcttcttccaccgcctggaggagagcttcctggtggaggaggacaagaagcacgagcgccaccccatcttcggcaacatcgtggacgaggtggcctaccacgagaagtaccccaccatctaccacctgcgcaagaagctggtggacagcaccgacaaggccgacctgcgcctgatctacctggccctggcccacatgatcaagttccgcggccacttcctgatcgagggcgacctgaaccccgacaacagcgacgtggacaagctgttcatccagctggtgcagacctacaaccagctgttcgaggagaaccccatcaacgccagcggcgtggacgccaaggccatcctgagcgcccgcctgagcaagagccgccgcctggagaacctgatcgcccagctgcccggcgagaagaagaacggcctgttcggcaacctgatcgccctgagcctgggcctgacccccaacttcaagagcaacttcgacctggccgaggacgccaagctgcagctgagcaaggacacctacgacgacgacctggacaacctgctggcccagatcggcgaccagtacgccgacctgttcctggccgccaagaacctgagcgacgccatcctgctgagcgacatcctgcgcgtgaacaccgagatcaccaaggcccccctgagcgccagcatgatcaagcgctacgacgagcaccaccaggacctgaccctgctgaaggccctggtgcgccagcagctgcccgagaagtacaaggagatcttcttcgaccagagcaagaacggctacgccggctacatcgacggcggcgccagccaggaggagttctacaagttcatcaagcccatcctggagaagatggacggcaccgaggagctgctggtgaagctgaaccgcgaggacctgctgcgcaagcagcgcaccttcgacaacggcagcatcccccaccagatccacctgggcgagctgcacgccatcctgcgccgccaggaggacttctaccccttcctgaaggacaaccgcgagaagatcgagaagatcctgaccttccgcatcccctactacgtgggccccctggcccgcggcaacagccgcttcgcctggatgacccgcaagagcgaggagaccatcaccccctggaacttcgaggaggtggtggacaagggcgccagcgcccagagcttcatcgagcgcatgaccaacttcgacaagaacctgcccaacgagaaggtgctgcccaagcacagcctgctgtacgagtacttcaccgtgtacaacgagctgaccaaggtgaagtacgtgaccgagggcatgcgcaagcccgccttcctgagcggcgagcagaagaaggccatcgtggacctgctgttcaagaccaaccgcaaggtgaccgtgaagcagctgaaggaggactacttcaagaagatcgagtgcttcgacagcgtggagatcagcggcgtggaggaccgcttcaacgccagcctgggcacctaccacgacctgctgaagatcatcaaggacaaggacttcctggacaacgaggagaacgaggacatcctggaggacatcgtgctgaccctgaccctgttcgaggaccgcgagatgatcgaggagcgcctgaagacctacgcccacctgttcgacgacaaggtgatgaagcagctgaagcgccgccgctacaccggctggggccgcctgagccgcaagcttatcaacggcatccgcgacaagcagagcggcaagaccatcctggacttcctgaagagcgacggcttcgccaaccgcaacttcatgcagctgatccacgacgacagcctgaccttcaaggaggacatccagaaggcccaggtgagcggccagggcgacagcctgcacgagcacatcgccaacctggccggcagccccgccatcaagaagggcatcctgcagaccgtgaaggtggtggacgagctggtgaaggtgatgggccgccacaagcccgagaacatcgtgatcgagatggcccgcgagaaccagaccacccagaagggccagaagaacagccgcgagcgcatgaagcgcatcgaggagggcatcaaggagctgggcagccagatcctgaaggagcaccccgtggagaacacccagctgcagaacgagaagctgtacctgtactacctgcagaacggccgcgacatgtacgtggaccaggagctggacatcaaccgcctgagcgactacgacgtggaccacatcgtgccccagagcttcctgaaggacgacagcatcgacaacaaggtgctgacccgcagcgacaagaaccgcggcaagagcgacaacgtgcccagcgaggaggtggtgaagaagatgaagaactactggcgccagctgctgaacgccaagctgatcacccagcgcaagttcgacaacctgaccaaggccgagcgcggcggcctgagcgagctggacaaggccggcttcatcaagcgccagctggtggagacccgccagatcaccaagcacgtggcacagatcctggactcccggatgaacactaagtacgacgagaatgacaagctgatccgggaagtgaaagtgatcaccctgaagtccaagctggtgtccgatttccggaaggatttccagttttacaaagtgcgcgagatcaacaactaccaccacgcccacgacgcctacctgaacgccgtcgtgggaaccgccctgatcaaaaagtaccctaagctggaaagcgagttcgtgtacggcgactacaaggtgtacgacgtgcggaagatgatcgccaagagcgagcaggaaatcggcaaggctaccgccaagtacttcttctacagcaacatcatgaactttttcaagaccgagattaccctggccaacggcgagatccggaagcggcctctgatcgagacaaacggcgaaaccggggagatcgtgtgggataagggccgggattttgccaccgtgcggaaagtgctgagcatgccccaagtgaatatcgtgaaaaagaccgaggtgcagacaggcggcttcagcaaagagtctatcctgcccaagaggaacagcgataagctgatcgccagaaagaaggactgggaccctaagaagtacggcggcttcgacagccccaccgtggcctattctgtgctggtggtggccaaagtggaaaagggcaagtccaagaaactgaagagtgtgaaagagctgctggggatcaccatcatggaaagaagcagcttcgagaagaatcccatcgactttctggaagccaagggctacaaagaagtgaaaaaggacctgatcatcaagctgcctaagtactccctgttcgagctggaaaacggccggaagagaatgctggcctctgccggcgaactgcagaagggaaacgaactggccctgccctccaaatatgtgaacttcctgtacctggccagccactatgagaagctgaagggctcccccgaggataatgagcagaaacagctgtttgtggaacagcacaagcactacctggacgagatcatcgagcagatcagcgagttctccaagagagtgatcctggccgacgctaatctggacaaagtgctgtccgcctacaacaagcaccgggataagcccatcagagagcaggccgagaatatcatccacctgtttaccctgaccaatctgggagcccctgccgccttcaagtactttgacaccaccatcgaccggaagaggtacaccagcaccaaagaggtgctggacgccaccctgatccaccagagcatcaccggcctgtacgagacacggatcgacctgtctcagctgggaggtgactctggaggatctagcggaggatcctctggcagcgagacaccaggaacaagcgagtcagcaacaccagagagcagtggcggcagcagcggcggcagcagcaccctaaatatagaagatgagtatcggctacatgagacctcaaaagagccagatgtttctctagggtccacatggctgtctgattttcctcaggcctgggcggaaaccgggggcatgggactggcagttcgccaagctcctctgatcatacctctgaaagcaacctctacccccgtgtccataaaacaataccccatgtcacaagaagccagactggggatcaagccccacatacagagactgttggaccagggaatactggtaccctgccagtccccctggaacacgcccctgctacccgttaagaaaccagggactaatgattataggcctgtccaggatctgagagaagtcaacaagcgggtggaagacatccaccccaccgtgcccaacccttacaacctcttgagcgggctcccaccgtcccaccagtggtacactgtgcttgatttaaaggatgcctttttctgcctgagactccaccccaccagtcagcctctcttcgcctttgagtggagagatccagagatgggaatctcaggacaattgacctggaccagactcccacagggtttcaaaaacagtcccaccctgtttaatgaggcactgcacagagacctagcagacttccggatccagcacccagacttgatcctgctacagtacgtggatgacttactgctggccgccacttctgagctagactgccaacaaggtactcgggccctgttacaaaccctagggaacctcgggtatcgggcctcggccaagaaagcccaaatttgccagaaacaggtcaagtatctggggtatcttctaaaagagggtcagagatggctgactgaggccagaaaagagactgtgatggggcagcctactccgaagacccctcgacaactaagggagttcctagggaaggcaggcttctgtcgcctcttcatccctgggtttgcagaaatggcagcccccctgtaccctctcaccaaaccggggactctgtttaattggggcccagaccaacaaaaggcctatcaagaaatcaagcaagctcttctaactgccccagccctggggttgccagatttgactaagccctttgaactctttgtcgacgagaagcagggctacgccaaaggtgtcctaacgcaaaaactgggaccttggcgtcggccggtggcctacctgtccaaaaagctagacccagtagcagctgggtggcccccttgcctacggatggtagcagccattgccgtactgacaaaggatgcaggcaagctaaccatgggacagccactagtcattctggccccccatgcagtagaggcactagtcaaacaaccccccgaccgctggctttccaacgcccggatgactcactatcaggccttgcttttggacacggaccgggtccagttcggaccggtggtagccctgaacccggctacgctgctcccactgcctgaggaagggctgcaacacaactgccttgatatcctggccgaagcccacggaacccgacccgacctaacggaccagccgctcccagacgccgaccacacctggtacacggatggaagcagtctcttacaagagggacagcgtaaggcgggagctgcggtgaccaccgagaccgaggtaatctgggctaaagccctgccagccgggacatccgctcagcgggctgaactgatagcactcacccaggccctaaagatggcagaaggtaagaagctaaatgtttatactgatagccgttatgcttttgctactgcccatatccatggagaaatatacagaaggcgtgggtggctcacatcagaaggcaaagagatcaaaaataaagacgagatcttggccctactaaaagccctctttctgcccaaaagacttagcataatccattgtccaggacatcaaaagggacacagcgccgaggctagaggcaaccggatggctgaccaagcggcccgaaaggcagccatcacagagactccagacacctctaccctcctcatagaaaattcatcaccctctggcggctcaaaaagaaccgccgacggcagcgaattcgagcccaagaagaagaggaaagtctaaccggtcatcatcaccatcaccattgagttttacccctacgacgtgcccgactacgcctaataactcgagcatgcatctagagggccctattctatagtgtcacctaaatgctagagctcgctgatcagcctcgactgtgccttctagttgccagccatctgttgtttgcccctcccccgtgccttccttgaccctggaaggtgccactcccactgtcctttcctaataaaatgaggaaattgcatcgcattgtctgagtaggtgtcattctattctggggggtggggtggggcaggacagcaagggggaggattgggaagacaatagcaggcatgctggggaggatctgcgatcgctccggtgcccgtcagtgggcagagcgcacatcgcccacagtccccgagaagttggggggaggggtcggcaattgaacgggtgcctagagaaggtggcgcggggtaaactgggaaagtgatgtcgtgtactggctccgcctttttcccgagggtgggggagaaccgtatataagtgcagtagtcgccgtgaacgttctttttcgcaacgggtttgccgccagaacacagctgaagcttcgaggggctcgcatctctccttcacgcgcccgccgccctacctgaggccgccatccacgccggttgagtcgcgttctgccgcctcccgcctgtggtgcctcctgaactgcgtccgccgtctaggtaagtttaaagctcaggtcgagaccgggcctttgtccggcgctcccttggagcctacctagactcagccggctctccacgctttgcctgaccctgcttgctcaactctacgtctttgtttcgttttctgttctgcgccgttacagatccaagctgtgaccggcgcctacatgaccgagtacaagcccacggtgcgcctcgccacccgcgacgacgtccccagggccgtacgcaccctcgccgccgcgttcgccgactaccccgccacgcgccacaccgtcgatccagaccgccacatcgagcgggtcaccgagctgcaagaactcttcctcacgcgcgtcgggctcgacatcggcaaggtgtgggtcgcggacgacggcgccgcggtggcggtctggaccacgccggagagcgtcgaagcgggggcggtgttcgccgagatcggcccgcgcatggccgagttgagcggttcccggctggccgcgcagcaacagatggaaggtctcctggcgccgcaccggcccaaggagcccgcgtggttcctggccaccgtcggcgtctcgcccgaccaccagggcaagggtctgggcagcgccgtcgtgctccccggagtggaggcggccgagcgcgccggggtgcccgccttcctggagacctccgcgccccgcaacctccccttctacgagcggctcggcttcaccgtcaccgccgacgtcgaggtgcccgaaggaccgcgcacctggtgcatgacccgcaagcccggtgcctgagctagaagctcgctttcttgctgtccaatttctattaaaggttcctttgttccctaagtccaactactaaactgggggatattatgaagggccttgagcatctggattctgcctaataaaaaacatttattttcattgcaatgatgtatttaaattatttctgaatattttactaaaaagggaatgtgggaggtcagtgcatttaaaacataaagaaatgaagagctagttcaaaccttgggaaaatacactatatcttaaactccatgaaagaaggtgaggctgcaaacagctaatgcacattggcaacagcccctgatgcctatgccttattcatccctcagaaaaggattcaagtagaggcttgatttggaggttaaagttttgctatgctgtattttagaattccataccacatttgtagaggttttacttgctttaaaaaacctcccacacctccccctgaacctgaaacataaaatgaatgcaattgttgttgttttaccaatgcttaatcagtgaggcacctatctcagcgatctgtctatttcgttcatccatagttgcctgactccccgtcgtgtagataactacgatacgggagggcttaccatctggccccagtgctgcaatgataccgcgagacccacgctcaccggctccagatttatcagcaataaaccagccagccggaagggccgagcgcagaagtggtcctgcaactttatccgcctccatccagtctattaattgttgccgggaagctagagtaagtagttcgccagttaatagtttgcgcaacgttgttgccattgctacaggcatcgtggtgtcacgctcgtcgtttggtatggcttcattcagctccggttcccaacgatcaaggcgagttacatgatcccccatgttgtgcaaaaaagcggttagctccttcggtcctccgatcgttgtcagaagtaagttggccgcagtgttatcactcatggttatggcagcactgcataattctcttactgtcatgccatccgtaagatgcttttctgtgactggtgagtactcaaccaagtcattctgagaatagtgtatgcggcgaccgagttgctcttgcccggcgtcaatacgggataataccgcgccacatagcagaactttaaaagtgctcatcattggaaaacgttcttcggggcgaaaactctcaaggatcttaccgctgttgagatccagttcgatgtaacccactcgtgcacccaactgatcttcagcatcttttactttcaccagcgtttctgggtgagcaaaaacaggaaggcaaaatgccgcaaaaaagggaataagggcgacacggaaatgttgaatactcatactcttcctttttcaatattattgaagcatttatcagggttattgtctcatgagcggatacatatttgaatgtatttagaaaaataaacaaataggggttccgcgaacttgtttattgcagcttataatggttacaaataaagcaatagcatcacaaatttcacaaataaagcatttttttcactgcattctagttgtggtttgtccaaactcatcaatgtatcttatcatgtctggccagctagccaacaagctcgtcatcgctttgcagaagagcagagaggatatgctcatcgtctaaagaactacccattttattatatattagtcacgatatctataacaagaaaatatatatataataagttatcacgtaagtagaacatgaaataacaatataattatcgtatgagttaaatcttaaaagtcacgtaaaagataatcatgcgtcattttgactcacgcggtcgttatagttcaaaatcagtgacacttaccgcattgacaagcacgcctcacgggagctccaagcggcgactgagatgtcctaaatgcacagcgacggattcgcgctatttagaaagagagagcaatatttcaagaatgcatgcgtcaattttacgcagactatctttctagggttaaaaaagatttgcgctttactcgacctaaactttaaacacgtcatagaatcttcgtttgacaaaaaccacattgtggccaagctgtgtgacgcgacgcgcgctaaagaatggcaaaccaagtcgcgcgaggtacccagcttttgttccctttagtgagggttaattccgagcttggcgtaatcatggtcatagctgtttcctgtgtgaaattgttatccgctcacaattccacacaacatacgagccggaagcataaagtgtaaagcctggggtgcctaatgagtgagctaactcacattaattgcgttgcgctcactgcccgctttccagtcgggaaacctgtcgtgccagctgcattaatgaatcggccaacgcgcggggagaggcggtttgcgtattgggcgctcttccgcttcctcgctcactgactcgctgcgctcggtcgttcggctgcggcgagcggtatcagctcactcaaaggcggtaatacggttatccacagaatcaggggataacgcaggaaagaacatgtgagcaaaaggccagcaaaaggccaggaaccgtaaaaaggccgcgttgctggcgtttttccataggctccgcccccctgacgagcatcacaaaaatcgacgctcaagtcagaggtggcgaaacccgacaggactataaagataccaggcgtttccccctggaagctccctcgtgcgctctcctgttccgaccctgccgcttaccggatacctgtccgcctttctcccttcgggaagcgtggcgctttctcatagctcacgctgtaggtatctcagttcggtgtaggtcgttcgctccaagctgggctgtgtgcacgaaccccccgttcagcccgaccgctgcgccttatccggtaactatcgtcttgagtccaacccggtaagacacgacttatcgccactggcagcagccactggtaacaggattagcagagcgaggtatgtaggcggtgctacagagttcttgaagtggtggcctaactacggctacactagaaggacagtatttggtatctgcgctctgctgaagccagttaccttcggaaaaagagttggtagctcttgatccggcaaacaaaccaccgctggtagcggtggtttttttgtttgcaagcagcagattacgcgcagaaaaaaaggatctcaagaagatcctttgatcttttctacggggtctgacgctcagtggaacgaaaactcacgttaagggattttggtcatgattaaccctagaaagataatcatattgtgacgtacgttaaagataatcatgcgtaaaattgacgcatgtgttttatcggtctgtatatcgaggtttatttattaatttgaatagatattaagttttattatatttacacttacatactaataataaattcaacaaacaatttatttatgtttatttatttattaaaaaaaaacaaaaactcaaaatttcttctataaagtaacaaaacttttaaacattctctcttttacaaaaataaacttattttgtactttaaaaacagtcatgttgtattataaaataagtaattagcttaacctatacataatagaaacaaattatacttattagtcagtcagaaacaactttggcacatatcaatattatgctctcgttaattaa

SEQ ID NO: 152 - DNA, 12675 bp, synthetic construct
  source 1..12675: mol_type = other DNA
cgatgtacgggccagatatacgcgcaatgtcaacgcgtatatctaaaaaattctagttggtttaacgcgtaactagatagaaccgcgnnnnnnnnnnnnnnnnnnnnnnnnnnnnnngcaccgactcggtgccactttttcaagttgataacggactagccttattttaacttgctatttctagctctaaaacnnnnnnnnnnnnnnnnnnncggtgtttcgtcctttccacaagatatataaagccaagaaatcgaaatactttcaagttacggtaagcatatgatagtccattttaaaacataattttaaaactgcaaactacccaagaaattattactttctacgtcacgtattttgtactaatatctttgtgtttacagtcaaattaattccaattatctctctaacagccttgtatcgtatatgcaaatatgaaggaatcatgggaaataggccctccgcgttgacattgattattgactagttattaatagtaatcaattacggggtcattagttcatagcccatatatggagttccgcgttacataacttacggtaaatggcccgcctggctgaccgcccaacgacccccgcccattgacgtcaataatgacgtatgttcccatagtaacgccaatagggactttccattgacgtcaatgggtggagtatttacggtaaactgcccacttggcagtacatcaagtgtatcatatgccaagtacgccccctattgacgtcaatgacggtaaatggcccgcctggcattatgcccagtacatgaccttatgggactttcctacttggcagtacatctacgtattagtcatcgctattaccatggtgatgcggttttggcagtacatcaatgggcgtggatagcggtttgactcacggggatttccaagtctccaccccattgacgtcaatgggagtttgttttggcaccaaaatcaacgggactttccaaaatgtcgtaacaactccgccccattgacgcaaatgggcggtaggcgtgtacggtgggaggtctatataagcagagctggtttagtgaaccgtcagatccgctagagatccgcggccgctaatacgactcactatagggagagccgccaccatgaaacggacagccgacggaagcgagttcgagtcaccaaagaagaagcggaaagtcgacaagaagtacagcatcggcctggacatcggcaccaactctgtgggctgggccgtgatcaccgacgagtacaaggtgcccagcaagaaattcaaggtgctgggcaacaccgaccggcacagcatcaagaagaacctgatcggagccctgctgttcgacagcggcgaaacagccgaggccacccggctgaagagaaccgccagaagaagatacaccagacggaagaaccggatctgctatctgcaagagatcttcagcaacgagatggccaaggtggacgacagcttcttccacagactggaagagtccttcctggtggaagaggataagaagcacgagcggcaccccatcttcggcaacatcgtggacgaggtggcctaccacgagaagtaccccaccatctaccacctgagaaagaaactggtggacagcaccgacaaggccgacctgcggctgatctatctggccctggcccacatgatcaagttccggggccacttcctgatcgagggcgacctgaaccccgacaacagcgacgtggacaagctgttcatccagctggtgcagacctacaaccagctgttcgaggaaaaccccatcaacgccagcggcgtggacgccaaggccatcctgtctgccagactgagcaagagcagaaagctggaaaatctgatcgcccagctgcccggcgagaagaagaatggcctgttcggaaacctgattgccctgagcctgggcctgacccccaacttcaagagcaacttcgacctggccgaggatgccaaactgcagctgagcaaggacacctacgacgacgacctggacaacctgctggcccagatcggcgaccagtacgccgacctgtttctggccgccaagaacctgtccgacgccatcctgctgagcgacatcctgagagtgaacaccgagatcaccaaggcccccctgagcgcctctatgatcaagagatacgacgagcaccaccaggacctgaccctgctgaaagctctcgtgcggcagcagctgcctgagaagtacaaagagattttcttcgaccagagcaagaacggctacgccggctacattgacggcggagccagccaggaagagttctacaagttcatcaagcccatcctggaaaagatggacggcaccgaggaactgctcgtgaagctgaagagagaggacctgctgcggaagcagcggaccttcgacaacggcagcatcccccaccagatccacctgggagagctgcacgccattctgcggcggcaggaagatttttacccattcctgaaggacaaccgggaaaagatcgagaagatcctgaccttccgcatcccctactacgtgggccctctggccaggggaaacagcagattcgcctggatgaccagaaagagcgaggaaaccatcaccccctggaacttcgaggaagtggtggacaagggcgcttccgcccagagcttcatcgagcggatgaccaacttcgataagaacctgcccaacgagaaggtgctgcccaagcacagcctgctgtacgagtacttcaccgtgtataacgagctgaccaaagtgaaatacgtgaccgagggaatgagaaagcccgccttcctgagcggcgagcagaaaaaggccatcgtggacctgctgttcaagaccaaccggaaagtgaccgtgaagcagctgaaagaggactacttcaagaaaatcgagtgcttcgactccgtggaaatctccggcgtggaagatcggttcaacgcctccctgggcacataccacgatctgctgaaaattatcaaggacaaggacttcctggacaatgaggaaaacgaggacattctggaagatatcgtgctgaccctgacactgtttgaggacagagagatgatcgaggaacggctgaaaacctatgcccacctgttcgacgacaaagtgatgaagcagctgaagcggcggagatacaccggctggggcaggctgagccggaagctgatcaacggcatccgggacaagcagtccggcaagacaatcctggatttcctgaagtccgacggcttcgccaacagaaacttcatgcagctgatccacgacgacagcctgacctttaaagaggacatccagaaagcccaggtgtccggccagggcgatagcctgcacgagcacattgccaatctggccggcagccccgccattaagaagggcatcctgcagacagtgaaggtggtggacgagctcgtgaaagtgatgggccggcacaagcccgagaacatcgtgatcgaaatggccagagagaaccagaccacccagaagggacagaagaacagccgcgagagaatgaagcggatcgaagagggcatcaaagagctgggcagccagatcctgaaagaacaccccgtggaaaacacccagctgcagaacgagaagctgtacctgtactacctgcagaatgggcgggatatgtacgtggaccaggaactggacatcaaccggctgtccgactacgatgtggaccacatcgtgcctcagagctttctgaaggacgactccatcgacaacaaggtgctgaccagaagcgacaagaaccggggcaagagcgacaacgtgccctccgaagaggtcgtgaagaagatgaagaactactggcggcagctgctgaacgccaagctgattacccagagaaagttcgacaatctgaccaaggccgagagaggcggcctgagcgaactggataaggccggcttcatcaagagacagctggtggaaacccggcagatcacaaagcacgtggcacagatcctggactcccggatgaacactaagtacgacgagaatgacaagctgatccgggaagtgaaagtgatcaccctgaagtccaagctggtgtccgatttccggaaggatttccagttttacaaagtgcgcgagatcaacaactaccaccacgcccacgacgcctacctgaacgccgtcgtgggaaccgccctgatcaaaaagtaccctaagctggaaagcgagttcgtgtacggcgactacaaggtgtacgacgtgcggaagatgatcgccaagagcgagcaggaaatcggcaaggctaccgccaagtacttcttctacagcaacatcatgaactttttcaagaccgagattaccctggccaacggcgagatccggaagcggcctctgatcgagacaaacggcgaaaccggggagatcgtgtgggataagggccgggattttgccaccgtgcggaaagtgctgagcatgccccaagtgaatatcgtgaaaaagaccgaggtgcagacaggcggcttcagcaaagagtctatcctgcccaagaggaacagcgataagctgatcgccagaaagaaggactgggaccctaagaagtacggcggcttcgacagccccaccgtggcctattctgtgctggtggtggccaaagtggaaaagggcaagtccaagaaactgaagagtgtgaaagagctgctggggatcaccatcatggaaagaagcagcttcgagaagaatcccatcgactttctggaagccaagggctacaaagaagtgaaaaaggacctgatcatcaagctgcctaagtactccctgttcgagctggaaaacggccggaagagaatgctggcctctgccggcgaactgcagaagggaaacgaactggccctgccctccaaatatgtgaacttcctgtacctggccagccactatgagaagctgaagggctcccccgaggataatgagcagaaacagctgtttgtggaacagcacaagcactacctggacgagatcatcgagcagatcagcgagttctccaagagagtgatcctggccgacgctaatctggacaaagtgctgtccgcctacaacaagcaccgggataagcccatcagagagcaggccgagaatatcatccacctgtttaccctgaccaatctgggagcccctgccgccttcaagtactttgacaccaccatcgaccggaagaggtacaccagcaccaaagaggtgctggacgccaccctgatccaccagagcatcaccggcctgtacgagacacggatcgacctgtctcagctgggaggtgactccggcggaagctctggtggcagcaagcggaccgccgacggctctgaattcgagagccctaagaagaaaagaaaggtgagcggaggctctagcggcggaagcaccctgaacattgaagacgagtatagactgcatgaaacaagcaaggaacccgacgtgtccctgggctccacctggctgtccgactttccccaggcctgggccgagacaggaggaatgggcctggccgtgcggcaggcacccctgatcatccctctgaaggccacctctacacccgtgagcatcaagcagtaccctatgtctcaggaggccagactgggcatcaagcctcacatccagaggctgctggaccagggcatcctggtgccatgccagagcccctggaacacaccactgctgcccgtgaagaagccaggcaccaatgactatagacccgtgcaggatctgagagaggtgaacaagagggtggaggatatccaccccaccgtgcccaacccttacaatctgctgtccggcctgcccccttctcaccagtggtatacagtgctggacctgaaggatgccttcttttgtctgagactgcaccctaccagccagccactgttcgcctttgagtggagggaccctgagatgggcatctctggccagctgacctggacacgcctgcctcagggcttcaagaatagcccaacactgtttaacgaggccctgcaccgcgacctggcagatttccggatccagcacccagatctgatcctgctgcagtacgtggacgatctgctgctggccgccaccagcgagctggattgccagcagggaacacgcgccctgctgcagaccctgggaaacctgggatatagggcatccgccaagaaggcccagatctgtcagaagcaggtgaagtacctgggctatctgctgaaggagggccagagatggctgacagaggccaggaaggagacagtgatgggccagccaacacccaagaccccaagacagctgagggagttcctgggcaaagcaggattttgcaggctgttcatcccaggattcgcagagatggcagcacctctgtacccactgaccaagccgggcaccctgtttaattggggccctgaccagcagaaggcctatcaggagatcaagcaggccctgctgacagcaccagccctgggcctgccagacctgaccaagcctttcgagctgtttgtggatgagaagcagggctacgccaagggcgtgctgacccagaagctgggaccatggagacggcccgtggcctatctgtccaagaagctggacccagtggcagcaggatggccaccatgcctgaggatggtggcagcaatcgccgtgctgacaaaggatgccggcaagctgaccatgggacagccactggtcatcctggcaccacacgcagtggaggccctggtgaagcagcctccagatcgctggctgtctaacgcccggatgacacactaccaggccctgctgctggacaccgatcgcgtgcagtttggccctgtggtggccctgaatccagccaccctgctgcctctgccagaggagggcctgcagcacaactgtctggacatcctggcagaggcacacggaacaaggccagacctgaccgatcagcccctgcctgacgccgatcacacatggtataccgatggaagctccctgctgcaggagggccagaggaaggcaggagcagcagtgaccacagagacagaagtgatctgggccaaggccctgccagcaggcacatccgcccagcgggccgagctgatcgccctgacccaggccctgaagatggccgagggcaagaagctgaacgtgtacacagactccagatatgccttcgccaccgcacacatccacggagagatctacaggcgccggggctggctgacctctgagggcaaggagatcaagaacaaggatgagatcctggccctgctgaaggccctgtttctgcccaagcggctgagcatcatccactgtcctggacaccagaagggacactccgccgaggcaaggggcaatcggatggccgaccaggccgccagaaaggctgctattactgaaactcccgacacttccactctgctgattgaaaactcctccccttctggcggctcaaaaagaaccgccgacggcagcgaattcgagtctcccaagaagaagaggaaagtcggctctggccctgccgctaagagagtgaagctggactaaccggtcatcatcaccatcaccattgagttttacccctacgacgtgcccgactacgcctaataactcgagcatgcatctagagggccctattctatagtgtcacctaaatgctagagctcgctgatcagcctcgactgtgccttctagttgccagccatctgttgtttgcccctcccccgtgccttccttgaccctggaaggtgccactcccactgtcctttcctaataaaatgaggaaattgcatcgcattgtctgagtaggtgtcattctattctggggggtggggtggggcaggacagcaagggggaggattgggaagacaatagcaggcatgctggggaggatctgcgatcgctccggtgcccgtcagtgggcagagcgcacatcgcccacagtccccgagaagttggggggaggggtcggcaattgaacgggtgcctagagaaggtggcgcggggtaaactgggaaagtgatgtcgtgtactggctccgcctttttcccgagggtgggggagaaccgtatataagtgcagtagtcgccgtgaacgttctttttcgcaacgggtttgccgccagaacacagctgaagcttcgaggggctcgcatctctccttcacgcgcccgccgccctacctgaggccgccatccacgccggttgagtcgcgttctgccgcctcccgcctgtggtgcctcctgaactgcgtccgccgtctaggtaagtttaaagctcaggtcgagaccgggcctttgtccggcgctcccttggagcctacctagactcagccggctctccacgctttgcctgaccctgcttgctcaactctacgtctttgtttcgttttctgttctgcgccgttacagatccaagctgtgaccggcgcctacatgaccgagtacaagcccacggtgcgcctcgccacccgcgacgacgtccccagggccgtacgcaccctcgccgccgcgttcgccgactaccccgccacgcgccacaccgtcgatccagaccgccacatcgagcgggtcaccgagctgcaagaactcttcctcacgcgcgtcgggctcgacatcggcaaggtgtgggtcgcggacgacggcgccgcggtggcggtctggaccacgccggagagcgtcgaagcgggggcggtgttcgccgagatcggcccgcgcatggccgagttgagcggttcccggctggccgcgcagcaacagatggaaggtctcctggcgccgcaccggcccaaggagcccgcgtggttcctggccaccgtcggcgtctcgcccgaccaccagggcaagggtctgggcagcgccgtcgtgctccccggagtggaggcggccgagcgcgccggggtgcccgccttcctggagacctccgcgccccgcaacctccccttctacgagcggctcggcttcaccgtcaccgccgacgtcgaggtgcccgaaggaccgcgcacctggtgcatgacccgcaagcccggtgcctgagctagaagctcgctttcttgctgtccaatttctattaaaggttcctttgttccctaagtccaactactaaactgggggatattatgaagggccttgagcatctggattctgcctaataaaaaacatttattttcattgcaatgatgtatttaaattatttctgaatattttactaaaaagggaatgtgggaggtcagtgcatttaaaacataaagaaatgaagagctagttcaaaccttgggaaaatacactatatcttaaactccatgaaagaaggtgaggctgcaaacagctaatgcacattggcaacagcccctgatgcctatgccttattcatccctcagaaaaggattcaagtagaggcttgatttggaggttaaagttttgctatgctgtattttagaattccataccacatttgtagaggttttacttgctttaaaaaacctcccacacctccccctgaacctgaaacataaaatgaatgcaattgttgttgttttaccaatgcttaatcagtgaggcacctatctcagcgatctgtctatttcgttcatccatagttgcctgactccccgtcgtgtagataactacgatacgggagggcttaccatctggccccagtgctgcaatgataccgcgagacccacgctcaccggctccagatttatcagcaataaaccagccagccggaagggccgagcgcagaagtggtcctgcaactttatccgcctccatccagtctattaattgttgccgggaagctagagtaagtagttcgccagttaatagtttgcgcaacgttgttgccattgctacaggcatcgtggtgtcacgctcgtcgtttggtatggcttcattcagctccggttcccaacgatcaaggcgagttacatgatcccccatgttgtgcaaaaaagcggttagctccttcggtcctccgatcgttgtcagaagtaagttggccgcagtgttatcactcatggttatggcagcactgcataattctcttactgtcatgccatccgtaagatgcttttctgtgactggtgagtactcaaccaagtcattctgagaatagtgtatgcggcgaccgagttgctcttgcccggcgtcaatacgggataataccgcgccacatagcagaactttaaaagtgctcatcattggaaaacgttcttcggggcgaaaactctcaaggatcttaccgctgttgagatccagttcgatgtaacccactcgtgcacccaactgatcttcagcatcttttactttcaccagcgtttctgggtgagcaaaaacaggaaggcaaaatgccgcaaaaaagggaataagggcgacacggaaatgttgaatactcatactcttcctttttcaatattattgaagcatttatcagggttattgtctcatgagcggatacatatttgaatgtatttagaaaaataaacaaataggggttccgcgaacttgtttattgcagcttataatggttacaaataaagcaatagcatcacaaatttcacaaataaagcatttttttcactgcattctagttgtggtttgtccaaactcatcaatgtatcttatcatgtctggccagctagccaacaagctcgtcatcgctttgcagaagagcagagaggatatgctcatcgtctaaagaactacccattttattatatattagtcacgatatctataacaagaaaatatatatataataagttatcacgtaagtagaacatgaaataacaatataattatcgtatgagttaaatcttaaaagtcacgtaaaagataatcatgcgtcattttgactcacgcggtcgttatagttcaaaatcagtgacacttaccgcattgacaagcacgcctcacgggagctccaagcggcgactgagatgtcctaaatgcacagcgacggattcgcgctatttagaaagagagagcaatatttcaagaatgcatgcgtcaattttacgcagactatctttctagggttaaaaaagatttgcgctttactcgacctaaactttaaacacgtcatagaatcttcgtttgacaaaaaccacattgtggccaagctgtgtgacgcgacgcgcgctaaagaatggcaaaccaagtcgcgcgaggtacccagcttttgttccctttagtgagggttaattccgagcttggcgtaatcatggtcatagctgtttcctgtgtgaaattgttatccgctcacaattccacacaacatacgagccggaagcataaagtgtaaagcctggggtgcctaatgagtgagctaactcacattaattgcgttgcgctcactgcccgctttccagtcgggaaacctgtcgtgccagctgcattaatgaatcggccaacgcgcggggagaggcggtttgcgtattgggcgctcttccgcttcctcgctcactgactcgctgcgctcggtcgttcggctgcggcgagcggtatcagctcactcaaaggcggtaatacggttatccacagaatcaggggataacgcaggaaagaacatgtgagcaaaaggccagcaaaaggccaggaaccgtaaaaaggccgcgttgctggcgtttttccataggctccgcccccctgacgagcatcacaaaaatcgacgctcaagtcagaggtggcgaaacccgacaggactataaagataccaggcgtttccccctggaagctccctcgtgcgctctcctgttccgaccctgccgcttaccggatacctgtccgcctttctcccttcgggaagcgtggcgctttctcatagctcacgctgtaggtatctcagttcggtgtaggtcgttcgctccaagctgggctgtgtgcacgaaccccccgttcagcccgaccgctgcgccttatccggtaactatcgtcttgagtccaacccggtaagacacgacttatcgccactggcagcagccactggtaacaggattagcagagcgaggtatgtaggcggtgctacagagttcttgaagtggtggcctaactacggctacactagaaggacagtatttggtatctgcgctctgctgaagccagttaccttcggaaaaagagttggtagctcttgatccggcaaacaaaccaccgctggtagcggtggtttttttgtttgcaagcagcagattacgcgcagaaaaaaaggatctcaagaagatcctttgatcttttctacggggtctgacgctcagtggaacgaaaactcacgttaagggattttggtcatgattaaccctagaaagataatcatattgtgacgtacgttaaagataatcatgcgtaaaattgacgcatgtgttttatcggtctgtatatcgaggtttatttattaatttgaatagatattaagttttattatatttacacttacatactaataataaattcaacaaacaatttatttatgtttatttatttattaaaaaaaaacaaaaactcaaaatttcttctataaagtaacaaaacttttaaacattctctcttttacaaaaataaacttattttgtactttaaaaacagtcatgttgtattataaaataagtaattagcttaacctatacataatagaaacaaattatacttattagtcagtcagaaacaactttggcacatatcaatattatgctctcgttaattaa

SEQ ID NO: 153 - DNA, 38 bp, synthetic construct
  source 1..38: mol_type = other DNA
cgcagggctctgcggctggagggggtggggttgctgtt

SEQ ID NO: 154 - DNA, 39 bp, synthetic construct
  source 1..39: mol_type = other DNA
cgcagggctctgcggctggaggtgtaaggggttgctgtt

SEQ ID NO: 155 - DNA, 29 bp, synthetic construct
  source 1..29: mol_type = other DNA
ggctggaggtgtaaggggttaagcaccga

SEQ ID NO: 156 - DNA, 38 bp, synthetic construct
  source 1..38: mol_type = other DNA
aattgaggactgcggctgggggtggtggctcacacctg

SEQ ID NO: 157 - DNA, 38 bp, synthetic construct
  source 1..38: mol_type = other DNA
aattgaggactgcggctgggggttggggttcacacctg

SEQ ID NO: 158 - DNA, 26 bp, synthetic construct
  source 1..26: mol_type = other DNA
ggctggaggttggggttaagcaccga

SEQ ID NO: 159 - DNA, 38 bp, synthetic construct
  source 1..38: mol_type = other DNA
cttggtgcactgcggccggaggaggtggaggatggaaa

SEQ ID NO: 160 - DNA, 38 bp, synthetic construct
  source 1..38: mol_type = other DNA
cttggtgcactgcggccggaggttggggaggatggaaa

SEQ ID NO: 161 - DNA, 26 bp, synthetic construct
  source 1..26: mol_type = other DNA
ggctggaggttggggttaagcaccga

SEQ ID NO: 162 - DNA, 38 bp, synthetic construct
  source 1..38: mol_type = other DNA
ggctgggcactgagggtggaggtgggggcagtcatctc

SEQ ID NO: 163 - DNA, 38 bp, synthetic construct
  source 1..38: mol_type = other DNA
ggctgggcactgagggtggaggttggggcagtcatctc

SEQ ID NO: 164 - DNA, 26 bp, synthetic construct
  source 1..26: mol_type = other DNA
ggctggaggttggggttaagcaccga

SEQ ID NO: 165 - DNA, 37 bp, synthetic construct
  source 1..37: mol_type = other DNA
ctgagggcaatgcggctggaggcggaggcaacggcgg

SEQ ID NO: 166 - DNA, 38 bp, synthetic construct
  source 1..38: mol_type = other DNA
ctgagggcaatgcggctggaggttggggttaacggcgg

SEQ ID NO: 167 - DNA, 26 bp, synthetic construct
  source 1..26: mol_type = other DNA
ggctggaggttggggttaagcaccga

SEQ ID NO: 168 - DNA, 38 bp, synthetic construct
  source 1..38: mol_type = other DNA
tgccgggcacgacggctggaggtggggggttgggagtg

SEQ ID NO: 169 - DNA, 37 bp, synthetic construct
  source 1..37: mol_type = other DNA
tgccgggcacgacggctggaggttggggttgggagtg

SEQ ID NO: 170 - DNA, 26 bp, synthetic construct
  source 1..26: mol_type = other DNA
ggctggaggttggggttaagcaccga

SEQ ID NO: 171 - DNA, 38 bp, synthetic construct
  source 1..38: mol_type = other DNA
acagcagctctgcggctggaggagggggagtggtgatg

SEQ ID NO: 172 - DNA, 38 bp, synthetic construct
  source 1..38: mol_type = other DNA
acagcagctctgcggctggaggttggggagtggtgatg

SEQ ID NO: 173 - DNA, 26 bp, synthetic construct
  source 1..26: mol_type = other DNA
ggctggaggttggggttaagcaccga

SEQ ID NO: 174 - DNA, 38 bp, synthetic construct
  source 1..38: mol_type = other DNA
gtgaaggcactggggttggaggtgggggctcgggactc

SEQ ID NO: 175 - DNA, 38 bp, synthetic construct
  source 1..38: mol_type = other DNA
gtgaaggcactggggttggaggttggggctcgggactc

SEQ ID NO: 176 - DNA, 26 bp, synthetic construct
  source 1..26: mol_type = other DNA
ggctggaggttggggttaagcaccga

SEQ ID NO: 177 - DNA, 38 bp, synthetic construct; identical to SEQ ID NO: 156
  source 1..38: mol_type = other DNA

SEQ ID NO: 178 - DNA, 38 bp, synthetic construct; identical to SEQ ID NO: 157
  source 1..38: mol_type = other DNA

SEQ ID NO: 179 - DNA, 26 bp, synthetic construct
  source 1..26: mol_type = other DNA
ggctggaggttggggttaagcaccga

SEQ ID NO: 180 - DNA, 38 bp, synthetic construct; identical to SEQ ID NO: 159
  source 1..38: mol_type = other DNA

SEQ ID NO: 181 - DNA, 38 bp, synthetic construct; identical to SEQ ID NO: 160
  source 1..38: mol_type = other DNA

SEQ ID NO: 182 - DNA, 26 bp, synthetic construct
  source 1..26: mol_type = other DNA
ggctggaggttggggttaagcaccga

SEQ ID NO: 183 - DNA, 38 bp, synthetic construct
  source 1..38: mol_type = other DNA
ggcggggcactgggctggaggcgggggataaggggacc

SEQ ID NO: 184 - DNA, 38 bp, synthetic construct
  source 1..38: mol_type = other DNA
ggcggggcactgggctggaggttggggataaggggacc

SEQ ID NO: 185 - DNA, 26 bp, synthetic construct
  source 1..26: mol_type = other DNA
ggctggaggttggggttaagcaccga

SEQ ID NO: 186 - DNA, 41 bp, synthetic construct
  source 1..41: mol_type = other DNA
gacaccatggtgcatctgactcctgaggagaagactgctgt

SEQ ID NO: 187 - DNA, 41 bp, synthetic construct
  source 1..41: mol_type = other DNA
gacaccatggtgcatctgactcctgtggagaagtctgctgt

SEQ ID NO: 188 - DNA, 34 bp, synthetic construct
  source 1..34: mol_type = other DNA
gtgcacctgactcctgtggagaagtctgcaccga

SEQ ID NO: 189 - DNA, 40 bp, synthetic construct
  source 1..40: mol_type = other DNA
ctgagggcaatgcggctggaggcggaggcaacggcggctg

SEQ ID NO: 190 - DNA, 39 bp, synthetic construct
  source 1..39: mol_type = other DNA
ctgagggcaatgcggctggaggtgtaaggggttaagctg

SEQ ID NO: 191 - DNA, 29 bp, synthetic construct
  source 1..29: mol_type = other DNA
ggctggaggtgtaaggggttaagcaccga

SEQ ID NO: 192 - DNA, 38 bp, synthetic construct; identical to SEQ ID NO: 168
  source 1..38: mol_type = other DNA

SEQ ID NO: 193 - DNA, 40 bp, synthetic construct
  source 1..40: mol_type = other DNA
tgccgggcacgacggctggaggtgtaaggggttgggagtg

SEQ ID NO: 194 - DNA, 29 bp, synthetic construct
  source 1..29: mol_type = other DNA
ggctggaggtgtaaggggttaagcaccga

SEQ ID NO: 195 - DNA, 38 bp, synthetic construct; identical to SEQ ID NO: 153
  source 1..38: mol_type = other DNA

SEQ ID NO: 196 - DNA, 39 bp, synthetic construct; identical to SEQ ID NO: 154
  source 1..39: mol_type = other DNA

SEQ ID NO: 197 - DNA, 29 bp, synthetic construct
  source 1..29: mol_type = other DNA
ggctggaggtgtaaggggttaagcaccga

SEQ ID NO: 198 - DNA, 36 bp, synthetic construct
  source 1..36: mol_type = other DNA
acagcagctctgcggctggaggagggggagtggtga

SEQ ID NO: 199 - DNA, 37 bp, synthetic construct
  source 1..37: mol_type = other DNA
acagcagctctgcggctggaggtgtaaggggtggtta

SEQ ID NO: 200 - DNA, 29 bp, synthetic construct
  source 1..29: mol_type = other DNA
ggctggaggtgtaaggggttaagcaccga

SEQ ID NO: 201 - DNA, 37 bp, synthetic construct
  source 1..37: mol_type = other DNA
gtgaaggcactggggttggaggtgggggctcgggact

SEQ ID NO: 202 - DNA, 40 bp, synthetic construct
  source 1..40: mol_type = other DNA
gtgaaggcactggggttggaggtgtaaggggttcgggact

SEQ ID NO: 203 - DNA, 29 bp, synthetic construct
  source 1..29: mol_type = other DNA
ggctggaggtgtaaggggttaagcaccga

SEQ ID NO: 204 - DNA, 37 bp, synthetic construct
  source 1..37: mol_type = other DNA
ggcggggcactgggctggaggcgggggataaggggac

SEQ ID NO: 205 - DNA, 40 bp, synthetic construct
  source 1..40: mol_type = other DNA
ggcggggcactgggctggaggtgtaaggggttaaggggac

SEQ ID NO: 206 - DNA, 29 bp, synthetic construct
  source 1..29: mol_type = other DNA
ggctggaggtgtaaggggttaagcaccga

SEQ ID NO: 207 - DNA, 38 bp, synthetic construct; identical to SEQ ID NO: 153
  source 1..38: mol_type = other DNA

SEQ ID NO: 208 - DNA, 39 bp, synthetic construct; identical to SEQ ID NO: 154
  source 1..39: mol_type = other DNA

SEQ ID NO: 209 - DNA, 29 bp, synthetic construct
  source 1..29: mol_type = other DNA
ggctggaggtgtaaggggttaagcaccga

SEQ ID NO: 210 - DNA, 38 bp, synthetic construct; identical to SEQ ID NO: 168
  source 1..38: mol_type = other DNA

SEQ ID NO: 211 - DNA, 40 bp, synthetic construct; identical to SEQ ID NO: 193
  source 1..40: mol_type = other DNA

SEQ ID NO: 212 - DNA, 29 bp, synthetic construct
  source 1..29: mol_type = other DNA
ggctggaggtgtaaggggttaagcaccga

SEQ ID NO: 213 - DNA, 38 bp, synthetic construct; identical to SEQ ID NO: 171
  source 1..38: mol_type = other DNA

SEQ ID NO: 214 - DNA, 38 bp, synthetic construct; identical to SEQ ID NO: 172
  source 1..38: mol_type = other DNA

SEQ ID NO: 215 - DNA, 26 bp, synthetic construct
  source 1..26: mol_type = other DNA
ggctggaggttggggttaagcaccga

SEQ ID NO: 216 - DNA, 37 bp, synthetic construct; identical to SEQ ID NO: 165
  source 1..37: mol_type = other DNA

SEQ ID NO: 217 - DNA, 38 bp, synthetic construct; identical to SEQ ID NO: 166
  source 1..38: mol_type = other DNA

SEQ ID NO: 218 - DNA, 26 bp, synthetic construct
  source 1..26: mol_type = other DNA
ggctggaggttggggttaagcaccga

SEQ ID NO: 219 - DNA, 38 bp, synthetic construct; identical to SEQ ID NO: 153
  source 1..38: mol_type = other DNA

SEQ ID NO: 220 - DNA, 39 bp, synthetic construct; identical to SEQ ID NO: 154
  source 1..39: mol_type = other DNA

SEQ ID NO: 221 - DNA, 29 bp, synthetic construct
  source 1..29: mol_type = other DNA
ggctggaggtgtaaggggttaagcaccga

SEQ ID NO: 222 - DNA, 38 bp, synthetic construct; identical to SEQ ID NO: 156
  source 1..38: mol_type = other DNA

SEQ ID NO: 223 - DNA, 38 bp, synthetic construct
  source 1..38: mol_type = other DNA
aattgaggactgcggctgggggttggggctcacacctg

SEQ ID NO: 224 - DNA, 26 bp, synthetic construct
  source 1..26: mol_type = other DNA
ggctggaggttggggttaagcaccga

SEQ ID NO: 225 - DNA, 38 bp, synthetic construct; identical to SEQ ID NO: 162
  source 1..38: mol_type = other DNA

SEQ ID NO: 226 - DNA, 38 bp, synthetic construct; identical to SEQ ID NO: 163
  source 1..38: mol_type = other DNA

SEQ ID NO: 227 - DNA, 26 bp, synthetic construct
  source 1..26: mol_type = other DNA
ggctggaggttggggttaagcaccga

SEQ ID NO: 228 - DNA, 38 bp, synthetic construct
  source 1..38: mol_type = other DNA
accctggcactggggctgggggagggggtctaccttcc

SEQ ID NO: 229 - DNA, 38 bp, synthetic construct
  source 1..38: mol_type = other DNA
accctggcactggggctgggggttggggtctaccttcc

SEQ ID NO: 230 - DNA, 26 bp, synthetic construct
  source 1..26: mol_type = other DNA
ggctggaggttggggttaagcaccga

SEQ ID NO: 231 - DNA, 40 bp, synthetic construct
  source 1..40: mol_type = other DNA
tcttggatgtctggtgccagaaacaagggtgttattgaag

SEQ ID NO: 232 - DNA, 40 bp, synthetic construct
  source 1..40: mol_type = other DNA
tcttggatgtctggtgccagaaacaggcgtgttattgaag

SEQ ID NO: 233 - DNA, 31 bp, synthetic construct
  source 1..31: mol_type = other DNA
cctggtgccagaaacaggcgtgacgcaccga

SEQ ID NO: 234 - DNA, 43 bp, synthetic construct
  source 1..43: mol_type = other DNA
gcactcacggggcacctgactcctgaggcgacagccttcacct

SEQ ID NO: 235 - DNA, 42 bp, synthetic construct
  source 1..42: mol_type = other DNA
gcactcacggggcacctgactcctgtggagaagtctgcacct

SEQ ID NO: 236 - DNA, 34 bp, synthetic construct; identical to SEQ ID NO: 188
  source 1..34: mol_type = other DNA

SEQ ID NO: 237 - DNA, 40 bp, synthetic construct
  source 1..40: mol_type = other DNA
aaaaaaatgactacaggtcagatgagggctctgaatgcta

SEQ ID NO: 238 - DNA, 40 bp, synthetic construct
  source 1..40: mol_type = other DNA
aaaaaaatgactacaggtcagatgagtgctctgaatgcta

SEQ ID NO: 239 - DNA, 42 bp, synthetic construct
  source 1..42: mol_type = other DNA
tctgcaggccagatgagtgctccagatggcacattgcaccga

SEQ ID NO: 240 - DNA, 43 bp, synthetic construct
  source 1..43: mol_type = other DNA
gcgccccggtggcactgcggctggaggtgggggttaaagcgga

SEQ ID NO: 241 - DNA, 77 bp, synthetic construct
  source 1..77: mol_type = other DNA
gcgccccggtggcactgcggctggagggtttaattgagttgtcatatgttaataacggtatttggggttaaagcgga

SEQ ID NO: 242 - DNA, 43 bp, synthetic construct; identical to SEQ ID NO: 240
  source 1..43: mol_type = other DNA

SEQ ID NO: 243 - DNA, 77 bp, synthetic construct
  source 1..77: mol_type = other DNA
gcgccccggtggcactgcggctggagggtttaattgagttgtcatatgttaataacggtattgggggttaaagcgga

SEQ ID NO: 244 - DNA, 43 bp, synthetic construct
  source 1..43: mol_type = other DNA
aaacagacaccatggtgcacctgactcctgaggagaagtctgc

SEQ ID NO: 245 - DNA, 77 bp, synthetic construct
  source 1..77: mol_type = other DNA
aaacagacaccatggtgcacctgactcgtttaattgagttgtcatatgttaataacggtatctgtggagaagtctgc

SEQ ID NO: 246 - DNA, 43 bp, synthetic construct; identical to SEQ ID NO: 244
  source 1..43: mol_type = other DNA

SEQ ID NO: 247 - DNA, 77 bp, synthetic construct
  source 1..77: mol_type = other DNA
aaacagacaccatggtgcacctgactcgtttaattgagttgtcatatgttaataacggtatctgaggagaagtctgc

SEQ ID NO: 248 - DNA, 43 bp, synthetic construct
  source 1..43: mol_type = other DNA
caatccttggggcccagactgagcacgtgatggcagaggaaag

SEQ ID NO: 249 - DNA, 80 bp, synthetic construct
  source 1..80: mol_type = other DNA
caatccttggggcccagactgagcacggtttaattgagttgtcatatgttaataacggtatctttgatggcagaggaaag

SEQ ID NO: 250 - DNA, 43 bp, synthetic construct; identical to SEQ ID NO: 248
  source 1..43: mol_type = other DNA

SEQ ID NO: 251 - DNA, 77 bp, synthetic construct
  source 1..77: mol_type = other DNA
caatccttggggcccagactgagcacggtttaattgagttgtcatatgttaataacggtattgatggcagaggaaag

SEQ ID NO: 252 - DNA, 43 bp, synthetic construct
  source 1..43: mol_type = other DNA
cgcacctcatggaatcccttctgcagcacctggatcgcttttc

SEQ ID NO: 253 - DNA, 77 bp, synthetic construct
  source 1..77: mol_type = other DNA
cgcacctcatggaatcccttctgcagcgtttaattgagttgtcatatgttaataacggtatacctgcatcgcttttc

SEQ ID NO: 254 - DNA, 43 bp, synthetic construct; identical to SEQ ID NO: 252
  source 1..43: mol_type = other DNA

SEQ ID NO: 255 - DNA, 77 bp, synthetic construct
  source 1..77: mol_type = other DNA
cgcacctcatggaatcccttctgcagcgtttaattgagttgtcatatgttaataacggtatacctggatcgcttttc

SEQ ID NO: 256 - DNA, 43 bp, synthetic construct
  source 1..43: mol_type = other DNA
ggaagggcctgagtccgagcagaagaagaagggctcccatcac

SEQ ID NO: 257 - DNA, 77 bp, synthetic construct
  source 1..77: mol_type = other DNA
ggaagggcctgagtccgagcagaagaagtttaattgagttgtcatatgttaataacggtatgaagtgctcccatcac

SEQ ID NO: 258 - DNA, 43 bp, synthetic construct; identical to SEQ ID NO: 256
  source 1..43: mol_type = other DNA

SEQ ID NO: 259 - DNA, 77 bp, synthetic construct
  source 1..77: mol_type = other DNA
ggaagggcctgagtccgagcagaagaagtttaattgagttgtcatatgttaataacggtatgaagggctcccatcac

SEQ ID NO: 260 - DNA, 43 bp, synthetic construct
  source 1..43: mol_type = other DNA
gcatgttggggattcctggtgccagaaacaggggtgacgggag

SEQ ID NO: 261 - DNA, 77 bp, synthetic construct
  source 1..77: mol_type = other DNA
gcatgttggggattcctggtgccagaagtttaattgagttgtcatatgttaataacggtatacaggcgtgacgggag

SEQ ID NO: 262 - DNA, 43 bp, synthetic construct; identical to SEQ ID NO: 260
  source 1..43: mol_type = other DNA

SEQ ID NO: 263 - DNA, 77 bp, synthetic construct
  source 1..77: mol_type = other DNA
gcatgttggggattcctggtgccagaagtttaattgagttgtcatatgttaataacggtatacaggggtgacgggag

SEQ ID NO: 264 - DNA, 43 bp, synthetic construct
  source 1..43: mol_type = other DNA
agaagagggtgcattttcaggaggaagcgatggcttcagacag

SEQ ID NO: 265 - DNA, 77 bp, synthetic construct
  source 1..77: mol_type = other DNA
agaagagggtgcattttcaggaggaaggtttaattgagttgtcatatgttaataacggtatcgatgccttcagacag

SEQ ID NO: 266 - DNA, 43 bp, synthetic construct; identical to SEQ ID NO: 264
  source 1..43: mol_type = other DNA

SEQ ID NO: 267 - DNA, 77 bp, synthetic construct
  source 1..77: mol_type = other DNA
agaagagggtgcattttcaggaggaaggtttaattgagttgtcatatgttaataacggtatcgatggcttcagacag

SEQ ID NO: 268 - DNA, 43 bp, synthetic construct
  source 1..43: mol_type = other DNA
cgctcactttgatgtctgcaggccagatgagggctccagatgg

SEQ ID NO: 269 - DNA, 77 bp, synthetic construct
  source 1..77: mol_type = other DNA
cgctcactttgatgtctgcaggccagagtttaattgagttgtcatatgttaataacggtattgagtgctccagatgg

SEQ ID NO: 270 - DNA, 43 bp, synthetic construct; identical to SEQ ID NO: 268
  source 1..43: mol_type = other DNA

SEQ ID NO: 271 - DNA, 77 bp, synthetic construct
  source 1..77: mol_type = other DNA
cgctcactttgatgtctgcaggccagagtttaattgagttgtcatatgttaataacggtattgagggctccagatgg

SEQ ID NO: 272 - DNA, 43 bp, synthetic construct
  source 1..43: mol_type = other DNA
ccccttggcagtcatcttagtcattacctgaggtgttcgttgt

SEQ ID NO: 273 - DNA, 77 bp, synthetic construct
  source 1..77: mol_type = other DNA
ccccttggcagtcatcttagtcattacgtttaattgagttgtcatatgttaataacggtatctgagatgttcgttgt

SEQ ID NO: 274 - DNA, 43 bp, synthetic construct; identical to SEQ ID NO: 272
  source 1..43: mol_type = other DNA

SEQ ID NO: 275 - DNA, 77 bp, synthetic construct
  source 1..77: mol_type = other DNA
ccccttggcagtcatcttagtcattacgtttaattgagttgtcatatgttaataacggtatctgaggtgttcgttgt

SEQ ID NO: 276 - DNA, 20 bp, synthetic construct
  source 1..20: mol_type = other DNA
ggcactgcggctggaggtgg

SEQ ID NO: 277 - DNA, 20 bp, synthetic construct
  source 1..20: mol_type = other DNA
ggcaatgcggctggaggcgg

SEQ ID NO: 278 - DNA, 20 bp, synthetic construct
  source 1..20: mol_type = other DNA
ggcacgacggctggaggtgg

SEQ ID NO: 279 - DNA, 20 bp, synthetic construct
  source 1..20: mol_type = other DNA
ggctctgcggctggaggggg

SEQ ID NO: 280 - DNA, 21 bp, synthetic construct
  source 1..21: mol_type = other DNA
agctctgcgcgctggaggagg

SEQ ID NO: 281 - DNA, 21 bp, synthetic construct
  source 1..21: mol_type = other DNA
ggaactgaggctctgagggtg

SEQ ID NO: 282 - DNA, 20 bp, synthetic construct
  source 1..20: mol_type = other DNA
ggcactggggttggaggtgg

SEQ ID NO: 283 - DNA, 20 bp, synthetic construct
  source 1..20: mol_type = other DNA
aggactgcggctgggggtgg

SEQ ID NO: 284 - DNA, 20 bp, synthetic construct
  source 1..20: mol_type = other DNA
gacactgaggcaggaggtgg

SEQ ID NO: 285 - DNA, 20 bp, synthetic construct
  source 1..20: mol_type = other DNA
gaggctgcggctgggggtgg

SEQ ID NO: 286 - DNA, 20 bp, synthetic construct
  source 1..20: mol_type = other DNA
tgcactgcggccggaggagg

SEQ ID NO: 287 - DNA, 21 bp, synthetic construct
  source 1..21: mol_type = other DNA
gggactgcggctggaggtggg

SEQ ID NO: 288 - DNA, 21 bp, synthetic construct
  source 1..21: mol_type = other DNA
ggcactgtgggctggaggcgg

SEQ ID NO: 289 - DNA, 20 bp, synthetic construct
  source 1..20: mol_type = other DNA
ggcacagcagctggaggtgc

SEQ ID NO: 290 - DNA, 20 bp, synthetic construct
  source 1..20: mol_type = other DNA
agcactctgggtgggggttg

SEQ ID NO: 291 - DNA, 22 bp, synthetic construct
  source 1..22: mol_type = other DNA
ggcactgagggttgggggatgg

SEQ ID NO: 292 - DNA, 20 bp, synthetic construct
  source 1..20: mol_type = other DNA
ggcatcacggctggaggtgg

SEQ ID NO: 293 - DNA, 20 bp, synthetic construct
  source 1..20: mol_type = other DNA
ggctctgtggctggaggagg

SEQ ID NO: 294 - DNA, 20 bp, synthetic construct
  source 1..20: mol_type = other DNA
ggcgctgcggcgggaggtgg

SEQ ID NO: 295 - DNA, 20 bp, synthetic construct
  source 1..20: mol_type = other DNA
cacactgcagctggaggtgg

SEQ ID NO: 296 - DNA, 20 bp, synthetic construct
  source 1..20: mol_type = other DNA
ggtactctggctggaggtgg

SEQ ID NO: 297 - DNA, 20 bp, synthetic construct
  source 1..20: mol_type = other DNA
gacaccacggctggagatgg

SEQ ID NO: 298 - DNA, 20 bp, synthetic construct
  source 1..20: mol_type = other DNA
ggcactgagggtggaggtgg

SEQ ID NO: 299 - DNA, 20 bp, synthetic construct
  source 1..20: mol_type = other DNA
ggggctgcggccggaggtgg

SEQ ID NO: 300 - DNA, 20 bp, synthetic construct
  source 1..20: mol_type = other DNA
agcacaaaggctggaggtgg

SEQ ID NO: 301 - DNA, 20 bp, synthetic construct
  source 1..20: mol_type = other DNA
ggcgctgcggctggagccgg

SEQ ID NO: 302 - DNA, 20 bp, synthetic construct
  source 1..20: mol_type = other DNA
ggcactgctgctgggggtgg

SEQ ID NO: 303 - DNA, 20 bp, synthetic construct
  source 1..20: mol_type = other DNA
ggcacaatggctggaggtga

SEQ ID NO: 304 - DNA, 20 bp, synthetic construct
  source 1..20: mol_type = other DNA
ggcactggggctgggggagg

SEQ ID NO: 305 - DNA, 20 bp, synthetic construct
  source 1..20: mol_type = other DNA
ggctcttcggctggaggtag

SEQ ID NO: 306 - DNA, 20 bp, synthetic construct
  source 1..20: mol_type = other DNA
ggaactgtggctggaggtgg

SEQ ID NO: 307 - DNA, 20 bp, synthetic construct
  source 1..20: mol_type = other DNA
cccactggggctggaggtgg

SEQ ID NO: 308 - DNA, 20 bp, synthetic construct
  source 1..20: mol_type = other DNA
ggcactgagactgggggtgg

SEQ ID NO: 309 - DNA, 20 bp, synthetic construct
  source 1..20: mol_type = other DNA
ggcactgtggctgcaggtgg

SEQ ID NO: 310 - DNA, 20 bp, synthetic construct
  source 1..20: mol_type = other DNA
ggcactgcgggtggaggcgg

SEQ ID NO: 311 - DNA, 20 bp, synthetic construct
  source 1..20: mol_type = other DNA
agcactgtggctgggggagg

SEQ ID NO: 312 - DNA, 20 bp, synthetic construct
  source 1..20: mol_type = other DNA
ggtacagtggctggaggtgg

SEQ ID NO: 313 - DNA, 20 bp, synthetic construct
  source 1..20: mol_type = other DNA
aggactgcgcgtggagatgg

SEQ ID NO: 314 - DNA, 22 bp, synthetic construct
  source 1..22: mol_type = other DNA
gccactggttggctgggcgtgg

SEQ ID NO: 315 - DNA, 21 bp, synthetic construct
  source 1..21: mol_type = other DNA
tgcacagaggctggaggctga

SEQ ID NO: 316 - DNA, 20 bp, synthetic construct
  source 1..20: mol_type = other DNA
catggtgcacctgactcctg

SEQ ID NO: 317 - DNA, 20 bp, synthetic construct
  source 1..20: mol_type = other DNA
catggtgcatctgactcctg

SEQ ID NO: 318 - DNA, 20 bp, synthetic construct
  source 1..20: mol_type = other DNA
catggtgtggcgggcgcctg

SEQ ID NO: 319 - DNA, 20 bp, synthetic construct
  source 1..20: mol_type = other DNA
cacggggcacctgactcctg

SEQ ID NO: 320 - DNA, 20 bp, synthetic construct
  source 1..20: mol_type = other DNA
aatggagcacctgactccca

SEQ ID NO: 321 - DNA, 20 bp, synthetic construct
  source 1..20: mol_type = other DNA
gatggtgcatctgactccag

SEQ ID NO: 322 - DNA, 20 bp, synthetic construct
  source 1..20: mol_type = other DNA
gagtccgagcagaagaagaa

SEQ ID NO: 323 - DNA, 20 bp, synthetic construct
  source 1..20: mol_type = other DNA
gagttagagcagaagaagaa

SEQ ID NO: 324 - DNA, 20 bp, synthetic construct
  source 1..20: mol_type = other DNA
gaggccgagcagaagaaaga

SEQ ID NO: 325 - DNA, 20 bp, synthetic construct
  source 1..20: mol_type = other DNA
ggaatcccttctgcagcacc

SEQ ID NO: 326 - DNA, 20 bp, synthetic construct
  source 1..20: mol_type = other DNA
ggaaccccgtctgcagcacc

SEQ ID NO: 327 - DNA, 20 bp, synthetic construct
  source 1..20: mol_type = other DNA
ggaatatcttctgcagcccc

SEQ ID NO: 328 - DNA, 20 bp, synthetic construct
  source 1..20: mol_type = other DNA
ggcccagactgagcacgtga

SEQ ID NO: 329 - DNA, 20 bp, synthetic construct
  source 1..20: mol_type = other DNA
gacacagaccgggcacgtga

SEQ ID NO: 330 - DNA, 20 bp, synthetic construct
  source 1..20: mol_type = other DNA
cacccagactgagcacgtgc

SEQ ID NO: 331 - DNA, 20 bp, synthetic construct
  source 1..20: mol_type = other DNA
gtcatcttagtcattacctg

SEQ ID NO: 332 - DNA, 20 bp, synthetic construct
  source 1..20: mol_type = other DNA
gattcctggtgccagaaaca

SEQ ID NO: 333 - DNA, 20 bp, synthetic construct
  source 1..20: mol_type = other DNA
gatgtctggtgccagaaaca

SEQ ID NO: 334 - DNA, 20 bp, synthetic construct
  source 1..20: mol_type = other DNA
gattcttgatgccagaaact

SEQ ID NO: 335 - DNA, 20 bp, synthetic construct
  source 1..20: mol_type = other DNA
tattcctggagccagaagca

SEQ ID NO: 336 - DNA, 20 bp, synthetic construct
  source 1..20: mol_type = other DNA
cctccctggtgtcagaaaca

SEQ ID NO: 337 - DNA, 20 bp, synthetic construct
  source 1..20: mol_type = other DNA
ggaacctggtgccagaaaca

SEQ ID NO: 338 - DNA, 20 bp, synthetic construct
  source 1..20: mol_type = other DNA
ccgtcctagtgccagaaaca

SEQ ID NO: 339 - DNA, 20 bp, synthetic construct
  source 1..20: mol_type = other DNA
gaaacttggtgccagaaaca

SEQ ID NO: 340 - DNA, 20 bp, synthetic construct
  source 1..20: mol_type = other DNA
gcattttcaggaggaagcga

SEQ ID NO: 341 - DNA, 20 bp, synthetic construct
  source 1..20: mol_type = other DNA
gcattttcagaaggaagcaa

SEQ ID NO: 342 - DNA, 20 bp, synthetic construct
  source 1..20: mol_type = other DNA
gatgtctgcaggccagatga

SEQ ID NO: 343 - DNA, 20 bp, synthetic construct
  source 1..20: mol_type = other DNA
actgtctgcaggtcagatca

SEQ ID NO: 344 - DNA, 20 bp, synthetic construct
  source 1..20: mol_type = other DNA
taagtctgaaggccagatga

SEQ ID NO: 345 - DNA, 22 bp, synthetic construct
  source 1..22: mol_type = other DNA
aatgtttacaggccagatgagg

SEQ ID NO: 346 - DNA, 20 bp, synthetic construct
  source 1..20: mol_type = other DNA
aatgtccgcagcccagatga

SEQ ID NO: 347 - DNA, 20 bp, synthetic construct
  source 1..20: mol_type = other DNA
cctgtctgcaggccggatga

SEQ ID NO: 348 - DNA, 20 bp, synthetic construct
  source 1..20: mol_type = other DNA
gatgtctgcaggacagatgc

SEQ ID NO: 349 - DNA, 21 bp, synthetic construct
  source 1..21: mol_type = other DNA
gatgtctgcaggccagagacg

SEQ ID NO: 350 - DNA, 20 bp, synthetic construct
  source 1..20: mol_type = other DNA
gatgtctggaggtcagatgg

SEQ ID NO: 351 - DNA, 20 bp, synthetic construct
  source 1..20: mol_type = other DNA
ggtgtgtgcaggccagatca

SEQ ID NO: 352 - DNA, 21 bp, synthetic construct
  source 1..21: mol_type = other DNA
ggtgtctgcagggccagatgc

SEQ ID NO: 353 - DNA, 20 bp, synthetic construct
  source 1..20: mol_type = other DNA
tgtgtctgcaggccagaggg

SEQ ID NO: 354 - DNA, 20 bp, synthetic construct
  source 1..20: mol_type = other DNA
gatgtatggaggccagaaga

SEQ ID NO: 355 - DNA, 20 bp, synthetic construct
  source 1..20: mol_type = other DNA
gtcatctgcaggccagatgg

SEQ ID NO: 356 - DNA, 20 bp, synthetic construct
  source 1..20: mol_type = other DNA
aatatctgcaggtcagagga

SEQ ID NO: 357 - DNA, 21 bp, synthetic construct
  source 1..21: mol_type = other DNA
cccgtctgcaggccagatgga

SEQ ID NO: 358 - DNA, 20 bp, synthetic construct
  source 1..20: mol_type = other DNA
aatgactacaggtcagatga

SEQ ID NO: 359-362 - skipped (4 entries)

SEQ ID NO: 363 - DNA, 10 bp, synthetic construct
  source 1..10: mol_type = other DNA
gcgctggagg

SEQ ID NO: 364 - DNA, 10 bp, synthetic construct
  source 1..10: mol_type = other DNA
ggctctgagg

SEQ ID NO: 365-373 - skipped (9 entries)

SEQ ID NO: 374 - DNA, 11 bp, synthetic construct
  source 1..11: mol_type = other DNA
gggttggggga

SEQ ID NO: 375-395 - skipped (21 entries)

SEQ ID NO: 396 - DNA, 10 bp, synthetic construct
  source 1..10: mol_type = other DNA
cgcgtggaga

SEQ ID NO: 397 - skipped

SEQ ID NO: 398 - DNA, 10 bp, synthetic construct
  source 1..10: mol_type = other DNA
ggctggaggc

SEQ ID NO: 399 - DNA, 10 bp, synthetic construct
  source 1..10: mol_type = other DNA
tgggggttaa

SEQ ID NO: 400 - DNA, 10 bp, synthetic construct
  source 1..10: mol_type = other DNA
cggaggcaac

SEQ ID NO: 401 - DNA, 10 bp, synthetic construct
  source 1..10: mol_type = other DNA
tggggggttg

SEQ ID NO: 402 - DNA, 10 bp, synthetic construct
  source 1..10: mol_type = other DNA
gggtggggtt

SEQ ID NO: 403 - DNA, 10 bp, synthetic construct
  source 1..10: mol_type = other DNA
agggggagtg

SEQ ID NO: 404 - DNA, 10 bp, synthetic construct
  source 1..10: mol_type = other DNA
gtggggtgca

SEQ ID NO: 405 - DNA, 10 bp, synthetic construct
  source 1..10: mol_type = other DNA
tgggggctcg

SEQ ID NO: 406 - DNA, 10 bp, synthetic construct
  source 1..10: mol_type = other DNA
tggtggctca

SEQ ID NO: 407 - DNA, 10 bp, synthetic construct
  source 1..10: mol_type = other DNA
tggggggcag

SEQ ID NO: 408 - DNA, 10 bp, synthetic construct
  source 1..10: mol_type = other DNA
tggaggtggg

SEQ ID NO: 409 - DNA, 10 bp, synthetic construct
  source 1..10: mol_type = other DNA
aggtggagga

SEQ ID NO: 410 - DNA, 10 bp, synthetic construct
  source 1..10: mol_type = other DNA
gggaagaagt

SEQ ID NO: 411 - DNA, 10 bp, synthetic construct
  source 1..10: mol_type = other DNA
cgggggataa

SEQ ID NO: 412 - DNA, 10 bp, synthetic construct
  source 1..10: mol_type = other DNA
tgctggagca

SEQ ID NO: 413 - DNA, 10 bp, synthetic construct
  source 1..10: mol_type = other DNA
ttggggggat

SEQ ID NO: 414 - DNA, 10 bp, synthetic construct
  source 1..10: mol_type = other DNA
tggaggagtg

SEQ ID NO: 415 - DNA, 10 bp, synthetic construct
  source 1..10: mol_type = other DNA
tggagggggc

SEQ ID NO: 416 - DNA, 10 bp, synthetic construct
  source 1..10: mol_type = other DNA
aggtggaaga

SEQ ID NO: 417 - DNA, 10 bp, synthetic construct
  source 1..10: mol_type = other DNA
tggaggagct

SEQ ID NO: 418 - DNA, 10 bp, synthetic construct
  source 1..10: mol_type = other DNA
tggtggggag

SEQ ID NO: 419 - DNA, 10 bp, synthetic construct
  source 1..10: mol_type = other DNA
tggtggggtg

SEQ ID NO: 420 - DNA, 10 bp, synthetic construct
  source 1..10: mol_type = other DNA
tggtgggatg

SEQ ID NO: 421 - DNA, 10 bp, synthetic construct
  source 1..10: mol_type = other DNA
tgggggcagt

SEQ ID NO: 422 - DNA, 10 bp, synthetic construct
  source 1..10: mol_type = other DNA
tggtggcgct

SEQ ID NO: 423 - DNA, 10 bp, synthetic construct
  source 1..10: mol_type = other DNA
tggaggaggt

SEQ ID NO: 424 - DNA, 10 bp, synthetic construct
  source 1..10: mol_type = other DNA
cggcggccgg

SEQ ID NO: 425 - DNA, 10 bp, synthetic construct
  source 1..10: mol_type = other DNA
tggtgggagg

SEQ ID NO: 426 - DNA, 10 bp, synthetic construct
  source 1..10: mol_type = other DNA
tgaaggcaga

SEQ ID NO: 427 - DNA, 10 bp, synthetic construct
  source 1..10: mol_type = other DNA
agggggtcta

SEQ ID NO: 428 - DNA, 10 bp, synthetic construct
  source 1..10: mol_type = other DNA
tagcgggtag

SEQ ID NO: 429 - DNA, 10 bp, synthetic construct
  source 1..10: mol_type = other DNA
tggcagcagc

SEQ ID NO: 430 - DNA, 10 bp, synthetic construct
  source 1..10: mol_type = other DNA
tgggggtgtg

SEQ ID NO: 431 - DNA, 10 bp, synthetic construct
  source 1..10: mol_type = other DNA
tgggggtggg

SEQ ID NO: 432 - DNA, 10 bp, synthetic construct
  source 1..10: mol_type = other DNA
tggaggtact

SEQ ID NO: 433 - DNA, 10 bp, synthetic construct
  source 1..10: mol_type = other DNA
cggggggtgc

SEQ ID NO: 434 - DNA, 10 bp, synthetic construct
  source 1..10: mol_type = other DNA
agggggccct

SEQ ID NO: 435 - DNA, 10 bp, synthetic construct
  source 1..10: mol_type = other DNA
tggaagaagc

SEQ ID NO: 436 - DNA, 10 bp, synthetic construct
  source 1..10: mol_type = other DNA
tggtggcctc

SEQ ID NO: 437 - DNA, 10 bp, synthetic construct
  source 1..10: mol_type = other DNA
tggtggctca

SEQ ID NO: 438 - DNA, 10 bp, synthetic construct
  source 1..10: mol_type = other DNA
tgaaagcacc

SEQ ID NO: 439 - DNA, 13 bp, synthetic construct
  source 1..13: mol_type = other DNA
gtgcacctgactc

SEQ ID NO: 440 - DNA, 13 bp, synthetic construct
  source 1..13: mol_type = other DNA
gtgcatctgactc

SEQ ID NO: 441 - DNA, 13 bp, synthetic construct
  source 1..13: mol_type = other DNA
gtgtggcgggcgc

SEQ ID NO: 442 - DNA, 13 bp, synthetic construct
  source 1..13: mol_type = other DNA
gggcacctgactc

SEQ ID NO: 443 - DNA, 13 bp, synthetic construct
  source 1..13: mol_type = other DNA
gagcacctgactc

SEQ ID NO: 444 - DNA, 13 bp, synthetic construct
  source 1..13: mol_type = other DNA
gtgcatctgactc

SEQ ID NO: 445 - DNA, 14 bp, synthetic construct
  source 1..14: mol_type = other DNA
ctgaggagaagtct

SEQ ID NO: 446 - DNA, 14 bp, synthetic construct
  source 1..14: mol_type = other DNA
ctgaggagaagact

SEQ ID NO: 447 - DNA, 14 bp, synthetic construct
  source 1..14: mol_type = other DNA
ctgtagtcctagct

SEQ ID NO: 448 - DNA, 14 bp, synthetic construct
  source 1..14: mol_type = other DNA
ctgaggcgacagct

SEQ ID NO: 449 - DNA, 14 bp, synthetic construct
  source 1..14: mol_type = other DNA
ccaaggcatggtat

SEQ ID NO: 450 - DNA, 14 bp, synthetic construct
  source 1..14: mol_type = other DNA
cagaggctgtattc

SEQ ID NO: 451 - DNA, 15 bp, synthetic construct
  source 1..15: mol_type = other DNA
gtccgagcagaagaa

SEQ ID NO: 452 - DNA, 15 bp, synthetic construct
  source 1..15: mol_type = other DNA
gttagagcagaagaa

SEQ ID NO: 453 - DNA, 15 bp, synthetic construct
  source 1..15: mol_type = other DNA
ggccgagcagaagaa

SEQ ID NO: 454 - DNA, 13 bp, synthetic construct
  source 1..13: mol_type = other DNA
gaagggctcccat

SEQ ID NO: 455 - DNA, 13 bp, synthetic construct
  source 1..13: mol_type = other DNA
gaaaggcatggag

SEQ ID NO: 456 - DNA, 13 bp, synthetic construct
  source 1..13: mol_type = other DNA
agacggcgacaga

SEQ ID NO: 457 - DNA, 14 bp, synthetic construct
  source 1..14: mol_type = other DNA
atcccttctgcagc

SEQ ID NO: 458 - DNA, 14 bp, synthetic construct
  source 1..14: mol_type = other DNA
accccgtctgcagc

SEQ ID NO: 459 - DNA, 14 bp, synthetic construct
  source 1..14: mol_type = other DNA
atatcttctgcagc

SEQ ID NO: 460 - DNA, 17 bp, synthetic construct
  source 1..17: mol_type = other DNA
acctggatcgcttttcc

SEQ ID NO: 461 - DNA, 17 bp, synthetic construct
  source 1..17: mol_type = other DNA
accaggccccctccgtg

SEQ ID NO: 462 - DNA, 17 bp, synthetic construct
  source 1..17: mol_type = other DNA
cccaggttcatctcgag

SEQ ID NO: 463 - DNA, 13 bp, synthetic construct
  source 1..13: mol_type = other DNA
cagactgagcacg

SEQ ID NO: 464 - DNA, 13 bp, synthetic construct
  source 1..13: mol_type = other DNA
cagaccgggcacg

SEQ ID NO: 465 - DNA, 13 bp, synthetic construct
  source 1..13: mol_type = other DNA
cagactgagcacg

SEQ ID NO: 466 - DNA, 10 bp, synthetic construct
  source 1..10: mol_type = other DNA
tgatggcaga

SEQ ID NO: 467 - DNA, 10 bp, synthetic construct
  source 1..10: mol_type = other DNA
tgagggaagc

SEQ ID NO: 468 - DNA, 10 bp, synthetic construct
  source 1..10: mol_type = other DNA
tgctggagcc

SEQ ID NO: 469 - DNA, 15 bp, synthetic construct
  source 1..15: mol_type = other DNA
catcttagtcattac

SEQ ID NO: 470 - DNA, 14 bp, synthetic construct
  source 1..14: mol_type = other DNA
ctgaggtgttcgtt

SEQ ID NO: 471 - DNA, 13 bp, synthetic construct
  source 1..13: mol_type = other DNA
cctggtgccagaa

SEQ ID NO: 472 - DNA, 13 bp, synthetic construct
  source 1..13: mol_type = other DNA
tctggtgccagaa

SEQ ID NO: 473 - DNA, 13 bp, synthetic construct
  source 1..13: mol_type = other DNA
cttgatgccagaa

SEQ ID NO: 474 - DNA, 13 bp, synthetic construct
  source 1..13: mol_type = other DNA
cctggagccagaa

SEQ ID NO: 475 - DNA, 13 bp, synthetic construct
  source 1..13: mol_type = other DNA
cctggtgtcagaa

SEQ ID NO: 476 - DNA, 13 bp, synthetic construct
  source 1..13: mol_type = other DNA
cctggtgccagaa

SEQ ID NO: 477 - DNA, 13 bp, synthetic construct
  source 1..13: mol_type = other DNA
cctagtgccagaa

SEQ ID NO: 478 - DNA, 13 bp, synthetic construct
  source 1..13: mol_type = other DNA
cttggtgccagaa

SEQ ID NO: 479 - DNA, 11 bp, synthetic construct
  source 1..11: mol_type = other DNA
acaggggtgac

SEQ ID NO: 480 - DNA, 11 bp, synthetic construct
  source 1..11: mol_type = other DNA
acaagggtgtt

SEQ ID NO: 481 - DNA, 11 bp, synthetic construct
  source 1..11: mol_type = other DNA
actgggtctta

SEQ ID NO: 482 - DNA, 11 bp, synthetic construct
  source 1..11: mol_type = other DNA
gcagggcaact

SEQ ID NO: 483 - DNA, 11 bp, synthetic construct
  source 1..11: mol_type = other DNA
acaaggtaaaa

SEQ ID NO: 484 - DNA, 11 bp, synthetic construct
  source 1..11: mol_type = other DNA
acagagacaaa

SEQ ID NO: 485 - DNA, 11 bp, synthetic construct
  source 1..11: mol_type = other DNA
acatggaaaat

SEQ ID NO: 486 - DNA, 11 bp, synthetic construct
  source 1..11: mol_type = other DNA
acagggcattt

SEQ ID NO: 487 - DNA, 15 bp, synthetic construct
  source 1..15: mol_type = other DNA
attttcaggaggaag

SEQ ID NO: 488 - DNA, 15 bp, synthetic construct
  source 1..15: mol_type = other DNA
attttcagaaggaag

SEQ ID NO: 489 - DNA, 15 bp, synthetic construct
  source 1..15: mol_type = other DNA
cgatggcttcagaca

SEQ ID NO: 490 - DNA, 15 bp, synthetic construct
  source 1..15: mol_type = other DNA
caagggttctttata

SEQ ID NO: 491 - DNA, 13 bp, synthetic construct
  source 1..13: mol_type = other DNA
tctgcaggccaga

SEQ ID NO: 492 - DNA, 13 bp, synthetic construct
  source 1..13: mol_type = other DNA
tctgcaggtcaga

SEQ ID NO: 493 - DNA, 13 bp, synthetic construct
  source 1..13: mol_type = other DNA
tctgaaggccaga

SEQ ID NO: 494 - DNA, 15 bp, synthetic construct
  source 1..15: mol_type = other DNA
tttacaggccagata

SEQ ID NO: 495 - DNA, 13 bp, synthetic construct
  source 1..13: mol_type = other DNA
tccgcagcccaga

SEQ ID NO: 496 - DNA, 13 bp, synthetic construct
  source 1..13: mol_type = other DNA
tctgcaggccgga

SEQ ID NO: 497 - DNA, 13 bp, synthetic construct
  source 1..13: mol_type = other DNA
tctgcaggacaga

SEQ ID NO: 498 - DNA, 14 bp, synthetic construct
  source 1..14: mol_type = other DNA
tctgcaggccagag

SEQ ID NO: 499 - DNA, 13 bp, synthetic construct
  source 1..13: mol_type = other DNA
tctggaggtcaga

SEQ ID NO: 500 - DNA, 13 bp, synthetic construct
  source 1..13: mol_type = other DNA
tgtgcaggccaga

SEQ ID NO: 501 - DNA, 14 bp, synthetic construct
  source 1..14: mol_type = other DNA
tctgcagggccaga

SEQ ID NO: 502 - DNA, 13 bp, synthetic construct
  source 1..13: mol_type = other DNA
tctgcaggccaga

SEQ ID NO: 503 - DNA, 13 bp, synthetic construct
  source 1..13: mol_type = other DNA
tatggaggccaga

SEQ ID NO: 504 - DNA, 13 bp, synthetic construct
  source 1..13: mol_type = other DNA
tctgcaggccaga

SEQ ID NO: 505 - DNA, 13 bp, synthetic construct
  source 1..13: mol_type = other DNA
tctgcaggtcaga

SEQ ID NO: 506 - DNA, 14 bp, synthetic construct
  source 1..14: mol_type = other DNA
tctgcaggccagat

SEQ ID NO: 507 - DNA, 13 bp, synthetic construct
  source 1..13: mol_type = other DNA
actacaggtcaga

SEQ ID NO: 508 - DNA, 22 bp, synthetic construct
  source 1..22: mol_type = other DNA
tgagggctccagatggcacatt

SEQ ID NO: 509 - DNA, 22 bp, synthetic construct
  source 1..22: mol_type = other DNA
tcagggagaaagctggaatata

SEQ ID NO: 510 - DNA, 22 bp, synthetic construct
  source 1..22: mol_type = other DNA
tgaggggttcacagcaccatgg

SEQ ID NO: 511 - DNA, 22 bp, synthetic construct
  source 1..22: mol_type = other DNA
agaggaggaagcagtgagggga

SEQ ID NO: 512 - DNA, 22 bp, synthetic construct
  source 1..22: mol_type = other DNA
tgatggcaatggaaccaaaggc

SEQ ID NO: 513 - DNA, 22 bp, synthetic construct
  source 1..22: mol_type = other DNA
tgagagcttgtctggcagctct

SEQ ID NO: 514 - DNA, 22 bp, synthetic construct
  source 1..22: mol_type = other DNA
tgcagggtggagggagggtgcc

SEQ ID NO: 515 - DNA, 22 bp, synthetic construct
  source 1..22: mol_type = other DNA
acgaggagtgcacagagctcct

SEQ ID NO: 516 - DNA, 22 bp, synthetic construct
  source 1..22: mol_type = other DNA
tggagggaacagtctgggagga

SEQ ID NO: 517 - DNA, 22 bp, synthetic construct
  source 1..22: mol_type = other DNA
tcatggcaaatgcagtcacgaa

SEQ ID NO: 518 - DNA, 22 bp, synthetic construct
  source 1..22: mol_type = other DNA
tgctggtgaccgcctggccctg

SEQ ID NO: 519 - DNA, 22 bp, synthetic construct
  source 1..22: mol_type = other DNA
gggagggtgcctggggagttga

SEQ ID NO: 520 - DNA, 22 bp, synthetic construct
  source 1..22: mol_type = other DNA
agaggggtagccccactctgaa

SEQ ID NO: 521 - DNA, 22 bp, synthetic construct
  source 1..22: mol_type = other DNA
tgggggctgaggaatctgcttc

SEQ ID NO: 522 - DNA, 22 bp, synthetic construct
  source 1..22: mol_type = other DNA
ggagggatgtcagcagaggctg

SEQ ID NO: 523 - DNA, 22 bp, synthetic construct
  source 1..22: mol_type = other DNA
ggatggctgcagggtggaagaa

SEQ ID NO: 524 - DNA, 22 bp, synthetic construct
  source 1..22: mol_type = other DNA
tgagggctctgaatgctatgtg